European Patent Specification EP 3 472 362 B1, published September 6, 2023. Title: NUCLEIC ACID MOLECULES FOR REDUCTION OF PAPD5 AND/OR PAPD7 mRNA FOR TREATING HEPATITIS B INFECTION. Applicant: F. Hoffmann la Roche. The sequence listing filed with the application follows.

SEQUENCE LISTING (267 sequences)

SEQ ID NO: 1 - protein, 698 aa, Homo sapiens
MRPRPRSAPGKPRRRSRARLRSSRTPSGGASGGGGSSSSSSTATGGSGSSTGSPGGAASAPAPAPAGMYRSGERLLGSHALPAEQRDFLPLETTNNNNNHHQPGAWARRAGSSASSPPSASSSPHPSAAVPAADPADSASGSSNKRKRDNKASTYGLNYSLLQPSGGRAAGGGRADGGGVVYSGTPWKRRNYNQGVVGLHEEISDFYEYMSPRPEEEKMRMEVVNRIESVIKELWPSADVQIFGSFKTGLYLPTSDIDLVVFGKWENLPLWTLEEALRKHKVADEDSVKVLDKATVPIIKLTDSFTEVKVDISFNVQNGVRAADLIKDFTKKYPVLPYLVLVLKQFLLQRDLNEVFTGGIGSYSLFLMAVSFLQLHPREDACIPNTNYGVLLIEFFELYGRHFNYLKTGIRIKDGGSYVAKDEVQKNMLDGYRPSMLYIEDPLQPGNDVGRSSYGAMQVKQAFDYAYVVLSHAVSPIAKYYPNNETESILGRIIRVTDEVATYRDWISKQWGLKNRPEPSCNGNGVTLIVDTQQLDKCNNNLSEENEALGKCRSKTSESLSKHSSNSSSGPVSSSSATQSSSSDVDSDATPCKTPKQLLCRPSTGNRVGSQDVSLESSQAVGKMQSTQTTNTSNSTNKSQHGSARLFRSSSKGFQGTTQTSHGSLMTNKQHQGKSNNQYYHGKKRKHKRDAPLSDLCR

SEQ ID NO: 2 - protein, 651 aa, Homo sapiens
MRPRPRSAPGKPRRRSRARLRSSRTPSGGASGGGGSSSSSSTATGGSGSSTGSPGGAASAPAPAPAGMYRSGERLLGSHALPAEQRDFLPLETTNNNNNHHQPGAWARRAGSSASSPPSASSSPHPSAAVPAADPADSASGSSNKRKRDNKASTYGLNYSLLQPSGGRAAGGGRADGGGVVYSGTPWKRRNYNQGVVGLHEEISDFYEYMSPRPEEEKMRMEVVNRIESVIKELWPSADVQIFGSFKTGLYLPTSDIDLVVFGKWENLPLWTLEEALRKHKVADEDSVKVLDKATVPIIKLTDSFTEVKVDISFNVQNGVRAADLIKDFTKKYPVLPYLVLVLKQFLLQRDLNEVFTGGIGSYSLFLMAVSFLQLHPREDACIPNTNYGVLLIEFFELYGRHFNYLKTGIRIKDGGSYVAKDEVQKNMLDGYRPSMLYIEDPLQPGNDVGRSSYGAMQVKQAFDYAYVVLSHAVSPIAKYYPNNETESILGRIIRVTDEVATYRDWISKQWGLKNRPEPSCNGPVSSSSATQSSSSDVDSDATPCKTPKQLLCRPSTGNRVGSQDVSLESSQAVGKMQSTQTTNTSNSTNKSQHGSARLFRSSSKGFQGTTQTSHGSLMTNKQHQGKSNNQYYHGKKRKHKRDAPLSDLCR

SEQ ID NO: 3 - protein, 792 aa, Homo sapiens
MDPRVAWIQPEQKGPANALWMQIWETSQGVGRGGSGFASYFCLNSPALDTAAAAGAAGRGSGGLGPALPAASPPPPGPTAPAALPPALLTALGPAAEGARRLHKSPSLSSSSSSSSSNAESGTESPGCSSSSSSSASLGRPGGGRGGAFFNFADGAPSAPGTANGHPGPRGPAPAGSPSQHQFHPGRRKRENKASTYGLNYLLSGSRAAALSGGGGPGAQAPRPGTPWKSRAYSPGIQGLHEEIIDFYNFMSPCPEEAAMRREVVKRIETVVKDLWPTADVQIFGSFSTGLYLPTSDIDLVVFGKWERPPLQLLEQALRKHNVAEPCSIKVLDKATVPIIKLTDQETEVKVDISFNMETGVRAAEFIKNYMKKYSLLPYLILVLKQFLLQRDLNEVFTGGISSYSLILMAISFLQLHPRIDARRADENLGMLLVEFFELYGRNFNYLKTGIRIKEGGAYIAKEEIMKAMTSGYRPSMLCIEDPLLPGNDVGRSSYGAMQVKQVFDYAYIVLSHAVSPLARSYPNRDAESTLGRIIKVTQEVIDYRRWIKEKWGSKAHPSPGMDSRIKIKERIATCNGEQTQNREPESPYGQRLTLSLSSPQLLSSGSSASSVSSLSGSDVDSDTPPCTTPSVYQFSLQAPAPLMAGLPTALPMPSGKPQPTTSRTLIMTTNNQTRFTIPPPTLGVAPVPCRQAGVEGTASLKAVHHMSSPAIPSASPNPLSSPHLYHKQHNGMKLSMKGSHGHTQGGGYSSVGSGGVRPPVGNRGHHQYNRTGWRRKKHTHTRDSLPVSLSR

SEQ ID NO: 4 - DNA, 8114 bp, Homo sapiens
acaacgcgctccctgcggggcgggcggcaacctccatgcggcctcgtccacgctcagcaccggggaagccgaggcggagaagccgcgcgcgcctcagaagctcccggacgcccagcggcggcgcgagcggcggcggcggcagcagcagcagcagcagcacggccaccggcgggagcggcagcagcaccggcagccccggcggcgcggcctcggccccggccccggccccggccggcatgtatcgctccggggagcgcctgctgggcagccacgcgctgcccgcggagcagcgggacttcctgcccctagagacgaccaacaacaacaacaaccaccaccagcccggggcctgggcccgccgggcgggctcctcggcgtcctcgcctccctcggcgtcctcgtccccgcacccttcggccgccgtccccgccgccgatccagccgattcggcctcgggcagcagcaacaagaggaagcgcgacaacaaggccagcacgtatggactcaactacagcctgctgcagcccagcggagggcgggccgcggggggcggccgagcagacggcggcggggtcgtgtacagcgggaccccgtggaaacggaggaactacaaccagggagtcgtgggtctgcatgaagaaatcagtgatttttatgaatacatgtctccaagacctgaggaggagaagatgcggatggaggtggtgaacaggatcgagagtgtaattaaggagctctggcccagcgctgacgtccagatatttggaagttttaaaactggactttatttacctactagtgacatcgacctagtggtgtttgggaagtgggagaacctacccctctggactctggaagaagctcttcggaaacacaaagtcgcagatgaggattcggtgaaagttttagacaaagcaactgtacctattattaaattaacagattcttttactgaagtgaaagttgatatcagctttaatgtacagaatggcgtgagagcagctgacctcatcaaagattttaccaagaaatatcctgtattgccatacttggttttagtattgaaacaattcctattgcagagggaccttaatgaagtatttacaggtggaattggttcttatagtctctttttaatggcagtcagtttccttcagttacatcccagggaagatgcttgcatccccaatacaaactatggtgttctcttaatagaattttttgaattatatggacgacacttcaattatttaaagactggcatccggataaaggatggtggttcatatgtggccaaagatgaagtacagaaaaatatgctagatggctacaggccatcaatgctttatatcgaagatcctttacaaccaggtaacgatgttggaaggagttcatatggggccatgcaagtgaagcaggcctttgattatgcctacgttgttttgagtcatgctgtatcaccaatagcaaagtactatcccaacaatgaaacagaaagcatactaggtagaataattagagtaacagatgaagttgccacatatagagattggatatcaaagcagtggggcttgaagaatagacctgagccttcatgcaatggaaatggtgttaccttgatagtagatactcagcagttagataaatgtaataataatctatctgaagaaaatgaagcccttggaaaatgtagaagtaaaacctcggaatctcttagtaaacactcttcaaactcttcatcaggtccagtgtcgtcctcttctgccacacagtccagctctagtgatgtagattccgatgcaacaccatgcaaaaccccgaaacagctgctttgccgtccgtccactgggaaccgagtagggtcgcaagatgtatccttggagtcctctcaggcagttgggaaaatgcaaagcacccaaaccactaacacatccaacagcaccaacaaatctcagcatggatcagcaaggctctttcgttcttccagcaaaggcttccaaggtacaactcaaacaagccatggttccttgatgacaaacaaacaacatcaaggcaaatccaataatcagtattaccatggcaaaaagaggaaacacaagagggacgcgcccctctcagacctctgtagatagtcagcgctgcgcggtggactgtcttctctgtgcaatgatctcatgctcaggacagttgcgcagggactcctgggagatattcaggagcctcacactgttcagacgttgacttagcaactgcgttttttcccagctcgccacagaatggatcatgaagactgacaactgcaaaaaaaacaaaacaaaacaaaaaaaaaagcaagcaaaaaagagggaaaaaaaaggctgcttatttgataagtcatatgctacaacagggtcattttaagatttaaagcttgaatgtaaaataaatatatttctcattggctttatgcagagttatagggaatagtattcagtgttggtagggtgatagaaacaaaaaacagtatcagaggatgaggtggggaaggaaaacaaaggtatctgataggaagtccagattccaaaggggaaagtgatctgtgcatgttttttttttaaatatttttgcatatatttaccattttattgtgtgtatatatagaagaccatataggagattgatatttgtaatagtggatttgttaataatactttttacataacattactgtttaaattgtaaacagattttttctcaggattagtttgaaaaataatctaaattgtcatcttaacatccatatatagggaagtgattagttctattactcaatttgtttttctcagcattgaaatgacttaatagaacccttgtgtcctgctgcaaaaatttttcctctctaaagaaaaggtttatggtggcaaatgatgtttattttattttgtaaaaaaaaaaaaatgtactatgtacttttgtgtaaacactgaaaaatctctggtcatctccgagaattaacttgcaactgttttctatagtgctgtcgtcttgggcaatgggcaattacatgactttgtgtttgcttcctttgcagtcttttttttttccccccatttcttcctaataggaaaaaaaaaaaaaaaaaggtcacccatgtctggtctcattcctgttgcagtgaaacttcgagttccacagactttgcatgctggcttctctaaccctgtgtgctgcgtgtgcctgtttctcatctcttattctttttaaaattcatgcttaactactgtgggagaataactgtaaacagctttaattaaatcatacttataaaaaactattttcttatattccactctatgcttttggtattgttgatctttacaaattaaatggtctttgataatggatctattttgtattgccttattaagaccaaatacttcttgtcatcccattctttatcctcttctttcatggaattgttatcgttaattaaaacttttttaaacattggcttgtttcaatcatactgtaaattttggttgtagtcagctttgagtgcaatgagatgtataattctgttatcattacctgttgagtttgaaactcagttgggaatatttaatataatagaatgtaagtgacatttctgaaaatgctttctttcagggtgaaagctcttatgtttagcatcaatgtgtatggctctgttaaatgcagccatttctgagacgagattcttttatatatatatacatataaagtactattggcttttaggagtttcttttatatacatttatgaaatactgaagaccaatcagaccattaatggacacttagtgtaactttttataaagaaaataatgctaaagtaagaccaaaactgatgtcatcactgaaattaacaattttcaatatgttcatattttaattcacaatggaaaaatgtgttccaaaactggaaactcatagtactcgtgtaaactgtggaagatttcaaatgtgatgttattttgacaatgttttaaattttagagtcacattttattctgatcagaatttttattgagatgttgagcttttgtttttgaaactagtttgtcataacattgtgcataatcacagtatttattttctaggacaattgtgaatgtgtagacttatgtttactgctaagggaacaattatttataaaataatattaaatccagtattagctgcctatttcagacacttaatacttgcagagatctatgttacatttaccacactgaagttttttttgttgttttttgtttgtttttaaagaatcaccctcattgttgaaagtaaatgtactcttagggtgcgaatattagtgttccaataagcatgtgattatattaaggtggtggtagcgggaagataattctgattccattgggaatcttaggttttcgtaaatttattgggaaaatagtttttcctgtactgctgaagtttctttttggtaaacagtatctttctaaaagaaaaaagcatgaaggagaaattgaggtgtgtatacatttcctcaaatgaccagcattgtattcgtgaatactgtgtatcttgcagtgaacagtgtggaagctgttcatttttcaatctgaagtaaaatactttcaagaacttttagtttgcctgctcatttgttttatacatttcatctatttgactcctatcttatttcttttttgagttttaatacttcctatattttgtgaatatatcagaaatgtgtcatttatatattagagtccattcatatccatgaatcataaccttcctttgctaatacttgttgaatgggattttacaaattctccctcactctggtgacatttctcaggcagtcatgtatgtgtacctggccattagaaatattaatatttaaagactgttttttagaggagctgatgggttggtgaggtgtcagcacaaaatcttactggttatgttttgatgataaaagtatatccattttttccctccagctttaaggtgactgtgaaggtgcctggttttgaatgtctttgtttggtttggagatgtcgcactcagttttcaaatctagcttggatctgtaggacctatgttttttacaagtaattgccctccagtcttcaacagttgattctgttttatttttatcctgttttgagtgtactttacctttacttgcattttgagcctcattaatatttaggttatttgatttggctccagatattcctagatctgcacagggcaaaacatgggctatagggtgagcatttttaattgtctttttctgctggaaccttatatctctccatgtgttttctgctccttccctcccccatgaaatggtaagtgtgacttgtgtttgcctgaacctgtggactagtgtttggggtttctggaaacactagagggtcagaaaagagtaatgaccaccgtgacgtgcaggattctcttgctgtgacatgttcattgcaaagccctctccagtgactaggaggtgtagttattaaggttgatctgttagaaatcaccattattaggtattagtggtagatgttgctgatacttttattggtcatgactacatctcagttttactttaatattgatctatagtttgatcagttccttgaattctaatatgttgatttctcagtgtttctgtcactaaccaagaatgtttctaggcagttggttgcttcacagtcaaaactaaatggtaaactatcaaaaatacattcccaattttgctgtgataaatattgaaatgttaaaattaatgaacagaagaatttattcttacccatctattcttgttctcctagttcattaaactttcagttattggaaaggcacattctcaaagtattttatgagcaaaatattctataaatgcgtctaacaaacctaattgaatataaaagttatatttagtagttactgttgatagtaattttcatcagggtcatagttcatctagtaaaatatttagagaatgatgttaacattccagcattaaagtgggaacaaagatttatatatgaaattccttaaaagagttcatcttgccttggtttctgaccctcaagactctagctacctgccatcttgtcaaaacatttgtgggtagaataagtgttaaagatcaaattttaatatgcttctcgatatttaacatagctaagaagccagattttactgtagaagttatttacatgatttgaaaacttgacctaactggaagcctttttctcagtcatcttgttctaagccatcttgacttcacacccttagcgacttttcttttttttttggtcaaagataatgagctaaatatatatagacgttgaatgttgacaaaattattaaccagaaaaattgcttataaaggctgctgatctatttgatacctagaattaaatatttgaggacagtttttagttaataaactgctaatgtttattttactgtctctcaggtttttggtttttttaaaaaaaatgtgtttggcctttacattttctacttaagtgtgtactttattgagtttaaccttgtctgtagcctagtagcctgaaagaaaaggagacagaaccagagagatggatgtagtgcattccctttggttattacacatttgtggtagctcctggatttactgagagatattttagctatgtcaataagaacagctaatgatgtggaaatcaggtgttctcttgtgtatttcagtgaacatttttattagtagttgcatatcatctctagttccacattttaacttaacgtctttgtggcttcaccactgagctacctttcactacaccagcttctgtgtggcctggtaacatggaaggtctctcctaaggacagtctggacgtattttgggggaatgttatttatcttaaagatgcctagaaacaaaacgcatatagtaccagtgagaaactatgaagtaaacaagttgctcaggccgggcatggtggctcacgcctgtaatcccagcactttgggaggccgaagcgggaggatggcttgaggctgggagtttgagaccttcatctcttaaaaaaacaaacaaaaacctgaatggtgaggtgtggtggaattgggtaggggagggaaaggaggacttggaaaagcattctccaaagccagcaacttggtgaagttcagtacttgcctcttagaggttaggccatgcctttcaaagagagtgaaatgatgggttatcagccacattcttggagttaatatttttcttcatctttcagtttgggttctgtgctattcatagttcttccctaagaccatttcattattaccttttatatttagttgcaatttattataatatgttgttttgtccctgaacttaatctcctaattttaagatcctctctgatttttgcatattgaaacttacagaagtcactttaaaaaagtcttttgaaagtcctacaatcctaaaataaatcacaagcttgtttgttagacgtgtcaagagtctccagtctttactactaaaaagcagcactgccttaacacacattgttatgggtgaaaagtgagggacgaccagtgtagtttctggatataaagtgtgaaggactgttgagttaaacatttttagtggaatatacatagataacgtgtatttagaaactttggtgaagccagtatttgtttttagtaacctttttatgtatttccttctttgattagcattgtcttcagtgttaagaaatgtggactcctgtgaggtgctggaggtttgaatcatcttgaaaactttccaatcttgtctagttaccactgcagagacactaaggaatttaccagaaaaagatatttgatacaagtgatttaagaaatctcaacatttcctgaggccgtatcactgggcaaccagtgatgaaaactatgaatgaattgcacacctggaagattttttaagctaatgacagtttcttcaaagatgtcaattatttgccttggaaattttataaattgcatttctatgcacatcggcctctagtgcttaccactcggtttattattcataatctgcaattcaataaaggctttgtgttttcatttatcttcaaaa

SEQ ID NO: 5 - DNA, 7973 bp, Homo sapiens
acaacgcgctccctgcggggcgggcggcaacctccatgcggcctcgtccacgctcagcaccggggaagccgaggcggagaagccgcgcgcgcctcagaagctcccggacgcccagcggcggcgcgagcggcggcggcggcagcagcagcagcagcagcacggccaccggcgggagcggcagcagcaccggcagccccggcggcgcggcctcggccccggccccggccccggccggcatgtatcgctccggggagcgcctgctgggcagccacgcgctgcccgcggagcagcgggacttcctgcccctagagacgaccaacaacaacaacaaccaccaccagcccggggcctgggcccgccgggcgggctcctcggcgtcctcgcctccctcggcgtcctcgtccccgcacccttcggccgccgtccccgccgccgatccagccgattcggcctcgggcagcagcaacaagaggaagcgcgacaacaaggccagcacgtatggactcaactacagcctgctgcagcccagcggagggcgggccgcggggggcggccgagcagacggcggcggggtcgtgtacagcgggaccccgtggaaacggaggaactacaaccagggagtcgtgggtctgcatgaagaaatcagtgatttttatgaatacatgtctccaagacctgaggaggagaagatgcggatggaggtggtgaacaggatcgagagtgtaattaaggagctctggcccagcgctgacgtccagatatttggaagttttaaaactggactttatttacctactagtgacatcgacctagtggtgtttgggaagtgggagaacctacccctctggactctggaagaagctcttcggaaacacaaagtcgcagatgaggattcggtgaaagttttagacaaagcaactgtacctattattaaattaacagattcttttactgaagtgaaagttgatatcagctttaatgtacagaatggcgtgagagcagctgacctcatcaaagattttaccaagaaatatcctgtattgccatacttggttttagtattgaaacaattcctattgcagagggaccttaatgaagtatttacaggtggaattggttcttatagtctctttttaatggcagtcagtttccttcagttacatcccagggaagatgcttgcatccccaatacaaactatggtgttctcttaatagaattttttgaattatatggacgacacttcaattatttaaagactggcatccggataaaggatggtggttcatatgtggccaaagatgaagtacagaaaaatatgctagatggctacaggccatcaatgctttatatcgaagatcctttacaaccaggtaacgatgttggaaggagttcatatggggccatgcaagtgaagcaggcctttgattatgcctacgttgttttgagtcatgctgtatcaccaatagcaaagtactatcccaacaatgaaacagaaagcatactaggtagaataattagagtaacagatgaagttgccacatatagagattggatatcaaagcagtggggcttgaagaatagacctgagccttcatgcaatggtccagtgtcgtcctcttctgccacacagtccagctctagtgatgtagattccgatgcaacaccatgcaaaaccccgaaacagctgctttgccgtccgtccactgggaaccgagtagggtcgcaagatgtatccttggagtcctctcaggcagttgggaaaatgcaaagcacccaaaccactaacacatccaacagcaccaacaaatctcagcatggatcagcaaggctctttcgttcttccagcaaaggcttccaaggtacaactcaaacaagccatggttccttgatgacaaacaaacaacatcaaggcaaatccaataatcagtattaccatggcaaaaagaggaaacacaagagggacgcgcccctctcagacctctgtagatagtcagcgctgcgcggtggactgtcttctctgtgcaatgatctcatgctcaggacagttgcgcagggactcctgggagatattcaggagcctcacactgttcagacgttgacttagcaactgcgttttttcccagctcgccacagaatggatcatgaagactgacaactgcaaaaaaaacaaaacaaaacaaaaaaaaaagcaagcaaaaaagagggaaaaaaaaggctgcttatttgataagtcatatgctacaacagggtcattttaagatttaaagcttgaatgtaaaataaatatatttctcattggctttatgcagagttatagggaatagtattcagtgttggtagggtgatagaaacaaaaaacagtatcagaggatgaggtggggaaggaaaacaaaggtatctgataggaagtccagattccaaaggggaaagtgatctgtgcatgttttttttttaaatatttttgcatatatttaccattttattgtgtgtatatatagaagaccatataggagattgatatttgtaatagtggatttgttaataatactttttacataacattactgtttaaattgtaaacagattttttctcaggattagtttgaaaaataatctaaattgtcatcttaacatccatatatagggaagtgattagttctattactcaatttgtttttctcagcattgaaatgacttaatagaacccttgtgtcctgctgcaaaaatttttcctctctaaagaaaaggtttatggtggcaaatgatgtttattttattttgtaaaaaaaaaaaaatgtactatgtacttttgtgtaaacactgaaaaatctctggtcatctccgagaattaacttgcaactgttttctatagtgctgtcgtcttgggcaatgggcaattacatgactttgtgtttgcttcctttgcagtcttttttttttccccccatttcttcctaataggaaaaaaaaaaaaaaaaaggtcacccatgtctggtctcattcctgttgcagtgaaacttcgagttccacagactttgcatgctggcttctctaaccctgtgtgctgcgtgtgcctgtttctcatctcttattctttttaaaattcatgcttaactactgtgggagaataactgtaaacagctttaattaaatcatacttataaaaaactattttcttatattccactctatgcttttggtattgttgatctttacaaattaaatggtctttgataatggatctattttgtattgccttattaagaccaaatacttcttgtcatcccattctttatcctcttctttcatggaattgttatcgttaattaaaacttttttaaacattggcttgtttcaatcatactgtaaattttggttgtagtcagctttgagtgcaatgagatgtataattctgttatcattacctgttgagtttgaaactcagttgggaatatttaatataatagaatgtaagtgacatttctgaaaatgctttctttcagggtgaaagctcttatgtttagcatcaatgtgtatggctctgttaaatgcagccatttctgagacgagattcttttatatatatatacatataaagtactattggcttttaggagtttcttttatatacatttatgaaatactgaagaccaatcagaccattaatggacacttagtgtaactttttataaagaaaataatgctaaagtaagaccaaaactgatgtcatcactgaaattaacaattttcaatatgttcatattttaattcacaatggaaaaatgtgttccaaaactggaaactcatagtactcgtgtaaactgtggaagatttcaaatgtgatgttattttgacaatgttttaaattttagagtcacattttattctgatcagaatttttattgagatgttgagcttttgtttttgaaactagtttgtcataacattgtgcataatcacagtatttattttctaggacaattgtgaatgtgtagacttatgtttactgctaagggaacaattatttataaaataatattaaatccagtattagctgcctatttcagacacttaatacttgcagagatctatgttacatttaccacactgaagttttttttgttgttttttgtttgtttttaaagaatcaccctcattgttgaaagtaaatgtactcttagggtgcgaatattagtgttccaataagcatgtgattatattaaggtggtggtagcgggaagataattctgattccattgggaatcttaggttttcgtaaatttattgggaaaatagtttttcctgtactgctgaagtttctttttggtaaacagtatctttctaaaagaaaaaagcatgaaggagaaattgaggtgtgtatacatttcctcaaatgaccagcattgtattcgtgaatactgtgtatcttgcagtgaacagtgtggaagctgttcatttttcaatctgaagtaaaatactttcaagaacttttagtttgcctgctcatttgttttatacatttcatctatttgactcctatcttatttcttttttgagttttaatacttcctatattttgtgaatatatcagaaatgtgtcatttatatattagagtccattcatatccatgaatcataaccttcctttgctaatacttgttgaatgggattttacaaattctccctcactctggtgacatttctcaggcagtcatgtatgtgtacctggccattagaaatattaatatttaaagactgttttttagaggagctgatgggttggtgaggtgtcagcacaaaatcttactggttatgttttgatgataaaagtatatccattttttccctccagctttaaggtgactgtgaaggtgcctggttttgaatgtctttgtttggtttggagatgtcgcactcagttttcaaatctagcttggatctgtaggacctatgttttttacaagtaattgccctccagtcttcaacagttgattctgttttatttttatcctgttttgagtgtactttacctttacttgcattttgagcctcattaatatttaggttatttgatttggctccagatattcctagatctgcacagggcaaaacatgggctatagggtgagcatttttaattgtctttttctgctggaaccttatatctctccatgtgttttctgctccttccctcccccatgaaatggtaagtgtgacttgtgtttgcctgaacctgtggactagtgtttggggtttctggaaacactagagggtcagaaaagagtaatgaccaccgtgacgtgcaggattctcttgctgtgacatgttcattgcaaagccctctccagtgactaggaggtgtagttattaaggttgatctgttagaaatcaccattattaggtattagtggtagatgttgctgatacttttattggtcatgactacatctcagttttactttaatattgatctatagtttgatcagttccttgaattctaatatgttgatttctcagtgtttctgtcactaaccaagaatgtttctaggcagttggttgcttcacagtcaaaactaaatggtaaactatcaaaaatacattcccaattttgctgtgataaatattgaaatgttaaaattaatgaacagaagaatttattcttacccatctattcttgttctcctagttcattaaactttcagttattggaaaggcacattctcaaagtattttatgagcaaaatattctataaatgcgtctaacaaacctaattgaatataaaagttatatttagtagttactgttgatagtaattttcatcagggtcatagttcatctagtaaaatatttagagaatgatgttaacattccagcattaaagtgggaacaaagatttatatatgaaattccttaaaagagttcatcttgccttggtttctgaccctcaagactctagctacctgccatcttgtcaaaacatttgtgggtagaataagtgttaaagatcaaattttaatatgcttctcgatatttaacatagctaagaagccagattttactgtagaagttatttacatgatttgaaaacttgacctaactggaagcctttttctcagtcatcttgttctaagccatcttgacttcacacccttagcgacttttcttttttttttggtcaaagataatgagctaaatatatatagacgttgaatgttgacaaaattattaaccagaaaaattgcttataaaggctgctgatctatttgatacctagaattaaatatttgaggacagtttttagttaataaactgctaatgtttattttactgtctctcaggtttttggtttttttaaaaaaaatgtgtttggcctttacattttctacttaagtgtgtactttattgagtttaaccttgtctgtagcctagtagcctgaaagaaaaggagacagaaccagagagatggatgtagtgcattccctttggttattacacatttgtggtagctcctggatttactgagagatattttagctatgtcaataagaacagctaatgatgtggaaatcaggtgttctcttgtgtatttcagtgaacatttttattagtagttgcatatcatctctagttccacattttaacttaacgtctttgtggcttcaccactgagctacctttcactacaccagcttctgtgtggcctggtaacatggaaggtctctcctaaggacagtctggacgtattttgggggaatgttatttatcttaaagatgcctagaaacaaaacgcatatagtaccagtgagaaactatgaagtaaacaagttgctcaggccgggcatggtggctcacgcctgtaatcccagcactttgggaggccgaagcgggaggatggcttgaggctgggagtttgagaccttcatctcttaaaaaaacaaacaaaaacctgaatggtgaggtgtggtggaattgggtaggggagggaaaggaggacttggaaaagcattctccaaagccagcaacttggtgaagttcagtacttgcctcttagaggttaggccatgcctttcaaagagagtgaaatgatgggttatcagccacattcttggagttaatatttttcttcatctttcagtttgggttctgtgctattcatagttcttccctaagaccatttcattattaccttttatatttagttgcaatttattataatatgttgttttgtccctgaacttaatctcctaattttaagatcctctctgatttttgcatattgaaacttacagaagtcactttaaaaaagtcttttgaaagtcctacaatcctaaaataaatcacaagcttgtttgttagacgtgtcaagagtctccagtctttactactaaaaagcagcactgccttaacacacattgttatgggtgaaaagtgagggacgaccagtgtagtttctggatataaagtgtgaaggactgttgagttaaacatttttagtggaatatacatagataacgtgtatttagaaactttggtgaagccagtatttgtttttagtaacctttttatgtatttccttctttgattagcattgtcttcagtgttaagaaatgtggactcctgtgaggtgctggaggtttgaatcatcttgaaaactttccaatcttgtctagttaccactgcagagacactaaggaatttaccagaaaaagatatttgatacaagtgatttaagaaatctcaacatttcctgaggccgtatcactgggcaaccagtgatgaaaactatgaatgaattgcacacctggaagattttttaagctaatgacagtttcttcaaagatgtcaattatttgccttggaaattttataaattgcatttctatgcacatcggcctctagtgcttaccactcggtttattattcataatctgcaattcaataaaggctttgtgttttcatttatcttcaaaa

SEQ ID NO: 6 - DNA, 4511 bp, Homo sapiens
gggcgcgcgggccccgcgggggcggcgcgtggatggatccgcgcgtggcctggatccagcccgagcagaaggggccggccaatgccctgtggatgcagatctgggagacctcgcagggcgtgggccgcggcggctcgggcttcgcgtcctatttctgcctcaactcgccggcgctggacacggcggccgcggcgggggcggccgggcggggcagtggcggcctgggccccgcgctgcccgccgcgtcgcccccgccgcccggccccaccgcgcccgccgcgctgccccccgcgctgctgacggcgctggggcccgcggccgagggcgcgcggcgcttgcacaagtcgccgtcgctgtcgtcctcgtcgtcgtcctcctcgtccaacgcggagtcgggcaccgagagccccggctgctcgtcgtcgtcctccagcagcgcctcgctgggccggccgggcggcggccgcggcggcgccttcttcaacttcgccgacggcgcgcccagcgcccctggcacagccaacgggcaccccgggccgcgcggccccgcgcccgccggctccccgtcgcagcaccagttccacccgggtcgccggaaacgcgagaacaaggccagcacctacggcctcaactacctgctgtccggcagccgcgcggccgctctcagcggagggggcggccccggggcccaggcgccgcggcccggcaccccgtggaagagccgcgcgtacagcccgggcatccagggactacatgaggaaataattgacttttataacttcatgtccccttgtcctgaagaagcagctatgagaagagaggtggtgaaacggatcgaaactgtggtgaaagacctttggccgacggctgatgtacagatatttggcagctttagtacaggtctttatcttccaactagcgacatagacctggtggtcttcgggaaatgggagcgtcctcctttacagctgctggagcaagccctgcggaagcacaacgtggctgagccgtgttccatcaaagtccttgacaaggctacggtaccaataataaagctcacagatcaggagactgaagtgaaagttgacatcagctttaacatggagacgggcgtccgggcagcggagttcatcaagaattacatgaagaaatattcattgctgccttacttgattttagtattgaaacagttccttctgcagagggacctgaatgaagtttttacaggtggaattagctcatacagcctaattttaatggccattagctttctacagttgcatccaagaattgatgcccggagagctgatgaaaaccttggaatgcttcttgtagaattttttgaactctatgggagaaattttaattacttgaaaaccggtattagaatcaaagaaggaggtgcctatatcgccaaagaggagatcatgaaagccatgaccagcgggtacagaccgtcgatgctgtgcattgaggaccccctgctgccagggaatgacgttggccggagctcctatggcgccatgcaggtgaagcaggtcttcgattatgcctacatagtgctcagccatgctgtgtcaccgctggccaggtcctatccaaacagagacgccgaaagtactttaggaagaatcatcaaagtaactcaggaggtgattgactaccggaggtggatcaaagagaagtggggcagcaaagcccacccgtcgccaggcatggacagcaggatcaagatcaaagagcgaatagccacatgcaatggggagcagacgcagaaccgagagcccgagtctccctatggccagcgcttgactttgtcgctgtccagcccccagctcctgtcttcaggctcctcggcctcttctgtgtcttcactttctgggagtgacgttgattcagacacaccgccctgcacaacgcccagtgtttaccagttcagtctgcaagcgccagctcctctcatggccggcttacccaccgccttgccaatgcccagtggcaaacctcagcccaccacttccagaacactgatcatgacaaccaacaatcagaccaggtttactatacctccaccgaccctaggggttgctcctgttccttgcagacaagctggtgtagaaggaactgcgtctttgaaagccgtccaccacatgtcttccccggccattccctcagcgtcccccaacccgctctcgagccctcatctgtatcataagcagcacaacggcatgaaactgtccatgaagggctctcacggccacacccaaggcggcggctacagctctgtgggtagcggaggtgtgcggccccctgtgggcaacaggggacaccaccagtataaccgcaccggctggaggaggaaaaaacacacacacacacgggacagtctgcccgtgagcctcagcagataatggctcctggctgcgtcagcctcccccacccctctgcagactgccccgcggcctcggccaccggcaggggaaccgagaccagcaccccgcacgtcagccgggctcgcggcacgcccgccgctgatcactctgcatgtttcttcgtgtggtggtcgcgtccatcttcaagaacagctcgttgtgctcatctgtgaagccttattaaacgtggacgttgttttctgccttcccaggattcttccttcagtgctgaggcaggtcgggctcaggaactgcagggacgtgaacatgcgcttgcggtttgaggtagccgtgtctgttccttcgcggtttgctattttcatttcctgttcgtcaaagcagcagaggagatcaaaccccgttcgtgtgtctttcctccacggataagcttgggaggtcattgttttactgccctcacattttgtttgaaatttcagaactgtttttctatgtaaatattgaaaacttatgatttgtgcaataactcagatattttttatttaatttcctattttcacataagttatatttaagggaggagggaattttttttaaacaagcttaggtcctttcccgagctgcattttctaagttgggtcatcgtgtcggctggttgtctgacgagcatcgttacaaacaccatgatgaggggtttggggttttattttgatgtcttttcttttggtcggaagtgagtgaaggagccaggtcgccctgaaggttttccaaagggcttggctccagagccacctggcagactgcccgtggccctgctgtcgggccccaggccgttgtcctgctctgaccacagagttttaatgttttggttttcacttcttttaaactggacaacaaatccagcatttcaagtgccagaagtataactttctaaggagagaagggttgtcacattataaaatctttaggaaaatgtgaactggaaaacgcttcggtcagttttagtgacatagcctgtgatgatgggtctggtgactattattgcggaccgtggtacccagttttaggaatgtggagaaaggaattctgttgattccgttgaggaatctgtagcgtatgcattcgttctgttaagagcaaatctaggagaagtgcttcagctgcccagtgcgccgtggggagtgttttaacggatcgtgtcgcaggagagcacagcccagcgttggggccgggaccgctggcgcccgacgtcggaagcatacaggtatactatgcaagtgtattctgccacaacaaccactgtctttgttacctttttttgaacaagaatatatccatcctgcctaaccctgagtttttggagcaccacagttgtcctgggagttggttgcatcttgtaggccatctgacttcctgtttttaaaacgggggtctggtcttgctaaacactacaggtaggttggtctttgaagtccactagtggagaatgtcaagacaagatacttattaccatgacatctgatgcatgtgcagcagtggggagttctagattgatctctgaatgtgatcgacgcccagcaaggacaagctttaaaatgtctgcggtctgcccttttgaagcaggactggctcactctgtcattgggagctgtcagctgcgactgcaggttctctaggaggcattccagaatagagtagcacactgtgtctgcagttctcgatgaccgaaagttatcaaaaatatttaaaatatttaaattgtgaacctattgataaagaatatttataaaaactgatctgtaggcctgtactaatctctacgcattagcaatattgactgtaaacccacattaaggaaaccactacgggtctggcagtgcgtgtcccgtggggtgtgcattttaaaactcgattcatagacacaggtaccatgttccatttccgtcatggtgaagcaaatgaattggcctggctaccactgtggtcgcgtgctacaggtttgacaaaaagatatcatgtttcgatttttttgtgtgtggacaacaatatggaagctaaaattgacatatttttatgtaaagtttttctattctttgatttttaataaactttggaaaccag

SEQ ID NO: 7 - protein, 474 aa, Homo sapiens
TYGLNYSLLQPSGGRAAGGGRADGGGVVYSGTPWKRRNYNQGVVGLHEEISDFYEYMSPRPEEEKMRMEVVNRIESVIKELWPSADVQIFGSFKTGLYLPTSDIDLVVFGKWENLPLWTLEEALRKHKVADEDSVKVLDKATVPIIKLTDSFTEVKVDISFNVQNGVRAADLIKDFTKKYPVLPYLVLVLKQFLLQRDLNEVFTGGIGSYSLFLMAVSFLQLHPREDACIPNTNYGVLLIEFFELYGRHFNYLKTGIRIKDGGSYVAKDEVQKNMLDGYRPSMLYIEDPLQPGNDVGRSSYGAMQVKQAFDYAYVVLSHAVSPIAKYYPNNETESILGRIIRVTDEVATYRDWISKQWGLKNRPEPSCNGNGVTLIVDTQQLDKCNNNLSEENEALGKCRSKTSESLSKHSSNSSSGPVSSSSATQSSSSDVDSDATPCKTPKQLLCRPSTGNRVGSQDVSLESSQAVGKMQST

SEQ ID NO: 8 - protein, 419 aa, Homo sapiens
LLQPSGGRAAGGGRADGGGVVYSGTPWKRRNYNQGVVGLHEEISDFYEYMSPRPEEEKMRMEVVNRIESVIKELWPSADVQIFGSFKTGLYLPTSDIDLVVFGKWENLPLWTLEEALRKHKVADEDSVKVLDKATVPIIKLTDSFTEVKVDISFNVQNGVRAADLIKDFTKKYPVLPYLVLVLKQFLLQRDLNEVFTGGIGSYSLFLMAVSFLQLHPREDACIPNTNYGVLLIEFFELYGRHFNYLKTGIRIKDGGSYVAKDEVQKNMLDGYRPSMLYIEDPLQPGNDVGRSSYGAMQVKQAFDYAYVVLSHAVSPIAKYYPNNETESILGRIIRVTDEVATYRDWISKQWGLKNRPEPSCNGPVSSSSATQSSSSDVDSDATPCKTPKQLLCRPSTGNRVGSQDVSLESSQAVGKMQS

SEQ ID NO: 9 - protein, 320 aa, Homo sapiens
YSPGIQGLHEEIIDFYNFMSPCPEEAAMRREVVKRIETVVKDLWPTADVQIFGSFSTGLYLPTSDIDLVVFGKWERPPLQLLEQALRKHNVAEPCSIKVLDKATVPIIKLTDQETEVKVDISFNMETGVRAAEFIKNYMKKYSLLPYLILVLKQFLLQRDLNEVFTGGISSYSLILMAISFLQLHPRIDARRADENLGMLLVEFFELYGRNFNYLKTGIRIKEGGAYIAKEEIMKAMTSGYRPSMLCIEDPLLPGNDVGRSSYGAMQVKQVFDYAYIVLSHAVSPLARSYPNRDAESTLGRIIKVTQEVIDYRRWIKEKW

SEQ ID NO: 10 - DNA, 82393 bp, homo sapiens
acaacgcgctccctgcggggcgggcggcaacctccatgcggcctcgtccacgctcagcaccggggaagccgaggcggagaagccgcgcgcgcctcagaagctcccggacgcccaggtacgtgggagcactccacagatggcgcaagtacggttgggccaggcggttgcggccccgtcgcgccgcggcctctgtgacgcacggcgaggcctcccgggctgctgcgcggcgcagcgggggcggggcgagcgcgtgagggcggggcggtggggggggggggcggagcgagaggggcggagccggcagaggccccgccccggggccggaggagcgaggacgctacggagcaggcgcgtctcgctgccgccgctgccgccgccgccgctcgctcttctgtggagccgccgccgccgccgccgccatttgcacggggaccccagtgacaggggctcggcggaggggcggaggggcggagggagggggggagggcccgcggagcccccgagggcgggagcgacgccgccggcgccggccgggctccctgcgcgaccgcgccgcccgcggcgggccccgagcagcagcagcagcagcagcggcagcagcggcagcagcagcagcagccgaggccgggcgtgcgcctgaggcggcggcggcggcggccctgcgggcggccgggaggggcgggggcagcggccgccgccgtttgatggatccgaggatcgcctggtttcagccagagcagctcggaccgtccaacagtctgtggatgcagatctgggagacgacccaggggctgaggaacctctacttcaaccaccactgtcacagcagcggcggcgcgagcggcggcggcggcagcagcagcagcagcagcacggccaccggcgggagcggcagcagcaccggcagccccggcggcgcggcctcggccccggccccggccccggccggcatgtatcgctccggggagcgcctgctgggcagccacgcgctgcccgcggagcagcgggacttcctgcccctagagacgaccaacaacaacaacaaccaccaccagcccggggcctgggcccgccgggcgggctcctcggcgtcctcgcctccctcggcgtcctcgtccccgcacccttcggccgccgtccccgccgccgatccagccgattcggcctcgggcagcagcaacaagaggaagcgcgacaacaaggccagcacgtatggactcaactacagcctgctgcagcccagcggagggcgggccgcggggggcggccgagcagacggcggcggggtcgtgtacagcgggaccccgtggaaacggaggaactacaaccagggagtcgtggggtgagtgctggctctgcggcccgatggcctggccggtgcgaatgcgcagccgggcacacgcccacagaggggggttgtgagggtctaggagcggccacccccacggcctgccttcgctgctgttgcacgggggtgctgctggccatccccaaccccccagtcgttcacacctttccccaagcctccttagccgtccacaccctccgtctcctgtcctcccttagtcgtccacaccttcctcccctccctcttaaccgtccacaccttccccaggcccccccctttatccattcactctcctcccatcccccttagttaaacacatctacccttgaccaccaccccgcctccagccctccacacctttttccccatcatcacaactcaagatgagaccgcttagcacgggcctatcattcattccctgagaacattggtgtgtgagtgttttttgatggtgcaggacccggaggtgctttccttgccaagaatagaaacatccagaatgctcctccccatcccccaatcccagacagcaattatgtcagccctgtaaggcattgcctgctcttgaccctttggcccatctttttatttttaaaaaattcccatgtcacagatgccctgtctatgcagagggtggcgtgggatgggtgaccactaagtttaggctggtgaaggtggtgagcccttctgaggccctgatagaactttccaggagttcatggtccgcggctccagcttctcactgtaaagttgtcatcctggcagaggcagccaatgcttttcattctagggggtagagatttatgctaatgagtgaatattgcaccactagtgactttctgtttaaagttcagctcttagaaaatggaatcttacctgacccctagtgaattatgtacataagcagggaatgtttccaactagatctcccttcagaagagtccctgtgctggaataggtcactgaatcttatttgttttgtaaaacaaagcttttgggtctcgtgggtgtgtgtgtgtgtgtgtgtgtgtgtgtgtgtgtgtgtgtagcttgagtatggagaaccggctttcaaattgcttttcatttttcaggttgtgttttacattgagggctttagcatgcaaatgaaattaccaattagtaatcccatgtgaaccttttcctggatttattcattcagatctgccctgctttggctgagagagagagttctgtgtacctttttgaaggtctggataaaatgagttggtgggttccatctgcttccagtgggctggtgtctgctctatgctactattacaactcctaccttttgtggaaaatgcagtcaagcgttctaggactggtgctgtggtacatgtcaaacctgccctcacattccagaaagggaacccttttagggttgagtcctctgttgctaagcttcaagggtgctctccatggtcatcacgttttattaaaggcttgtggttccatcctgttagcatttccaagtctacgcgtaaacctgtggtttagtgacaagcaaattgatgttgagggtttctggtagtttcatttcacaggagtaagctccagttaggtaatcactgtcaacgaaaaccttgaagttccttaattgcattttactgaagcctctttgcatgtgtctagcaaaagatataagtccaagatgcttattttttttttgataaattagaaattgtcctctcctctacttgctatttaatgcagaagatactctaaaaggttcatatttatacttagaagcaagatgttcttgttcctgattcaaatatattgccctcaaagggattaggagaggaattttcatttcccggagggattactgtttaaaaactggttgtaaacctctttaaaaactgcttatcacttcaccagattttccattcttttgcctcctcccttagaggatgtcagcagttaattttttttttaaattaaaaaaagttcaattctgagacctcctagtttcaaaaaatacattaaacaattcccaagagtgttaagagtgtctgggtgcttagaaattcttgctttgattcatgtattctgattttttttttttttttgagacggagtttcgctcttgttgcccaggctggagtgcagtggctcgatctcagctcaccgcaacctctgcctcccaggttcaagcgattctgctgcctcagcctcccgagtagctgggattacaggcgcttgccaccacgcctggctaattttttatttttagtagagacggggtttcttcatgttggtcaggctggtctcgaactcctgacctcaggtgatctgcccgtcttggcctcccaaaggactgggattacaggcatgagccaccgtgcccggcctcattatcctgatttcttttttttcttttgagactgggtctcactctgctgcctaggctggagtggagtgacgtgatcatagctcactgtatcctctaactcttgggctcaagtgatcctcctgccttagcttcctggagtagctgggactacaggcacatgtcaccacacctgcctaatttttttatttttactttttgtagagatggggcctccatttgttgcctaggctggtcttcaaccggcctcaagcagtcctcccaccttggcctcacagagtgctgggattataggcatgagccaccattctcgccagtatccttatttcttaactttagaaagtttttctatttttaatataggtatttaaaaaaatctgaattcagagtgcacctcgatgttatgctgttctgagattaaatatactaaaactgttaccattgttttctgaattcttaagatgtgactgatagttagctaataggttaacacattgtggtggttcttggcctctgaactgatagtccagatggggagaggagaccagaaagcatgtgaaaatggactagaaccatgggacagctatatagtctctcgcagctgtcttttgtgttctctgcttccaccaaattggttgatttatttagaatgctgacctcttgcattgcctaagtccttgatgtttttggtttctcctctgaactctcaaaggtactcacttcatgctcttggtatagcccacttatgtttaactttccttttattatgtgttccctcttacacatgacatggacatttctttaatatgtagagtaagatattggatttcatcctaaagtcttcaaaataaaactcttgagctcatcatctcagacttcttcatgtacccacagaccagggattttgtttgctttttaaaacatttttttattttgtgttttattatttttaaattttaatttaattttatggagacagggtctcgctctgttgcccaggctggagtgcagtggtgtgatctcggctcactgcagcctttgcctgggctcaagccatccacatgccttggcctcccagtgtgctgggattacaggtgtgagccactgtgcctggcctaaatttatttttttaattttttttgagacagggtcttgctctgtcgctcaggctggagtgcagtgtcataatcatgggtcacagcagccttggcctcccaggctgaagtgaacttcccacctcagcctcctgagtagttgggactacaggcgagtgccaccatgcctggctcattttggttttttttgtaaagatggggtcttgtcatgttgcccatgaaggtctccaactcctggtccaagtgatcctcccgcctccgcctagcaaaatgttgggattacaggtgtgagccaccatgcctggccttatttatttatttaattatgaatgaatgaatgaattaatgagagggagtcttgctctcttgcccaggctggagtgtggtggcacaatcttggcccactgcaacctccgtctcccaggttcgagcaattctcctgcctcagcctcccgagtaactgggattacaggcgcccgccaccatgcccaggtaatttttgtatttttagtagagatggggtctcaccatgttggccagactggtttcgaacttctgacctcaagtgatctgcccaccttggcttcccaaagtgtcaggattacaggcatgagccaccatgcctggcctggccttttatgttttaagttgcttccactgattctcttgggctttgctcccctccagaactggccatggtttaggatgctgtccacctgctgctgcttgtccatgaaaacgagccataaacccttttcttttgaaagacttaattgtttatcactatggagaaagaggggatggcaagaagtagcaaatacagggaatttgcagaacttggtcttgagccctgggtccagaaacttcttctggaaggtgcttggtgtttgtccaagctcatgataggtttctgttggctgtactgccagatctgtagatgcttttttaaggcttggatgacttgttcaaaacaatgttttggagtacaaatttggctgtggggacatcaagaccttgttgggaaacttgggtttaaggtacaatttcttaaactaggatggtgggaatggggatgtgaagggagaatgaatgtgagaggtattacagggtaaggatggagatgattcagattccttaagtggatttaataatcacactgtagctttgaacttgagtgactggggaaatatttgtggtgtttttggaaataagggccagaaggactattggtttgggtaagaagatagtagggggatgtataggtggacctgctagtggggagctgagatttggagggctgagatgtagtgctcttcactgccgtagggcagtatcctcttgtatgtgccatcctctagtgcccattgttcatcatgtcatagtaagcccaagatgttcatgccttttttcagcactgcattagggcttatatctgcttctctttctctctctctctcgctctcgctccctccctctctctctctttctgttttttttttttttttagacggagtttcacttgtgttgcccaggttggagtgcagtggcgcgatcttggctcattgcaacctctgactcccgggttcaagcaattctcctgcctcagcctcccaagtagctgggattacaggcatgtgccaccatgcctaattttgtatctttagtagagatggggtttctccatgttggtcaggctggtgtcaaactcccaacatcaggtgatctacctgcctcggccgcccaaagtgctgggattacaggcatgagccaccgcgcccggcctctctctgcttatttctacacagtgttaccaatgagattggtgttactgctgggctccaaagcaatcagacagattaaagtagattgaatatgaaagaatttagaggcctttttccaagtgatttgtgctctatttaatttctgtgcatttgcagatatagcccacagtaattcttagtgaactagaaccttcaggttattgaattttactgatttgggtactgacatgcgcttttaagaagacattaggttttctatagtgtagattgtacactaacaatataattcatatttaagaatgtctcaaaatttagtatactgtgttcaactaacttaactttctttgttttttttgttttgttttgtttttgttttttgagacggagtcttgctatgccacccaggctggagtgcagtggcgtgatcttggcttactgcaacttcaacactcctgggttcaagtgattttcctgcctcagcctcctgagtagctgggattacaggcacccgccaccacaccggctaatttttgtatttttagtagagacggggtttcgccgtgttggccaggctggtcttggactcctgactcaaatgatctgcctgccttggcctcccacagtgctaggattacagacatgagccactgcgcccggccgctaacttaactttcattccacaacttccatcttttatccaaaatctgtgatcattgaatactgtcaccattaatcattggcatttcagtgtttggactttttttttcccccttcgtctttgtggactcttttttaacactcataaagttttaactattgaaaagcaaaggaaacggtgagtgactttttggagtctgtctacccagtggtcacacaaaaggcttactacattacaggaaagataggatgggaaagggatactagaaaattctaagtcaggaacgggggtgtgtattagaaaaattctgatcctggcatgccagatggccttacatctcaatttcttccgtgaaattcctgccaacaaatcatagtgttagaagtacagaagggtccatgggaacagaatttaagggctccgttggtgatacggaactgatcagatggttctcacttgttctcagataacctgtatactgaatatcacaggaagggtatagacgtcatggcagtggttagatattcttgcacctgctgaagctgagaaaattaaagtaattttttttcctgtggaaagtagaaaatcaagcttttgtatgatttcacacagctttctattctctcttttgttgactctgttaagagtaacatttagtggtggaaactatttcaggatcacacccacaacactagagactgtattaatcacttacacacacataggtatagagtaatcttgaaggggctgtaggccaaagataatgcttttttgaagaattagagactagttaccagcacctggtatttgctgtttcctacagagctgactggacagcctagagtctgctgaggaattcagaggatggccagtagaatgttctttccaccccagaatatttggtagggactcagctgctgtggaatgccaaaaaggctttgagtttgtttcactattcttaagattacacgtaattgtttttttgtaagagattatatatattcaagttgaggatggctttgagttagactttccttaatttggaatcacacagcagatgatacatttatttccatctgataagttacttgatgatgtaaaaagacatttgagttaaagatttttgggaaaaaagctgaatgttgagccatttatgttgtgtactggttccctattcacttggacaattttaagtcttaaaacaatcttaaccatgtgcacaagagatttcacatagtatttggtaattaaattaaggaattctagctcaagtcatgctttttgctgaaatagttgtatatatttagtgcggaaacctgtgttttcaaattaatgtaataaaagtttcaataaaatggaagcctttattaccgtgtttcaaatgctatgctaaaccttttccatttgttattatattaacctcctcatacatagccctactaatttttttactttctattttgaaataattacagatttataggaagttgtgaaaaatagtacagagcccatgttcccttcaccaagtttcacctaatggtagtagctcacataacgataatttaatgtcaagaaccaggaaattgtcatcgttgcaatccataagccttttttagatttcaccagtttcacatgtatttgtgtgtgtgtgtatatatataattgtatgcaattttatcatgtgtagatctggatagccactgtaacagtctatagttctatatacagagctactccatcacctcagggctccctatgctaccactttatagccgcacgcacccttccagcaaccactaatctgtttgcatctctgtaattttgccattttgagaatgttatataaatggaatcatacagaatgtaactttggctttttttcttttaccatacttcctttgagagccatccaaattgctgcatgtatcagtagttcatttctttttactattgagtagtagtccatagtatggctgaaccacacaatttgtttaaccatttacttattgaaggacataccagaagggtggtttccagttttttggctattgcaaataaagctgctataaacattcatgtatataaatatttttatgtgaatataaagttttcattttgggggaataaatgcccaaatgtttggattgtatggtaagtgcatgtttggtttttagagaaactgctgaactatttattttctagaatgactatatcctcttatattcctatcaacaatatatgagatatccagtttctctgcatccttgctagcatttagtgttaccacttttttatttgagcggttctaatatgtgtagtgatagcctgttttgccttatattaatcaataaaaatagcctcatctaatcttaactttttttattttaaaacatcttggcagtattgaactttctcaatgaaaaatctctaaaattgtgacttgaaaggctttaattttccagtttttctttggttttactcttagcagtaacattttaacttttttttgtctttgaagtaattttcagtgtttcctttacatgttgctttttcttagaaactagttactagcatgaagtagatctttagcctcgttttctaaaaacataaaaaagtaaaactgtggggtttatttcaaaattgagagtcctgtcttttcatatgaggatattttatagtctgttggcttggctatattttagggagtaaacctgtggttagtggtttgttgttggtggtggtaaagttttcttacagtatttttatacctgaataatacctttagactctatagaatagatacttgatcttcaaatctatcctagaataaattgttttatctaaacagctttgtgacctgagaattgggacttagtcccttagttttcccttactggccctttgtagtcactgttttgattttgtgaaagtaacttaactcttagcactgtcaggtattgtacattcctgccaaagcaagaataagaatacataggattgtgttttaattctataattaggtgacttttggctaatttccaggaacttggacttaataaagtactagtgataagtttggaaattttagtgtccttgttctttgaagttattcaccctttactttcttgtttgtttggggtgtttatactactgtccctaaatatagctgaaataaaggaagaaaaataacccctgtaatatcactaccaggatataatttcttttttttttttttttttgagatggagtctcgctctgtcgcccaccatctcggctcactgcaagctctgcctcctgggttcacgccattctcctgcctcatcctcccgagtagctgggactacaggcgcccgccaccacacccggcttattttttgtatttttagtagagacggggtttcactgtgttagccaggatggtcttgatctcctgatcttgtgatccacctgcctcggcctcccaaagtactgggattacaggcatgagccaccgcgcccggcctgatataatttctgttaacagtttgatgtaaatattttttgactttttagtgtttttatatatatatatattttatgtttttcttttatcaatacgcactcttactgtgggaataattttaatgtttttaaagagttgggttttatttgtttattttattttatagaaatggggtctcgccgggtgcgatggctcacgcctgtaatcccagtactttgggaggccaaggcaggagcatcacctgaggtcgggagttcgagaccagcctgaccaacatggataaaccgcctctctactaaaaatacaaaattagccgggcgtggtggcacgtgcctgtaattccagctacttgggaggctgaggcaggagaatcacttgaacccggccggtggaggttgcagtgagcaaagattgtgccattgcactccatcctgggcagcaagagtgaaacttcatctcaaaaaaaataaaaaataaaaaagaaagaaagaaagaaatgggatctcaccattttggctggttttgaacttgtggtctcaagcagtcttcctacctcagcatcccaaagtattgggattacaggtgtgagcccatcctgtttgttgttgttcttttgttgttgttgtttttagatgaagtctccctctgtcacccaggctggagtgcagtggcgctatcttggctcactgcaagccccgccacccaagttcaagcaattttctgcctcagcctcccgagtagctgggattacaggcgcccaccaccatacctggctaatttttgtatttttagtggagacgaggtttcaccatattggccaggctagtcttgagctcctgacctcgtgatccacctgcctcggcctcccaaagtgctgggattacaggtgtgagccactgcgcctggcctgttgttgtttaaataaaagaaatttattctcttacagtcgaggccagaacttagaactggttttcaatctaaattttttttcttctttgggagaagggcatcagaatattgtggatatacttttttgacttaaaaaaaaaggttttactgggctgggcatggtggctcacctgggattaactgcctgtaaccttggcactttgggaggctgaggcaggtggatcgcttgagtccaggagttcaagagcagcttgggtgacatggtgaaactccgtctctaccaaaaaaaaaaaattagccaggcatggtgatggcgtgcccttgaagtcccagctacttgggaggcttagctgggaggatcgcttgagaccaagaggcagaggttgcagtgagctaagttcatgccactgcactccagcctgggtgacagagcgagacctcgtctgaaaaatttttttttttttttactaatatgacaaacatcttttcatttcaaatatatttctataccatttttaatatctcattgcctttagaatgaccttgtattcatagtacatatgtatgtgatattccatttatttattttttttcttttgtctttttttggttatattccattgatttaatgtaccttaatttatcttaccaatttcttgttgaccattttgtttccagtcttttgtttttttaccagacatggattaagctgagcctttgccccagacgacattatttcttttttatcagcaaaatatgcgtgtaatgaaattagaattaaaaggcaaaaaaggttatcctttatttttctacttatttttattgagatagtaattcacataccataaatttaacccttttaaagtgtacagttcagtggttttcatatattagaaggttgtacaaccatcgcaactaattccagaacattttcatcaccccagaaagaaactctgaacccattatcactccccactccctcacacaccctaaccctggcagtcacatatagactctctgtctctgtggatttgtttactctggacctttcatataagtggaatcataacagtttgtggccttttgtgcttggcttctcaaacttatctgtttccaaaggttatctgtgtcgtagcatgtgtcagtacttcattcctttttatggctgaatattttattgcatgtatatgccacattttgtttatccattcacctgtagaaggacatttaggttgtttccattttttggctgttatgaatattactgctgtagacgttcatgtacaagtttttatgtgaacgtgttttcatttttcttgggtatatacttaagtgaggaattcctgggtcttaagttaactctctgtttaacattttgaggaactgccaaattattttttaaagtggctgtgacattttatattctaccagcagtgaatgaaatttccaatttctccacatacttgacagcacttttttttttttttttttttgaggtgaagtcttgctttattgcccaggctggagtgcagtagcatgatcttggctcactgcaacctccacctcccaggttcaagcaattcttgtatctctcagcctcccgagtagctgggattacaggcgcatgtcaccatgcctggctaatttttgtattttttatagagacagggttttgccatgttggtcaggctggtcttgaactcctgatttcaagtgatccacctgccttagcctcccagagttctgggattacaggcgtgagccactgcacccagtctgcactttctttattatctgtcttctttattatagccaatctagtgggtatgaagtaagtgtgtcatttgtgattttgattgttagtggtgactaaaaatgttgaatatctttacatgagcttgttggccatgtgcacatctttgttggagaaatatctattcaaatcttttgactattttaaaattgggttatttatctttttattgttgagctataggagttctttattttattttactgagacagggtcttgctctgtcacctaggctggagtgtagtgatgccatcttgactcactgcaacctctgcccccaccccaggctcaagtgatcctcccacctcagtcagcatcccacagctgggaccacaggcgcatgccaccatgcctggctaattttttttttttttttttttttgtattttagtatagacagagtctcaccttattgcccaggctggtctcaaactcctgagctgaagcaatccgcccatctcagcttcccaaagtgctggaattagaggcatgagccactgtgcctggcctattttattttaaagatgaggcctcactttgtcacccaggttggagtgcagtggcgtgatcatagttcactgccattttgccctcctgggctcaaacagtactcacgactcatcttcctgagtagctaggactgcaggcatgtcgctagcatgcccagctaaaacagttctttatattctagatcggggtgtccaatcttttgacttccctgggccacattagaagaagaagaattgtcttgggccacacataaaatacactaacagtaatgacagctgatgagctaaaaaaagaattaccaaaacatctcataatgttttaagaaagtttacaagtttatgttgggccacattcaaagccatcgtgggcctctggccgtgggttggatgagcttgttctaaatgctagacccttatcagatggatggtttgtagatatttatcgcatgctgtgggttttttttttttactttcttttaggtttttttttttcttaaataattaaactgattaaaagctttaatcttttcattttcttgataatgtcttttaaagcacaaagttttgtttcaatgatgtctaatttgtctatttttttttctttggttgcttgtcatacgtaagaaactgttgctaaatccagaatgctgaagatttacttgtgaactttgtttccttctatgagttttatagttttagctcttgtatttaggtctttgatacattttgaggtttttttgttgttgttgagacagtcttgctctgtcgcccaggctggagtgcagtggtgtgatcttggcttactgcaccctctgcctcctcggttcaagcaattctcatgcttcagcacccgagtagctcggattacaggcgtgcaccaccaagcctggctaatttttgtatttttagtaaagagggggcttcaccatgtttgtcaggttggtcttgaactcctgggctcaagcaatcctctcatctcggcctccccaagtgctgggattacaggcatgagccaccacgcccagcctgttttgagttcatttttaaaatatggtgtgaggtagaggtcccatttcattcctttgcctgtgggtatccagttgtcccagaaccatttgttgaaatgactcttgtttcctcattgagcaatgtcgtgagaccctatctccataaaaaataattaaaaaaaaaaaagaatgcagaaggaaacagttttgccaattttgtagtatttactgacaatttgcatatgtctttacattctttagctatttatttttcttttgaattactgcctttgttcatttttcttttggagttgtttgtctttttcttattaatttgtaagagattttgcaaatatatacaatttcttttctcttttttttgagatggagttttgctcttcttgcccaggctggagtgcagtggcatgatcttggcttactgcagcctctgcctcctggtttcaagagattcttctgcctcagcttcctgagtagctgggattacaggtgcccaccaccacacccagctaattttttttttttttttttgtatttttagtagagactcggtttcatcatgttggccagactggtctcaaactcctcacctcagttgatccacccaccttggcctcccaaagtgctgggattacagttgtgagccaccgtgcctggacctcccacattattttgaaacaaattccatatcacataatttcttttttttgagacagagtctcgctctgtcacccaggctggaatgctgtggcgtgacctgtgcttactgtaccttctgcctcctaggttcaagcgattctcctgcctcagtctcctgagtagctgggattacaggcacgcaccaccacacctggctagtttttgtatttttagtagagatggggtttcaacatgttggccaggctggtcttgaactcctggcctcaggtggtccgtccacttcggcctcccaaagtgctgggattacaggcttgagccactgcacccagccaatatcatataatttcatataaatagttctttgtgtatctttagataaggacttaaaagaaggcataatcgtaacaccattattaatacctaaaagaagtgagcaataaataattcatttgccgtatcaaatatccaatgttcatatttcctccattgtcccataataatttttaaaagtttgctcaaatcaaaatccaaacaagattatttcaaagcattgtttgaggtacattttaaatcttaatttatagatttctctgctgtctcttttcccccatatttatttgttgaagaaaccaagcgttgtttcctgtggactttcctactctctggattttgctggttatattcctctggtatcagtttactatgatccctttttcccctgtattttctgtaaatttgtaactagatctagagatttgtttagattttgtgggttttttttttttttttttttttttttgcaaaaatgcatcataaatggtggtgtgtacatctctcagaagacacatatcttaatgtctttttgtggtattagttattaatgattactgcctatatttattaattcattatttggattgtaagtttatgatagtctcttgatgctttttctgttgttagctggaatgcttctaaaaggagaaggctttcctcttcaagctacttggttgtcttgagggtttgcttcttatagggaaagcaggctaagggtgaaaaaggaaatagtttctaactgggtctgttaatgagctgtcaccccaggcaaagagaagcaaggcaggtcacaggaaagtgaagtgggcttgggatgattggtgccccatgcgtgcatgcatgaagggaagttaatcctccctgtagtgaactctactgggcttttggtcagtagccaagactgtcaaggaagacctttgtcagaagccatacctggcctttgcttttagctgttggtagctgaaggaaaccagaacagacctatgacctgtgaacttctgctcagtagacaaagttctctcagcctaaattcagtaagcaggagtaagatgcttgctttcccttgaagtgaaacgtgaattatatgtttcttcaacttgtgctaatattctttttttttttgagatggagtctcacactgtctcccaggctggagtgcagtggtgcaatctccgctcactgcaacctcagcctcccgagtagctgggattacaggcgcctgccaccacgcctggctaattttttgtatttttagcagagatggggtttcactatgttggccaggctggacttgaactcctgacctcacgatctgcctgcctcggtctcccaaagtgctgggattacaggcgtgagccaccacacctgggcaacttgtgctaatattcttaaccttcatgtgaatcattcctgccctcaggctagcataacccatacagccttccttataggaagatttcctactgggagtgaatttgtccagtgattcccccaagatatcccccaatcaaatattttaaaagtcatcatttacatgtaaaaactatgtaacaagcatggtagcagcagcgttaaagaaatggcagtatggcccctgtaagggaaggctccagaagatgagccgcactcagcctctaggtcacagctaccttaggagtttgcagttgttcctggggaagtcagtagacaaagctatctctcaggcctgggcaagatagggattttttttttttctttgagatggagtctcaccctgtcatccaggctggagtgcagcagcatgatctcggttcaccacaacctccacctcctgggttcaagtgattttactgcctcagcctcctgagtagctgggactacaggtgcgggccatcatgcctggctcatttttgtatttttagtagagatggggtttcaccatgttggctaggctagtctcaaactcctgacctcaggtgatccacctgcctcccagagtgctgggattataggcatgagccactgtgcccagtgtttttttttttttaattgtagtgacaggatctcactttgtttcctgggctattcccaaactccaggcctcaagccgtcctcctaccttagcctcccagagtgctggggttacaggtttgacccactgtgcctagtctcagaattcatgtttttaaaagtcactctgtgccaggctcatgcctgtaatcctaatactttgggaggctgaggcaggagggttgcttgagcccaggagtttgagaccagcctggaaaccatagcaaaatcctaactctacaaaaaatacaaaaaatagccaggtgtggtggcatgcacctgtagtcccggttacttgggaggctgaagtgcaaggatcgcttgagcctaggaagttgaggctgcagtgagctgtgatcatgccactgcacaacagcctgggcaacagagtgagaagtaactctggctgtggtggggaaagtggattagtggagaatggaagctgggaaacatggtggttcttgctaagtcagtatcaagggatcacagatgagggggctatttcgtcctaataagggccttggtctcccagatagtcatggatttttctatttagaagctccttctcagtttttcttgcccaaggcatatacggttgatatttgtacaacacaggctggatctgtatgggtccacttatatgtggattttttttcaaccaaacttggattaaaaatatagttgtaggccaggcacagtgacttatgcctgtaagcctagcactttgggagcccaaggcaggcggatcagctgaggtcaggagtttgagaccagcctggccaatgtggtgaaaccatgtgcctactaaaaatacaaaaaatagctgggtgtggtggtgtgcacttgtaatcccagctactcaggaggctgaagccagagaattgcttgaacccgggaggtggaggttgcagtgagctaacgcagcagaggttgcagtgagctaacgcagcagaggttgcagtgagccaacggggtggaggttgcagtgagccaagattgcaccaccacactctagcctgtgtgacagagcaagactctgtctcaaaaataaataaataaaaatacagtgtaggccaggtatagtggctcatgcctataatcccagaactttgagaggccaaggcaggcagatcagttgaagccaggagtttgagaccaacctggctaacatggtagaaccccacctctactaaacagaagtacagaaattaaccaggcataggtggtgcatgcctgtaatcccagctgcttgctaaactgaggcaggagaattgggaggcagaggttgcagtgagctacgattgtgccactggactccagactgggtgacagagcgagactctgtctccaagagaaaaaaaaaaattgtacttacaggacatgaaacccacctgtacggtgtgctgactgggagactggagtatgcatagttcttggtaaacaaggggattcctgaaaccaatcccctgagtatatggagggttgactatatattttaatagaatttattacttttttttttttttttagcagttttaggtttatggaaaaattgagcaggagtacatagtttctctatctccctcacatttccccattactagcatcttgaaatagtgtggtacatttgttacaactgaagagccaaatattgatacattactgttaactaaggtccgtaatttactttagagttcactcttggtgttgcagtttctatgagtgttggcaaatatatcatgacatgtatctagcattatagtatcatattgagtagtttcactgccctaaaaatcccctttgttccaccttttcatccctccatctacctgaacccctgataaccactgatccttttacagtctctatagttttaccttttacagaatgtcatatagttggaatcatacagattggcttctttccatgttccttcctggcttgatagctcttttcttttttttgagatggagtctcgctctcgcccaggctggagtgcagtggcgcaatcttggctcactgcaaactctccgcctcctgggttcaagcaattctcctgtctcagcctcccaagtagcttggactacaggcgcatacctcccctgcctggctaatgtttgtatttttggtaaaggtggggttttaccatattggtcaggctggtctcaaacacctgtcctcaggtgatccacccacctcggcctcccaaagtgctgggattacaggcgtgagccaccctgccctgccagctcttttttttgtactgctgaataatactccattgtataggtgtatgagtttatctattcaccttctgaaggacattttggttgctcctaagttttggcaattatgcatgaagttactataaacatctgtgtgtaggtttttgtgtggtcatgtttttagctcatttggataaataccaaggagcacgattgttggatcgtatggtaagagtatgtttagttttgtaagaaactgccaaactgtctttcagggtgactgtaccattttgcattcccaccagcaatgaatcaagttcctgtcgctccacatcctcgttagcatttggtgttgtcagtgttttggcttttcaccattctaatagatatgtagtgatatcttgtcttactttgcagttctctaatgacgtatgatgttgagcatcttttcatctgcttatttgttgttgttgttgttgtgttgttcattgaaatggaatctcgctctattgcccaggctggagtgcaatggtacaatcttggctcactgcaacctctgcctcctgggttcaagtgattctcctgcctcagctccccaggtagctgggattacaggcgcccgccaccatgcccggctagtttttgtatttttagtagagacaggatttcaccatgttggccaggctggtcttgaactcctgaccttaggtgatctgcccgcctcggcctcccaaagtgctgggattacaggcgtgagccactgcgcctggctttcatctgcttatttgatatgtgtatatgttatttggcaaagtatctgttctgatcttttgcccattttttaatcagattgttcttttattgcttctggggttctttttgtttgctttttttgagacagagtcttgctctgtcgcccagtctggaatgcagtggcatgatctcagctcactgcgacctctgcttcctgggttcaagtgattcttgtgccttagcctcccaaatagctgggattacaagcatgtgccactgcacctggctaatttttgtatttatagtagggacagggttttgccatgttggccaggctggtcttggactcctggtcttcagtgatccacccacctttgcctcccaaagtaatgagattacaggcgtgagccaccatgcccggcttattgttaagttttaagagttctttgtatatgtgtattttttgattcttttaaaattaatacttaataaaataattgtacatatttatgggatgcatgtgatattttgatacatgcatacaatgtggatcaaatcaaggtaattagagtattacctcaaacatttgtcatttctttatgttgggaacatttcaaaatgtctagctattttgaaatatacaataaattattatctataagtcacctcattgtgctgtcaaacattagaacttattctttctacctggctttattttttttaccccttaaccaaccattcttcatcagctccccgtctcccctactctttttttttttttttttttttgatacggagtcgctctgttacccaggctagagtacagtggcacaatctcgactcactgcagcttccgcctcccaggtttaagcaattctctgcctcagcctcccgagtagctgggattacaggcgaatgctaccacacccgactaatttttatatttttagtagagatggggtttcaccatcttagccagactggtcttgaactcttgacctcctgatccacccgcctcagcctcccaaagtgccgggattacaggggtgagccaccatgcctggcccctcttactcttttcttagcctctggtatctatcattctactctctacttctatgagatcaacttttttttagctcccacatatgagtaagaacatgtaatatttctctttctgggtctggcttctttgtatattttggataataagtcttttattagatacgtgttttgcaaatattttttccgagtccgtgacttatcttttcattctcttaaatagtgtcttttgcagagcacacattatacattttagtgcagtccagtttaccaattctttctttgatggattttgcttttggtattgtgtctagaaagtcttcgccaaaccacagtcatctagagttccccttatattatcttacaggagttttatagtttttgttttacatttaggtctgtgatctattttaagttaatttttatgtgaaagatataagatctatgtctggattctctctttttttgagatggagtctcgctttgtcgccaggctgaagtgcagtggcgcgatctcggctcactgcaacctctgactccctggttcaagggattctcctgcctcagcctcccgagtagcacatgacaccacgcccagctaatttttgtattttgagtagagacggggttgcaccatgttggccaggatggtcttgatctcttgacctcgtgatccgcccgcctcagcctcccaaagtgctgagattacaggcatgagccaccacgtccggccagtttttttgttttatttatttatttatttgaaacagggtcttgttctgttgcccaggctgcagtatagtgacaccatcaaggcttcgttgcagccttgacctcctagggtcaagttatcttcttgcttcagcctcctgagtagctgggactacaggtgagcaccactctgaccaggtactttttaaatttattttagagacagggttttaccatgttgcccaggctggtcttgaactcctgggctgaaatgcccctcctaccttggcctcccaaagtgttgggattacagacatgaggcactcagcccagccaatataattcttttttttttttttgagacagtcttactctgttgcccaggctggagtgcagtggcatgatcacagctcactgcaacctctgcctcctggactcaagctgtcctcccacctcagcctcccaagcagctgggattatgggtgcccatgaccacacccagctaagtttttaaatttttttagagattgaatctttctttttctcagcctggtctcaaactcctgagctcatatgatctgcccgcctccgtctcccaaagtgctgcgattacaggcatgaaccactacgcccagcctacaatttatttgtaatccaagttttattgaaaaaaaaatccacatataagtggacatatgtagatccaacctgtgttgttccagtgtcaaccatatataccaataattcttttttttttttttttttttttttttttttgagatggagtcttgctctgtcgcccaggctggagtgcagcggtgcaatctcatctcactgcaacctctgcctcccgggttcaagtaattctcctgcctcagcctcctgagcagctgggactacaggcatgcaccaccacgcccagataatttttgtatttttagtagagatggggtttcaccatattggccaggctggtctcaaactcctgacctcaagtgatccacccgccttggcctcccaaagtgttgggattacaggagtgagccactgtgcctggcctataattctttacgtatattgttagattcagtttgctagtattttatttagcatttgtgtatctgtgttcatgagaggtattgttctgtagttttctttggtttcttttctgtctggtttagggtaatgctggcctcatagaataggttaggaaatatttcctctgcttctgtttctgaaagagaattgaggtaatatctatttttttttttttgagatggaatcttgctctgtcgcctaggctggagtgtagtggcgcaatcttggttcactgcaacctctgcctcccaggttcaagtgattctcctgcctcagtctcctgagtagctagaattacaggcatgcaccaccatgcctggctaatttttgtatttttagtagagatggggtttcactatgtgggccaggctggtcttgaacttctgatctcaggtgatccacctgtcttgtcctcccaatgtgctgggattacaggcgtgagtcactgtgcctggcccgagataatatctaatttaacagtttggtagaattcaccagtgaacccatctgggcctggtgccttttgctttagaaggttattgattattgattcaatttccttaatagataaaggtgcattgagattgtcttttcttcttgggtaagttttaatacattgtgtctttcaagaaattgttccatttcatctaggttatcaaatttgtgggattagagtccttcataatatttctttgttttgcttttggtgtccataggttcagaagtgatggccctttttcattttttctattagtaatttgtgtctttgcccttttttttctttgttaatctggctagaagcttatcaattttgttgatcttttcaaagaaccagtttttggtttcactgatttttctctattaattttgttttcaatttaattgatttctgctctaattggttttcttctgctcactttggatttaattttttttagtttttctagaaaactaagtttttaagtgaaaactgagattattgatttttagatcttttttctaatgtttacagttaacactgtacaatttcctgtaagcactgctttctctatatcttacaaattttgatgtcatattttcattttcatttagttagaaatatctcttgagacttctttgacccatctgttatttagaagtgtattgtttaatctccaagtatgtattttgggatttttctggctatctttctgctgttgatttctagtttaattacatgtggtctgagagcataccttgtatgctttctattcttttcaatttgttaaggtgctctttgtggctcaaggtggtctactttttttttttttttttttttaaagaaaagctggccaggtgcagtggcttatgcctgtactccagcactttgggaggcgtaagtgggaggatcacttgaggtcaggagtttgagaccagcctgggcaacatatagagacttcacttgcacaacaaatttttaaaatattagttgggtatggtggcatatacctgtatatggctgaagtgggaggattgcttgagccctggaggttgaggctacatgagccatgatcgcaccactgtactccagcctgggcaacagagtgaaattttgttctctcttgaaaagaaaaaaaaagttgatgacataaagttcattcatcttttttgtatgtgacttcaaaataactactgatggttaaaaaaaaaatcagaatgatgcaacccaagtgtccatcaatggatgaatagataatatgtggtgtatgaatacaatgggctactattattcagcctttaaaaataagaaaatgctgacactgctgtaacatggatgaacgttcagatcattatgctaaatgagaaaagccagacacaaaaggacaaatattgcatgattgcacttatatgaggtatctggaatataagagtcatagaaacagtaattcagtaattagaataatgcttgccagggcctgtggggaggagggaatgaggaattcatgtttaatgggtacagagtttcatttggaaaagattaaaaagttatggaggtggatggtggtgaggattgcacaacagtgtgaatgtacttaataccactgaactgtacacctaaaaatgattaaaatggtacattttatgttacatatgttttacaacaatttttacagatggaaaaaaattataaaaaacatcaggatggtgttgacagtgaaaaggttaaagagttactttaaaaatttactttattccagccgggtgcggtggctcacacctgtaatcccagcactttgggagaccgaggcgggtggatcacctgaggtcaggagtttgagaccagcctgaccaacatggagaaaccccgtctctactaaaaatacaaaattagccaggtgtggtggcgcatgcctgtaatcccagctacttgggaggctgaggcaggagaatcgcttgaacccgggtggtggaggttgcagtgagccgagatcttgccattgcactccagcctgggcaacaaagcgcaactccgtctcaaaagaaaattttttttttttactttatcccaaatgtttatatttactttggggcttatgtgaccagtttaattttcatttgtaattgacttgatagaacacactaatgttcagttaagatttcttatggtgtggtgaggagtaggatttttatgtaaataagcccaaaattgtatatatgaggttaatctgatatttgcagaagatattcatgcattactgtaaggaccactctgcttattcatttgaccgatttgttacaacatggttagaaatcatcaaggtgtttgagatcaaaggatcttcagaggtgatttactccaatccttttttaaaaaattaataacttgagcctcagagaagttaagtgacattaccaagttctgctgttagtatagtgactttatctttacctgaatccagggtttcttagccctagtctgtaatgtgtcctagtgtgcctctagaatctggtcctgtcagcccaagtctgttaaatcaaataaaaccagggcttggtgcttcaccttgtcttctgccataccgttgggtttcctgtggaccatgcagataatgatgatgggctcagtgggcttgatagtgataactcctaaagcagctccttctaagtgcggttctcaatctgaggaagttaaaaaaaaaattagtgactagaacccacttctcaggtactctgataaaatacatttgtaggggagtgatagttttcactttctttttttctttttcttttttttttgagatggcgtctcgctcttttgcccaggctggagtgcaatggtgcgatctcagcttactgcaacctctgcctcccagtttcaagtgattcttctgccttagcttcctgagtagctgagattacaggtgtgtgccaccatgcctggctaatttttgtatttttattagagacgggatttcaccatggttggtcaggttggtctcgaactcctaaccttgtgatctgcctgcctcagcctcccagagtgctgggattacaggcatgagccactgtgcccagccttcacatattttttgaaataataggccagttgcggtggttcatgcctgtaatctcacactttgggaggccgaggtgggcagatcacttgaggccaggagttcaaggccaccctggccaacatggcgaaaccctgtttctactaaaaatacaaaaaaattagccgggtatgatggcatgtgcctgtggtcccagctactctggaagttgaggcatgagaatcgctttaacttaggaggtggaggttgcagtgaggcaagatcgtgcccctgcactccagcctgggtgacagagcgagactccatctcaaaaaaaaaaaaaaaaatcgtatgcagtaaaggttgaaaactgctgcccaaaggcgctattaaactataggttcccaaacctggccaattgtcaaaatccctcaagaaggggcagtggggtctaagggaccccattgctgtagaggagattagtagtccaagagtgagatgaactgttggaagtcctcaaacttccaaactattaaaatagaatagttttgcttccttaaaatagaatagttttcttcctcactgatttttctgtattgattagaaccataacaagtgaattaaacaactacaaaatagttatgtgggccacagacattattgtaatgaagtgaagtttggctcaggccttgtaacacaattgctttttggattaaaagtaaaaatattaaattgtgaaattatgtgtaagttttaaaaaattggtcttgtacaaaagtgttgggtttttctttgtttttaactggatttgtttttaagcaagacagaatatttatattgttggagagtcacaaaggaggtgtgtttgtggatttaaatgtggagacagtgtgccttgaaatgccctttatcagtctgattcaagccacctgcaatcatggatttgaacttttttttttttttcccctgagatagggttgcctaggctggggtgcagtggtgtgatcttggctcactgcaacctctggctcagcctcttggagtacctgggactataggcacacaacatcatatccagctattgtatttttttttttttttttttttatagagacagagtttcaccatgttgtccaggctggtcttgaactcctgagctcaagcaactcacctgcctcggccttccagagtgctgagattataggtgtgagccaccatgcccagccttcactttatttaaaaaccatagtttttaaaagccacattcctactgatgaacacagaggttgtttccagtgttttcatttgcagggctgtagtgattgtttttgcacatgcctctttatgtacatgtgctgtgtcttctgggacagagagtggacattttaagtgttttattggtcctgctaaattgtctttcagccaaactgctgcagaggtgatggagatgaggtgggtactcaggagaattatgctcagtgcttgtgtgctagtcactgacctggaaacattttattaaaaatgctagattaggttagtgatgtaaataccaggtgatagtaaccagaataattgtgtcaaaacatcaagaatcatcaagagatgccaggcatggtggctcatgcctgtaatctcagccctttagtaggaggccgaggtgggcagattgcttgagctcaggagttcaagaccagcctaggcaacatggtgaaaccctgtctctaccaaaaatacaaaaatttgctggatgcagtggtacgtgcatgtggtcccagctactcagtaggctgaggcgggaggatcgcttgagcctgggaggcagaggttgcagtgagccaagactacactacagcccgggcaacagagtgaaaccctgccataaaaaaaggagaaaaagaatcatcaagagaaaacttaatttgatgtgctctgcgttttctttggtgcttcatgtcagtgttagaaactataggttgtatatttattaatttttctcctacatttgttcaacttgactaaaatattaactccaaatgcctagaatttcaaaatacctcttcgttataaagtatcaactatttcttagtccccttaagctgatagtattgtgtcattgtaaaagatcccttgtgaaaaataatttttgtcaacatgaaaggtcttaatgtgtctcctagtttacattttacatggtcttttccatgtatttatatagttgacatatatagctttttttgtaaatacactttcctatgtgaacatgccaaggtttacttaagcattctcttattcttggacatctaaattgcttcttattttctattgtaaataaagtgctagaagcttctttcctgaaaagttatttacttttcacctagtatttccatctgtgttcctcaaaataagattgctgagattcatgtatgttgccagaaagattgtgaggtttaacagtgaatgaggaaaacttttaacactcaaggtctaccaagtacagcaagttttattttacctttttttttttttttttttttttttttttttgagttaggccaagttgcctaggctgggctcaagcaatccttctgcctcagcctccggagtagctgggattataggtgtgcagcaccacacccggctttcttgtattttttttttatttttatttatttatttatttttgagatggagtttcactcttgtcacccaggctggagtgcaatggcccaatctcgactcaccgcaacctctgcctcccaggttcaagcgattcttctgcctcagcctcccaagtagctgggattacaggcatgtgccaccacacccggctaatttttctatttttagtagagacggggttcctccatgttggtcaggctggtctcaaactcccgacctcaggtgatccacccacctgagcctcccaaagtgctgggattacaggtgtgagccaccgtgcctggctgctttcttgtattttatcttgctgtagcggttgtgggatttttgcctggtgtgttcattggagtgtgtgtgtgtgttttgagatgtatgactgtgttggttgtgttgtcatactttgaaggttcattaatgtgctggtctttctatttttcttgttatacttagtcacttaaaaacccttttttttttttttttggaattcttatttttacagtactttgaattcctgttttattaatcaccttcttatctgaaagtgaagtaatagtgtacttggcaccattgaattagaaaattgtgtgtccttggccagaagatcacatacacaggaactcgataagttgagagatttagccgtttcagaaatgggcatttgtgtcttccagtggagaagcatctgcaaaagaattgggcagatttggccaggcgcggtagctcatgcctgtaatcccagcactttgggaggccgaggtgggcagatcacctgaggtcaggagtttgagaccagcctggccaacatggtgaaaccccgtctctactaaaaatacaaaattagccaggcgtggtggctaacccatttaaagtgggtgaattatatcttttatgttttaatgtattcctagagttgtgcaaccatcaccagaataagttgtagaacattttcatcaacccaaaaagaaactttgtattcattagtcgttcctcctcatttctcccctaacctcccagcactaggcaaccatcagaatactttttgtctccacggatttgactgttttggacatttcatattaatggaatgcacaatacagtagtataatacattaattttggaaggccaaaattaatggcttttgatgtctgccttttttcacttagaataatgtcttccaggtccatctgtgttatagcatgtatcattactttatcctttatgtggctgggtaatattccattgtatggttataccatgttttgtttatctattcatcagttgatggacatttaggttgttttccattgactattaagagtaatgctgccggccgggcgcggtggctcacgcctgtaatcccagcactttgggaggctgaggcgggtggatacgagggtcaggagatcgagaccatcctggctaacacggtgaaaccccgtctctactaaaaaacaaaaaattagccgggcgtggtggcgggcgcctatagtcccagctacgcaggaggctgaggcaggagaatggcgtaaacccgggaggcggagctggcagtgagccgagatggcgccactgcactccagcctgggcgacagagcgagactccatctcaaaaagaaaaaaaaaagagaataatgctgccatcatgcttgagggtttttttttattttgttttgttttgtttgtggggggagcggagggcacagtctcactctgttacgcaggctggagtgtagtaggcttactgcagcctcctccgccccctggttctagtgattcttgtgcctcaggctcctgagtatcatgctgcaatttttgtgtgagcatacatttttcatttctcttgggtcaatatctaggagtatccccacttttggttctgagtgttaattgagcctgttgtgttctcacattccctgtacttagatggaaatagtgctttgcctaaaaagaaaataaaagacctgattgtgcaggcgagtgagaaagagagagaggcgctagggttatttccaccctgatactctttgggtagtcttggtatgactagcaaagaagcaagctccaagttgtagtttgcttccaagtttctggcttctgtgggaatttctgcatctaagtaatgacaattttcagttacttgcagtaagtaaattatcaaccaatcttactgtgtattactagcctagtaggaatttacttgtatatcgagaggaatgctgcagctttcaccttacttctaatggggattaatgcttacttaacttgcagttttggaggcaagtacaaagtacaggaccaattatggtcatgaagtgagagagaagtctggctagtgaatggtgattggcaactccagttgactgttcatggcatcttagatctgtgaggagggaggagggaaggaaagttcaagctggtctttatggtaagttctggaacatttccctgtgtcaatgggtcatctgttcattcactgtgtaaaatggttgagggaagttttaatttacatgcttccttattgtgtaaacctttgatttttagtgatttcagagtttgtttttataattacttaacacgtgaagaggatgcagagtaacgtatcgaagctctggttaccttccactgggatttgacacatttgatttcctttattccctccttccttcccttcctccctctctcttttcttaaggaatgcaactactcagattcacctgcacacccttggcatacctctcactcccccttacccccacttcctcagaggtgacctgtcctcagaggcaaatgtgtgccctttccatccgtacttttatgctctcatctatgtttacatctattagtacactattgtctgtatttttaaacattacataaatggtgtaatttttacttttaattctgtagtggtgtttctcaaattaagttctgcacaaaacatttttatagatatccagtgttagcttaacgtttttcttattgtggtaaaatatacataagataaaatttaccattttagccatttttaagtttacaagtcagtggcattaagtacattcacagtgttgtataaccatcaccattgtccattgccagaacttttcatcatcctaaacagaaactctgtactcattaaacaatagtttatcactccttccctgcaactagatgctggcaatcaccattctactttctatctctatcaatttgcctcttccatctaagtggaatcctacatatttgtcgctttgtttctggcttttttttcttcttgtgatgctttgttttaattatgttcctggctttcatcatctagcaggctgattccaaggtttgtccatgtggtagcttgtatcactttaatgtttttagagatagttaatattacattgtttatatataccacattttgttttttcattcaaccttgatggacatttgaattgtttccccctttacctgttgtgaataatgctgccgtgaacattgataaccaaatatttgtttgaatctctgatttcagttcttttggttccatacctaggagtggaattgctggatcatatgataattctatgtttaactctttgagggatggccagacttttccaccatagctaaatcattttaccttcccacaagcaaagttcaagggctccagtctctccccataaggtcctttgcacttttttttttgagacggaatctcactctgttgcccaggctggagaacagtggcaccatcttgcctgacctcaagtggcacctgccttggcctcccaaagtgctaggattgtaggcgtgggccactgcactctgccaattttttaatttttattttcatttatttttctttttttaatttttaatttttttattttttgaagggataaggtctcactttgttgcccaggctggtcttgaactcctggcttcaagcaatcctcctacctcggcttctcagagtgctgagattataggtgtaagcccctgcacatggcctttactctcttgatagtgtcctttgatgcacaaaagctttcaattttgatgaagtttattttttatcttgttacctgtacatttggtgtcatatatctaagagaccattgccaaatgcagtgtcatgaagctttccctcagtgttttctttctgcagttttatgattttagctcctaagtttaggtctttgatccattttgagttaatttttgtatacagtttgagagtcacacttgaggctctgggcgcagtggctcacgcctgtaatcccactacttggggaggccgaggcggatggatcacctgaggtcaggagtttgagaccagcctggccaacatgccgaaaccctgtctctactaaaaatacaaaaattagccaggcatggtgatgcatacctgtggtcccagctacttgggaggctgaggcaggagaattgcttgaacacaggaggcggaggttgcagtgagccgagattgtgccactgcactccagcctgggcgacagagcgagactccatcgtgcggggtggggggtaaaagtcaaacttgagtcttttgcctgtggatatccagttttcccatcactatttgttgaaaagactatcctttctcaactgtgaatggtcttggtaccctagctgaagttatttttattattatgttacttaggaatgcacataaggcctggcacggtggctcatgcttgtaattgcagcactttgagaggtcaaggtgggaggattccttgagccgaggagtttgagaccagcctgggcaatatagcagcaagaccccatctctatattttaaaaaaagaagaaaaaaaaacctctgatgcataaaatatttaaacttgtatgcattcttttctttctttattttttaaaaattgagacagcagcttactctgttgtccaggctggtcttgaactcctgggctcaagcagttcctctcaccttggcctgcagtgctgagatgacaggtgtgaaccactacacctggcctgcttacagattataaaaagaaaataagtttacaagttaaagacagataaaatgacaaaatcagtaaaattaaaattacttttatggagccgatgatgtttattccagttgctcctctcattgtgaatatggtattgttgctgtggcagatttggaggccgtggcagatttggaggctttggcaatggcttctgttaccttgccatgaggtaactcagttccctcatcacttttctctgagaactataaaaccttggaggggtgccttctgcccttcgcttggcatgtatattatgcagggatcaggtcttactccgttcttgattgttagtacaaattagttaaaattgtattgtttggccttagcctgatggtaaacacaacagcacacgtgggctgtgaaatctctgggcagctctgtgtttctagggaagcatctcgatgatccagaacaggcttatactaatgttttagtgtaattttgaaatgaaaacacagcatttaaaaattcttatagagaatgtatagaccttgagaagtgttagcagacccagtttacgacatgtctcaatattatgaaacattgctttattccctatcctgcttgtacatttaattttttcatccagttttaaacaacttgggtactgtggcctgtgcctgtattcccagctactagggaggctgaggcaggaggattgcttgagcacaggactttgagggctgtagtgagctgtgattgtgcctgtgaatagccattgtgctccagcctgggcaacatagcaagaccctgataccttgggtttttaaaaaacaaaacaagatacatgctgacatttctggtttggcaggcagagcttgttctgctccccaccctcccttttcccatagtaaccatttataggacatctcactgttgtctactctgtgttgcctctgcttccctgcgtggtagatctaggaatcttaggatttcttagttttagctggtgatccgtatctttttcttaattccattgtaacttcagcttttcttattgcttgtaggaaggctgtttccattgaatacaaacaaaataaaagcttttattcttaatcttagagataggatgtttgtatttaaaaataattgtgctgtcaaaattctgtcaagttggcttttaccacattagttttttttaatgtggtttatatgaccctggagtaccttgtcttctcactgttaaattctcaactgagttgtccctatttaaagtgtgagactgtgccagtttgattttaaaatattgcaagtgcgttatggcaagataaaactgcaaagaaagaaccttcatgtccctttgattataaatgcttttggcacttgtttctactttttcctaatgttttttgaggaaagaacctccaactctccagacaggtctgggggcaaatgactaaaacatgaactgaggccctgggctgtctctgtgaggatatcccctctattctctctgaaatgtcccagcatgtggtgcatttcttgttagtgtggactcctctgtatataacacatcttatttatcttctgtgcataacatgaagtagtgccctaatgcaattccaggatgtaattcagcatttctataaaaatacagtgtttttctacatttgcatcaaaaaataaccagataattatatttattaagaaaatagcatttttggctgggtgtggtagctcacgtaatcccagcactttgggaggccgaggcaggcagatcacttgaggtcaggagtgaggcaggcagatcacttgagatcaggagttcgagaccagcctggccaacatggtgaaaccccatctctactaaaaatgcaaaattagcctggcgtagtggtgcatgcctgtaatcctagctactcaggagactgaggcaggagaatcacttgaacttgggaaggggagattgcagtgagctgagattgtgccactgcactccagcctaggcaacagagtgagactctgtttcaaaaaaaaaaaaaaaaaacaaagaaaagaaaagaaagaaagaaatgtatttttggtatttgttttcacaaactagagcatttatgtgaaataacattgctagtattgatattataccatagtataatacttagttcttcagcgatgtatctctgctgatcagctacatgatatctacttgagctgttggattttttttaagaacagtgcatttttgaatgcttttgaaaaattgtagtaaaatacataaaacaacatttaccttgtaagcattttaattggtacaattcagtgacattaagtacagtcccagtttagtgcaaccactgttactgtctagtttcagaacgtttttgccccagatggatactctgtacctgttgaacattcagtcctcatggcccaataatctttatgtctgtatagatttgcctattctgcatattttatataaatggaatcatgtcttttgtgtctggcttcttttacctagcatagtattttcaaggttcatccatgttgcagcatgtttcaatactttgttcctttttatgtccattgtatggatatgccacatttcgttaatgacaattcttttgggtagctacattttaaaacattatagtagaatacatatagcatacaatttactatcttaaccatttaagcctgcagttcagtggcattaaatacattcacgttactgtgcaattatcaccaccatctgtttgcagaaacttttcatctcctccatttgaaactctgtatacattaaacatgaactctcccttctccccttcctccagccctggcagccaccgttctacatttttatctttctgacagagattttactactctaggtacctcacataagtgaaatcaaccagtatttatccttttgtgaccagcttatttcattagcttaatgtcctcaaggttcatccatgttgtagcatatgtcaacatgactttccttttaaggttgaataatattccattgtatgtatatgtcacaatttgtttctccatttatccatcactggacatttgggttgcttttacctatcggctgtcttgaatcatgttgctatagctgtacaagtatctatttgagtttctgctatcaattctttaagtatatgcccagaagtggaattgctggatcatatggtaattccgtgtctggttttttttttgaggaagtgccatgctgttttccacacagctgtaccattgtacattccccccagcaatgtacgagggctctgatttcttcacatccttgctaacacttagtattttttttgatagaatagccatcctaatggctacttttaaagtatgtttaacattatttatttatttttaattttttttgtagagatggcatcttactgtgttgcccaggctggtcatgaactcctgggctcaagcagtcctcctgcttcagcctcccaaagtgttcggattataggcgtgagccaccatgcccagcccaaatttaaatatataactaaacacatagcagctaacaccaagcctttaaaaatatcattaataggccaggcgcagtggctcatgcctgtaatcccagcactttgggaggccgaggcgggcagatcacctgaggtcgcgagttcgagaccagcctgaccaacatggagaaaccctgtctctactaaaaatacaaaattagccgggcatggtggcacatgcctgtaatcccagctactggggaggctgaggcaggagaatcacttgaacctgggaggcggaggttgcggtgagtcgagatcgcaccattgccctccagcctgggcaacaagagcaaaactccatctcaaaaaaacaaacaaacaaacaaaatatatatatcattaataggccgggcatggtgtctcacgcttgtaatcccagtgctttgagaggccgaggtgggcagatcactggggtcaggagttcgataccagcctgggcaacatggtgaaaccctgtctctgctaaaaatacaaaaattagccacgcatggtggtaagcacctgtaatcccagctactcaggaggctgaggctggagaatgcttggacctgggaggtggaggctacagtgagctgagatcacactccagcctgggtgacagagcaagactctgtctcaaaaaaaaaaaaaaaaatcattaataaatgtgatcttttttcttcctatacaacaagttgtcaagcaagtatgaccttcttaattgaccctttgacatgaactgggatgagatcgtggaggatgttgaggagacagttgttaccatagtgcacttctaaaaactttaattctatagatttctttaaaattttttttaaaattattatgagtacacaataggtgcatctatagatttcattaccctcaaataaatgtacaaggcaatgcagagaaatgcacagtgtaacttggtagacttgacctatcaagttactgttgaatatattatggagcctgtgtattaccaggggcagcagacttttcctgtaaagatagttgttttcagctttgttgaatctgtggtctctgtcttaactacaactgagaaagccattgacaatatatagatgaatgtacatgactattctaataaaactgtgtacactgtaatttgaattgcacataattttcatgtgtctcctgtataattcttcttttgacttcttttcaaccattaaaaaatgtaaaaacaggccaggcgtggtggctcatgcttgtaatcccagcactttgggaggctgggtggattgctggagcccaggagcttgagatcagcctgagcaatgtgatgaaaccctgtctctacaaaaaattagctgggcatggtgttatgtgcctgtggtcccagctacttgggaggctgaggtaggaggattgcctgaacccgaggaagtcaaggctacagtggtttgtgccactgcactctagcctaggtgacagagtgagaccctgtctcagtgaatgaatgaatacattattagcttgtggactatacaaaaatcagaggctggaggtgagctgggtatggccattgggtgtggtttgctgacttctggtagagaggaattaggagatgttaaaggtggtggaactgtcagatacttgcattcttttagaaatactttggagttagctttttggttcaggcaaaggaccaaagggttaggagagtcaggccggtaaagaggagtggtgggcccatagcagcagttcctggagttttttttttttttttttttttgtgagacggagttttgctctgtcgcccaggctggagtgcagtggcacgatctcggctcactgcaacctctgcctcctgggctcaagcaattctcctgcctcagcctcccgagtagctgggactacaggtgcccaccgccacgcccggccaatttttttctatttttagtagagatgggatttcaccgtgtttgctaggatggtctcgatctcctgacctcgtgatccacctgcctcggcctcccaaagtgttgggattacaggtgtgagtcaccgcgcctggccaggtcctggagtctttaagaggaggtttgtctgatggttggttggacaaaagcctgggcatgttgtcaccttccataagtgtttgtgggaatgtaggtaatgaggaggagtaaaggattcctgaaggatgaggaggagggctggtggctgccataggaagtgatcactgttttggcagacctgtcttagagtaatgaccgtcatactctctcattgcccttgtgaactcatgaaatcccatggctgctaaagctgaaggtcaagtggggacttcccggccactgggcttagcaccccacagagctgtggagtgggcattaatgtcccttttttatagatgcggagactgagaatgaggactgttggtaacttttgaaagggcactcagctagaaaagtctgagccaggatttcaagtcccatggctttacctctgtggtcctaatatttggtgtgttcaagtgagatctgtttttttcctatttcattttgattattgattttcataaatttttttctcttttgagatagtatcttctctctcttttcttttttctgttctttctttctcttttctttctttttttttttttctctgagacggagtcttgctctgtcgcccaggctggagtgcaatggtgcaatctcagttcactgcaacctctgcctctcgggttcaagcgattctcccatctcagcctcctgagttgctgagattacaggcacctgccatcttgcctggctagtttttgtatttttgtagagacggggtttcatcacgttggccaggctggtcttgaacttctgacctcaggcgatccacccgcctctgcctcccaaagcgctgtgattatatgcatgagccaccatgcctggccattatttctttctttctttctttttctttttttcaggttcattgaatttgctttgagacagggtcttgctctgttgcccaggctgaagcgcagtggtgcagtcatggctcactggagcatcaatttcctgggctcaagcgatacttgcacttcagcacccctccacccccacccgctcctttcccccacagtagctggaactacaggcgctagccaccgtgcttggctaattttttttttttttttttttttgagacggagtctcgctctgtcacccaggctggagtgcagtggcgcgatctcggctcactgcaagctctgcctcccaggttcacatcattctcctgcctcagcctcccaagtagctgggactacaggcgcccgccaccatgcccggctaattttttgtattttttagtagagacggggtttcaccgtgttagccaggatggtctcgatctcctgaccttgtgatccgcctgcctcggcctcccaaagtgctgggattacaggcatgagccactgcacccggcctggctaatttttaaatttttttttgtagactgcccaggcttgtttaattgattttctatgtgatcttagggaaatcgattatttcccataaacatttttttaattagaagttaaattctgcctagtttgattcacaggattattgtggatgactgaaacagagaataggtaagagcttctttgaaaaatatgaggtaccatacagaagttagatgctttgtcctggtgataccccctccaaagcacagctaaggaaatgtggaaggcactcttatctcatcatatagctttgaaagcctagcattgaaagtacgaacttgattcttttggagaaatcctttggctctcagtgagtttactttctattaatgactgtgttaagcggaatgaaaactgaaagaggaaaggggaggaagtcagaattaagcaggaagagtgagcccatagcagagtccagatttagaccccaagctacttggaatgatactggacaattatgggtgtgtttaatgatggtcctgagtcatgaaaacaaaaggaggctttaaattatgtctggcttagtgtacagcatatttttgtcattattcaagttttagcatgtaaagaggaaagtgtgcagtacttatgcatatcattttcattaatgaaactaaatgaggcctctttaaaattatcagtgttcacagtatcttccaaaagacatgtaaatgtataaaggtataaaaaatatacatataaattttacaattttgtgagctatatagtagatctcttattttgtccataggtcttaaagatcttatactgtattcaggaataaagataacttcagtgggaggcctttacagggctaatgagtaagcattattttgataaagttctgtgttgtctacaatagatatagtagaaatactcttggaatggtaatcatcccaggccctgctttggagcggaagaaatagtcaatgtagaactttacagtatattgtacacagatgtgcctgctaataacttctgtagacagcaaagtttaagagaaattaggtggtaaatgcaacatatgtatctaaataaatttggtctgagggatttgataagatgaaacagtacatagtccagaaaatttttatactcaaagaattatagaaaatatctgaaatgttttcagttttgtgcatatccagaaaatgtcatcctgtgatctgctggttggcagcccaatggcagtattagatgtattgtttttattttgttttgtttgctatttatttggttaagagagttacctaattaggagtgtgaaaaaaaagatttattatagtagtgggcttttgtttgacttaaaacatttttgttgttaccacagtatgagtgccttgtttgtgaaatttgtttaccgggaagccatatacttagagtagcttttagtttatcattatcatcatcatcatcatcatcatcatcatcatcatcatctccttcatcatgaaaggaagaagctaccaatgttgctttattctgcaaaaaatacaatagatgcttgttgaaagtatggagtgaaatcttaaatatgtctgttaaaaagagtacaactggccaggggtagtgcctcatgcctgtaatcccagcactttgggaggccaaggcgggcagatcgcttgagccaggagtttgagaccagcctgggcaacatggtgaaatcctgtctctacaaaaaaaaaaaaaatagacaaaaattagctgggtgtgatggcatgcagctgtagtcccagctacagtggggctgaggcagggggattgcttgagcccaggaagtaaaggctgcagtgagctatggttgtgccactgcattccagtgtgggtaacagaacgaaaccctgtctcaaaaaaaaaaaaatagtacaactttaagcaggatgtgggcacatgcctgtagtctcagctacttgggaggctaagtcaggagagtcacttgagcccaggagcttgatgctgcagtgagatgtgattgtgccactgccttccagcctggggatgatagcaagaccccatctctaaaaaaaaaacaaaaaacaaaaaaaaaacagagtacaacaacctttggtaaacttggaatataaaggtgtttccttaacctgttaaagagctgataaagagtggtactttcaaaccagtacacattatgtgaaacactagagacacttcccatttgttaaaagaaaaaccttagccaaattaaatttaagttttttttggagacagagtcttgctttgtcacccaggctggagtgcagtggtgcaagcacagctcactgcaacctccgccttctgggttcaagtgattttcctgcctcagcctcctgcgtagctgggactacaggtgtgcaccaccacgcctgggtgatttttgtattttttgtagacatggggttttgccatgttgcccagtctggtcttgaactcctgggctcaagcaatctgcctgcctgggcctctgaaagtgctgggattacaggcgtgagccaccatgccatttaatggtttaattgagcaaagaatgatttgcaaattgggcagcctcccgagccagagtaggttcagagactccagcacagccatgtcgtggaaaaagatttatgaatggaaagaggaaagtgatgtaccgaaaacggaagtgaggtacagaaacagccggattggttacagctctgaatttgccttatttgaacacaagttgaggtttgtacagttggccacctttgattggccaaaactcggtgattggcacaagagcaggttatagtctgtttacatctccattttggttatagttcattatggacagaaaaacctgtaggtcaaacttaaaatatgtaaggagacagttttaggctaaacttgatttaacacattaaatccgtaacaagacaggatgcctgccctcaccatgttatttgatcttattttagtaattctagccaatgtagtagggcaagaaaactgcctgcttggctacaaaataaacacacaaaagtcagtatctgtaatatgtgacagaaaatataattaaaaaaaaaaaaaaaagccgggcacagtggcccatgactgtaatcctagcactttgggaggccaacgtgggtggatctcttgagctcaggagttcaagaccatcctaggcaacatggcaaaaccccgtctctacaaaaaatacaaaaaaattagccacgtgtggtggtgagctcctatagtcccagctactttggaggctgaggttggaggatcatttgaacctgagaagcacaggttatagtgagctgagatcacgccactgcactccagcctgggtgacaaagtgagactctgtctaaaaaaaaaaaaaaaagaagaaaaggaaaggaaagtaaaagaaaaaataatttcacttactagagcatcaaatccctaagataatttagagcaaagccagaaaagtgaagaaaatataaaaatctttacagtgggttgcattttaaaaaaaaacttgaagatatcagatcaactcactaatgtattaattaatataatttaaattaaaatcccactgatttttttgtggggagggtgggagagtcatttgttaaaatgattctaaagagcatctggaagaataagcaggcaagaatagccaagaacattttgaaaactaaagatgagtttggaagacgattggttttgtactgtcaactacttatagattttacatgaattttaaagggtaatctgagccctcgaatagacagaaatagccatagatctgaaagaacacttaagacctgatccagctatccatgagagtatatataatcaaagtctttgtgtgtgaatcaggagtctttcaggtgcaaggtaaataaactcataattgcttacgcaaaggtggtatttgctttagtgactccagagaaagctcaagtgcctatctctcccctgactttgattctttttggggttggctccattctctcctgttgctaatggcttcctttgtgcagccagaggaaaggaggtgtggttttttgatacttccaggcttctatttttatagcttgagatcaaagagggaagtgaccttccttagagtcagtgtgtaaagtcctaaggaagataccacgtggggtgctggggccatgtgcccatccctggcccatgaccatggggatgctacactaactgggggccacgcatggctgttcctgccctgaactgccagctggctttgcagtgcagcctcaccagaatcacatggaatagtagggatatgaattgtttcccaaagaaagtgtgtggggtggtagaattactagtgggggagtaaggggacaggccattgggcatactggagcagcatttactcagtcattgagaaaaggatggaacattcaataaagggtgctggacacatttgtgctctaaaaattttgtgtttcacctattaatttatccctccccttagcccctggcaaacactgatctgtttactgtctccatagttttgcctttcccagaatgtcacacccttggaatcatacagcatgtaaccttttcagattggcttcttttacgtagtaatatgcatttaggattccttcatgccttttcctggattgatagctcatttctttttagtcctgaataatattccattctatggatataccacaattgatccattcacctactgaaggtcattttgattgcttccaagttttgataatttaaaaaattttttaagacagggtgtcattgtgttttccatactggtctcctgaacacctgggctgatgtgaacccctctcctcagcctcctgggtaactgggattacagctatacaccactgtgcccagtgtgacaattatgaataaggctgctgtaaacttctgtgtaggtttttttgtgtgtggacattggttttcagttcattatggtaaataccaaggagtgcagttgctggattgtatggtaaaagtatgtttagtttgctaaggaactgccagctgggtgtggtggctcatgcctgtaatcctagcataatgggaggctgagacaggaggatcccttgaagccaggagttcgagactagcctgggcaacatagtgagacctcatctctacaaaaaatttaaaaattagctgggcgtggtcttatgtgcctatagtcctaactgcttgggagactgaggtgggaggatcacttgagcccaggagctggaggtggcagtaaactgtgatcataccactgcactgctgcctgggtgacaaagcaagaccctgacttaaaaaaaaaaagagaaaagaaaaaaagatgagtcagagggtaaggaagcaaaaataagtaaataaataaatagaagagaaaagaaaaaagaaaaaactgtctttcaaagtggctgcgccattttgcattcctaccagcaatgaatgagagtctgttgttgcacatcctcaccagcatttggtgttgtcagtgttctggattttgaatattctattaggtatataatgctgtctcacttgttttaatcaatgatatatgacattgagcatctttttaatatgtttacttctcatctatgtatcttctttagtgaggcctttgtttaggtcttctgcccattttaaaaaatgggttcattttcttattgttgaatatcatgagttctttgtctattttgaatacctgccttttgctttatttttgtgttttttattttttttttttattgagacaagttctcactctgttgcccaggctagagtgcagtggcatgaacatggctcactgcagcctcaacttctcccagcctcaagcaatcctcttgcctcagccttccgagtagctgggactataggcacacaccaccatgccctgctaatttaaaagagtttttttttgtagaggtgggatctcgccatgttacccaggtggtcttgaactcctggcctcaggcaatcttccagccctcagcctcccaaagtgctgattataggcctgagccacttagcctagctcagaatttattttttatttgttaattttgaaaaaatataggacctcataaaagtcagtctacatttgtacacattatgtttttggtgaatatgtaaatggattctttgtgaatcaatttggttttgtttttttgcttttaaaaataccagccctgggctggatgcggtggctcacgcctgtaatcctagcactttgggaggctgaggcaggtggatctcctgaggtcaggagtttgagaccagcctggccaacatggtgaaacgctgtctctactaaaaatacaaaaattagctgggcgtggtggcgcatgtcagtaatcccagctacttaggaggctgaggcatgagaatcgattgaacctgggaggcagaggttgcagtgagccgagatcgcgccactgcactccaaccttggcgatagagcaagactctgtctcaagaaaaaaaaaaatgccagcagtggctggctgaggtggctcacacctataatcccagcactttgggaagccaaggcaggtagatctcttgtggtcaggagttcaagaccagcctggcgaacatggcgaaaccccatctctaccaaaaatacaaaaattagctggatgtggtagtgcgcacctgtaatttcagctgctggggaggctgagacatgagaatcacttggaccctggaggcagaggttggagtgagccactgtattccagcctgggtgaaagagggatactctatttaaaaaaaaaaaaaaaaaaagcgggctggatacagtggtgcacacctgtaaccctagcactttgggaggctgaggtgctcagattgcttgagctcaggagtttgagaccagcctagacaacatagtgagacatcgtccctaaagaaaaaaaaaaaataccagcacttagccaaaagatttcaacagtgcagaaaaagaaagttgtgatatcttttctccaaattagtcttgttttcagtttcattatccaagtaaccactactaatagttaaaacatttgaaatacgtgtgggagcttgtcctatttaatataaattatttattgagcaaataatcaccactagtatgttttggatactggaattttcatatgtaggagtccttgaatgtaaggtgcccctttggtagttctgtgcttcttttacctgtactgtaacatagggaaagatgttacaaatggttgtatttttaacagagcagtatctattcttaaacaccagcccttccactaaaggtaaacaacaaatgaatacataaatgaagttttggtattgggattatgtgggttaaacacatccatatttcattattaatatttaagaatataacaaactttttattggcatttggaccttgtagctaaggaaagattaaactttgtttatttgtgctttgttttttttcttcactcagatatttgaggatttcccatttgaggaatacatttattaatcaagctttagtttcaagatccttgatcttagggaataccatcaaccgttcttctttaagcttcctaactttgcccaaatttggttagaactactcaagagtagtttgggtaattcagaaattttattggaaggggaaagaatttttgacccaaattagataaagcaactcttgggtaatgatttcttttcttgttctctctttataatcaattgaaagtagtagtaaggctgggtggcaaaagaaagaggcctggggagaatcgcgtggttttcattatctcttttcatagcagcaaagtgggaagggaccaagaggaaatcaactgaaaaaccatccttctgaaacattggcctaaaaaactgtagtccagaaattgagtgcaactggcagtggcatttaaaaggaatgctctaatttctaggaaagcaggcacgagtacctcttaaaagaagaaaaaaatgaaaactgtaatttaggacacatagacgagtatccattccctgtacttttactctcatgtcctaaccaaggaagggttgccatagcaaatatggcattccttagccatgattcactgttgtaaatgcctgcagcattcataaaagtaagatatatgggctcttctttttccttttaaatctttatttctgtatttaaatctgtatgtcatcatctgtattttctctcttgttttttttaaatcttgggagatggtacaaattatttaggggagggaatgagtttcttgtccacaaatagaggagagagagggctttttgtctttctgctttggaactggagagcttcctatttaggcatggcctttttcaagtgaccttgtattgttatcagtactgtagaaggtaggcacgttgtgtaaactttaaaattgaaagccattaggcattccacttgtaaaccttggctttttaaagaaaattacatgttcattgtgaatattttcttatcgacctatctctgtgcacatgcagacttcctttgcctacattctgaaaggtgtaattgccttctttaaggacagcggacatctatagttcttgggtcaaattgtcctccttctggttttgtcagttctcagccacactgtgtgagcatccattttcttggattctggttcggagctcattttaaggaacatcatgtcccttttgagactctgtggacattggggtgggtagatgtccccctgtgaacagaaggtccctccctaaggaggtgcttctctgtgttgagtcctgcatctgggcacacagagcccgaagcaggaagagttgagtctgaatagggaggcctgtaagcctgactgctctgccacgggtaggcctggtctgccatgctccaggagcccccaggaggctctgaagtcattctgcctctgggaattttacagaggagctaatatttgagctgagtgagaaggtgattcttgaaaaagcaaggcgtgccctggtccagttctgtggggctgtcgtagaagagggctcggaagctcttgggagtgaggctagaaaggtaggcagtgttaccataaggaggttggaagtgacacagataggctaaggaaggggacttcagtaatcatgcagcaatggcctggaaaagggagaggctcatagtagggagaccagtttggaggctgccatagtgttctactgagagagaaaaagacttgaactcagagcacggtcagggaaggtggaggggcagggtctgatttggaagtgttttgttttttggttttgggaacaaggatttggaaacctcttggctccgtagatgaagaaaggtgaaccaaggaagactgaagtttccactcaaggaaacagtaactcagggaagaaaacacaggagtaggaataggtttaagagaatgacaagcagttgtgttttggacttgtttagttcgaggtgacatctttgtagggatgtctagctggtagctgcaagtataggaggaggctggatgtgtgcatgagtttcttggtaaagatccatctgcagtctcctgaagatgtcacccagattgccctgccatcaccccagggccttgagtcactcgcttctcttggtgtctaggcaggcttgaagaaaatcaaacagtacaaaatcatgcaaattcagacctctattccaccccagaggaaagtcctgctagcagtttttgtgtattcttccagaaatttgccttgcaacgcgtttgagtatataaataatcccagaaaggatgggccagacactagcagaaactcaccacacacactgcactgggcatgcagaaactttgcaaaatgtactggtgtgtgctgtcactgcattcctgggtttggaggtcttctgtgtccccagctgtcagtattgcccacaggctgaccactgagctccttccacagccggcccatatcaccctctttcgaagtgtgtctgcaaggctagattattagagtaatttaagtgtttctgctttgtgttttctttaatgaatttttttatgatgaagttcttgttttaaaaatatacagtggtaattaacatgtatgcatttttcttaaaatgacccccccagtccctcttcggatgtgatcactgttaacagtatcgtatatagaccctgttctgtgtggggcgggcagagggctggttagtgggtggaacatgcatactcacaaccatatttttcacatgggaaaatataaaggtgacaacaaatctcctggactataatctcatcaagcagacaataatctctgtttcaaaagtggacaaatacatgctgattttttaaaaaaaattataatagtacagaaagatacaaaaataagttaaagtcttcctaactctcctgcctgtgccctccactgggcaaaagtccctgtccctaaggtaatatctgttaacagttctccttccagaaaacttgcaatgcaaataggaacattttgtgtgtctgcctctgtgtgtatgtgtttacatgtcttttttttttttttttttttttttttttttttttttttttttttttttttgagacagagtcttgctctgttatccaggctggagtgcagtggcatgatctcagcttgctgtgatctctgcctcctgggttcaagtgattctcatgcctcagcctcccgagtagctggaattacaggcgcctgccaccacacccagctaatttttgtatttttagtagagatggggtttcgccatgttggccaggctggtctgaaactcctgacatcaagtgatctacccgcctcagcctcccaaagtgctgggattacaggtgtgagccactgcttctgcccctgcacatgtctaacgcacacaaaagagattctgctgaacacattttttatgctttttctttccaatttaacatatttgacatctttatcagcttatatagctttatttttttaagaggttattggctataaagggaaagtgctttatgggtgcttctgttgttatttaattggatcctgttgatggacattgatatcatttctaaattttttagtatcctaattaatcctgtggtgagcatccttatacagatatccttgttccctcatgaaaatatttctggaggatggaaagaagggaaattttaaaaattatttgtgtaaacattatcgtttgttagtagaatgacctcaggagagattgtagtaatttatacttccccacatgcatatgaatgccttttcaatatattgtttcaaaattggatatcatgaaccttaagagataaatatatatgtatgtattttttttttttttttttttttggtgggggcatgtcctgttattgacagtttgttttggtggagggatgtcctgttattgacagttatcgaatagaactttgtcagttccttcatgtaagggatgaatttggtaataaaacaggtctgacttcagttatggaactgggaaagctggaccttgatgtggaggtgggctcagacatgctgtgtctgggcaggtatctcttgggaagcagtgtcatccctgaacagaaacatggatgagccgcaggggacggtgctgagcagaggggctggccgtgggtcatctgcctcccttggcctagaaggcacaagggagctttccaccttgcctttggttttgagaatgcagaagctactaagcaactcacagtgtgcccagggtggtccagctgaaggatgcgaaatggttcttccttttccagccaaagatcttgaacctcccaccccatgacaagcattataaaattcacataattttgataggctggattccttttctgtagcagatctttcctcagaacagaagtttgttttttttttttaacctaaattacctgtgagttttattttttaaatatggaatctgttttttggacacctccttgtcatattaaatgttctgttattaattttgagattttaatgtaaattttaccccagcaaattaattttgtttctcttgctctctctttttttttttttggcatcctttcccgttgtatagtggtgctcattttatcatactgcttttatatgacttttcttttgtgaacagggatcttgttcacttttccttttttaaaaatttttttatttttttgagacggagtcttgctctgttgcccaggctggagaacagaggcacaatctcagcccactgcaagttttgtcttccgggctcaagcgattctcccaccttagcctcttgagtagctgggattacaggcgtgcaccatcacgcctggctaatttttttgtatttttgtagagatggggtttcactatgtcatccaggctggtctcgaactcctggactcaagcgatccacccgcctcagcctcacaaaatgctagggttacaggcgtgagccactgtgcccgagccacttttccttttaacataaaaacattgatatcctagagagggcactgtattttgggtacatacaggttcagatcacggaagagttgtattctatactttttttcatcattcttagttcagtatgatgtattttataatttcatatgagaaactgtaacaatgggcatgtgtcatccagcaatacctactcataaatcatattaaattttgatccaaacatgggagaaactgaagttttctctgtgtacttggatgctttcagaggcataaaattatattaccatgtgaaagcaagcctacaaaattcctcaggtggtccactctgccactcaaatgagagccagacttacagtgcacactctacaaacggacttccagctcgtcagggtattttaagtgcctgaatatgcaaggcactgtgccagtaaaattactcagtcctgaggatagagcctgttagaattattttaaaatctgtacttgaagtttatttcctcagtattccaagatattttatctggttgttctctgagtatttcacacgtagctagttacatataggtgagatggtgatgcttgtgcctggtgtggatgagaaactgagcctggcagacccgagattggatttcctcttctgactttgcaagtgtggctttgctttaataatagccctcctctttttctgtattcctcttttctccttccagtgtggcaaatatgcatcaatcaaaatacaataacctgtggaaccattttttctaaaataggaaggtggtgccatgggctattgattgttgagggtagtcttcagagcctgtcttataaatctataataattccccccaaattaatgtgctagttagaaccctagaattgcagcactgaaagtgaattttagaatcttttccaactttttaccaagctcagaaagcccttttattggacctttgtttgcctcatggtcatctggtttctttatgctggtagtaacaggaaccttactaacctacaaggtgacccagtccatcctgggcagctgtgatcattggaaagctctgaatcattcatctggaagctgcctgtggcagaatagtacagaacatatgcattgcacacactacaaaactgctttaaataagtgttccttttcattgttagatggaagtgacccagggcaaggatcatgttttatgagccagttttctcctagtgccttgaacataggcacttggtagtgtttagagaatgaattgtcttttttttttttgagacaaagtctcactccattgcccaggctggattgcagtggcacggtgtcagctcactgcagcctccacctcccaagttgaagtgatttttgtgcctcatcctcccgaggagctggaattacaggcatgcgccaccacacccagctaatttttatatttttagtagagatggggttttgcgtgttggccagatggtctccaactcctggcctcaggcgatctgcctgcctcagcctcccaaagtgctgggattacaggcgtgagccactgcgcctggccagagaatgaattcttaataagtttcttatgacttcagattgactggcagttgtgctaaatattttttgcctttatttgaattagaaaattcgtaagggggccttgagagtagatgcagtcacatttaggagatttttcccccccattggttaaaatgcagtttttctatggatctgctttagaactacaaataaactccgatcactcacagcagactacgcaatgagataagaagcagtccatttgttctgtcgtttattcatggccctcatctttgccagccaacctgtgcagaagagcacagcaaagcataagcttcctaacagctattcccattcagctgctgtcttcaagaagcagaagggtttagataaccttagagaacataatcaaacctgggaaactcaaatcaaaacaaaacttcgaaacggaagttgaaggtcctgaggtacccagaggcatagcaaggaaaacgtccccactgggatatcttctggattcacctacagacctctctggagttttaagatccacgttttatgacatattgcatagcaaacaggccgaacgctgttgtaaatcatcctctacgaaaggcccaggttttgaaactgaaggcctgaaaaggctcctgcttaccagctgtgtgctgtacctgacacactgaagcctgagagtgccagtcacctgtcagagggaacacagctgccctcaggcagaacctgagtctagaactcaaggtttttgactcttaggctaaaaataaaaaatcagaaggaggaactatggattgcttaatcagtcacattttcactttctaaggtttcttgtagcaaaagttatagtctttggggattgggatgtagacacttttttttccttccctaaaacaatttttggcctgccagtttttcgagcttcctgctctggaccctgaagttgccatgcagttgcagacatgctcctccttcaaggctctgttaagctgtggctgcccttccttaccactgctgtgccccaggccaaaccccctgcccctccttcccctaaggcactttgcacctgttgctccgagccttctggtctatcccagttggtagagtccctgtgcttacctctgtggctcagtcctcgtgggtggtcagtgctctagggaaggtgagctgaccacttcactttcccttcccagccatagctcttcacagcctcaccaacttagaaaggaatgctgcttttctctctgtcccccgtcctgactatgttcaagtcattgctcagcccagtgagtttgtcctttcttccagaccagtagttttcccccagtccctcaggcttcagcccttgaaggcatccttagccccccaccaccatgatagtcaggcgctgcgcctatccgcagggtgtgggtatgtgtgtgtcttttgtttctggagcccattcctttccttccaccagcctctaggccttcatccaatccttttgcaactcagtgattcatgacttttccctgcatccagtctagtctctttgctggtccattgtttccatagttgccagtttaatcttcttaaaatgctgcatttttgaagtcagtctcttttggtccctctcagaaacatttaaatagctatctgttgccacagggggaaagcttgaacctcttagccagtcattcagagcctgccctctgctggggcctgctttcctctacagatgcttctcccactctgcctgccacagcccttgtagctggctgattgccctgtacctcgcaggctctggaagtcttcagctccttcatggagcctttgccagccattcttttcaagactttgctgttgttcactgcctgatttgttcatttgacacttaattcactgagcaaacattatgaaagatgtactgtttgctactgtgaggaatggatccccaagagataagagggtcagtccctactgccaggaaacttgcctgtgtcacctgggttcagtatcttgtgtctattagatcagaagtggaaaggcagaggccagcccgtatgcttgttttattttatttaaatcaccagcaccccagcaagtgttttgcacaggaaatttctcattatttaattattttgggttttttgattaaattctgtacattcccattttagcttatcttgagttataacattaaaattaaggtagtcatcagctgaattataagacttaattagataagattatttaagatagtgatttctcattagattggccctgttcatattaacttttctgtttttttcttcagtctgcatgaagaaatcagtgatttttatgaatacatgtctccaagacctgaggaggagaagatgcggatggaggtggtgaacaggatcgagagtgtaattaaggagctctggcccagcgctgacgtgagtcccttcctgggtagcttatgcttcggacagtccttgtccacgggctagaagcctatctgctggtatctcatgctagtcctcacatgcaagtagaagtgctctgtagagttgtggtctaattaaattttaaaggcaaacaattttctgcagtctttagaattgaggcttcctaactattttcattggattggatgactaacaactattttttttttgtagtgctaatagcaactactaaaggcaagctatccttagaaattattagtgtaaagagaagaaagacaaatcaaacctcattgttgtagtggtctgttattggatatgatatatcaaaacctcattactacttagttccagcctgccagggtaaacattatataattgtttacagctaaatgaaaatgtcaagtaagaacttttgtcacttgaagttcatttcctttggctaatgcacgcataagtcttttcttatttctttcctgaaattgccatttttcatctctctcagaccagctaattgccttttagacagctcccagtcagtgaacaaaatgattactcaggatttcttcttggcttatttgtcgtttttgttactggtactaagtcttttgttttttgtttttgagatggggtctcactctgttgctgaggctggagtgcaatagtgcgatcacgacttactgcagcctcgatttcctgggctcaggtgatccacctcagcatcccgagtagctgggactgcaggtgcacgccaccacacttagctaatttttgtatttttttgtagagactgagtctcactatgttgcccaggttggtcttgaactcctgggttcaagcaatgtgcccgccttggcctcccaaagtgctaggattacaggtgtgagccaccacacttggcctgttactggtactaagttaatacgtcactttttagggcactttgagggcctgttctacaattttgtgtatgcaaagaagtacacaaaataatactaataaaatccattactttgtgtttgtagcttttcttcaggcactgtcctgggtggtggtgggaagctagggaaggtttttttccaattggcaaaacaaagaagtttcattgtatgtaaaacttgcaagtatatgacagtatgtatatgacactgtaggtaaagggaaaaggcaagggtactaatgttttatgagcaatgaccatacatcgcattctttctcctatgtgatccaaatcagtggttctcagctagtggctattttgttctccagggggcatttggcaatgtccgagacatatttgattgtcctgactgggtacgcactgctagtacctagtgggtagaggccatggatgccatcagccattctatgatgaacagtataggcccttacaacaaagaattatccacccccaaatgccaatgttgagaagccgtgatctaacttaacccttatctttcttaggtggaggttgattatctatctatctctttctctccagccagccaggcagccatcatctgtctacctacagatgaggaacatgagcttgtggttaggttcccaggtccatctcgcctcagaggttgaactggtttcactgtttatcatttttttcccccgagatggagtctcgctctgtcgcccaggctggagtgcagtgacatgatctcagctcactgcagcctttgcctcccaggttcaagaaattttcctgtctcagcctcccaagtagctggggttcaggcgcccgtcaccacacctggctgatttttgtaattttagtagaggtgggatttcatcatgttggccaggctggtcttgaactcctgacatcaggtgacccacctgccttggcctcccaaagtgctgggattacaggcgtgagccactgtgcccggcctatcctttttttattacaattacctgcatacatatttctgcctgagttccaccgttctccatgggttgagatggaatgcatcccagttttatgccacagcatgatgttacctgatgttctttgtggaattgacctaaaggccctcacttgccctacagttaaagtagtctgatcccaatttagtaatctattcgaagactcctgcttagagaacaaaaatgaaggatttgtgattgtgtctctggataatgagggaacattagtgatctgaactgcttctgaaagtttcctgtggttggctttctgtatccacaggtaccacacctccatattaaaccaacaatggattgaaaatattcagaaaaaactataaaaataacaatgtaccaataaaaacaatacaaattattttaaaaatacagtataacaactatttaggtagcatttacatcatacttggtattataggtattataagtaatctaaagatgatgtaaagtacatgggaggactagcataggttgcatgcaaatactctaccattttatagcagggactcaagcatcttcagattttggcatggtgggactggaaccaatctcctgccgataccaagggacaactgtattttggtctatgtgtttcatattgaaccagataagtttaaattatattcagaatgtctgcttgtgaaacagaatccccgcttcatgaagcttggggttagaaaaaaatgctcttgtcataccaaaaagtaccagtagagggtagcaaaaactgacatttctccatatcttggtgactcaatatgataacaacttctgataactcaatataataacaacttctttttctgtttcaggtccagatatttggaagttttaaaactggactttatttacctactaggttagtacactcatgaatctttcaaaggacttttcttagagtgtattcattttggctgtcaaatttgtaaggagtagaaacaaaacaaatttataaaacaaaatggggctgggcatggtggctcatgcctgtaatcctagcacttcgggaggccaaggagggtggatcatttgaggtcaggagttcaagaccagcctggccaacatggtaaaaccccatctctactagaaatacaagaattagccaggcgtagcagtgcgcacctgtaatcccagctactcaggaggctgaggcaggagaattgcttgaacccgggaggtgaaggttgcagtgagccgagatcgcgccactgcactccagcctgggcgacagagcaagactctgtctcaaaaaataagtaagtaaataaataaaggatttaccagcatttaatttgatttaccttgaagtagaatatcacttcacatcatcttaccaagacatagatggtacagagagatggaaaagggatcatgttgcaatggaatcaattagttactaattttagaaattgactgcctggcagagtattgctcagtcccataacttaacccactgacacagatgttaatgtagtatcatgataaaatgtctgattatatatcctcttgaatgtgagttcccgctgtcttgctcactcactcttacactcaccctcgctttcaaattaagaactcattctactagttatggctccagcatcctgatccagaaattcagggtacagatctcttctctgagaaagatcttggcctttcaggactgttgttcagtttcagtcttctcaaatgagacctcttgtgacgcacagccttggaggctctcttttgggaaatgataatgtttctccaaagggtgaatacttgctctctaagaattgaaattgtttgaacattccatcatggttattattattattaccttaaattttaatctctccagaataaagtcagcatcatgtttttccatttgagcttgatttggtatactttaccccaacttaaagtgtgctgaagtggatggaccctggcaatttccgttcttctcatagatgcccttggcctgcaaaagtcataaaatactcaacttcgagttaatatttcttatttaggttgtcagcatcagtaaaacatgaaaaatcacctttcttaaaaaatttaattaaattttatgaataggtagtacattcacatagttcacatttggaaaaggcacaaaaatcaatacagggaaaagtctcagtcccacctctgccccctggttctccttggaacagccgcttttaccagtttctcacatatcctttcagagatatctgtgcatataaaaggacatgtgtgtatattaacacaaatggtagcatgctggatacctgttctgcatccagcttaaagcacttcataatatttctgagttgcaattaatctcatccggataggaaaatcattatgtctagtaccacaagcgtttattaaagaaaatacatgaagtgctttttgtttttttttctttgaggttttacttctttcaaaatcaccctatttcctgaggcctgaattctgtgaaatgactgagaggaggagtttgttaaaatcaacaactactatttcccttctccacaaaaccattatcaccaacacatttagtcttcgttggccagggtgggaaataggttttaattgtactaatgaagtctataagcatgagtgtcagttaaaacaagtttccaacttcttccgaccctcttgtatatgtattctgtgttcagtgacatcgacctagtggtgtttgggaagtgggagaacctacccctctggactctggaagaagctcttcggaaacacaaagtcgcagatgaggattcggtgaaagttttagacaaagcaactgtaagttctgcagcatttcatattaaaatccttagttatttacctatgaaacttgaattaaaattaaagtttggtgagcacagttgcattgcaagtgagtgattctttcattttgttaatgtcaccgtgcttgcacataaaaagttttctggttgtccacactggagtgtgaccatacaatctcggctcactacaacctgtgcctcctcggctcaagtgatccttctacctcagcctcttggggagctgtactacaaacacaacctgccatgcctggctaattttgttgtattttttgtagagacggggtttcaccgtgttacccagactgatctccaactcctgggctcaagtgatccacccacctctgcctcccaaaatgctgggattacaggcgtgagccactgcacctggtctgcatttcttttcacagcagcaaaatatgcaattttattatacacagtactcactgtagagatttttgtttgttttattcattttttttagagagatacagtctcactatgttgcccaggctggtctctaactcctggactcaagtgatcctcccacctcagccttatgtgtatctgggactaaggcgcaccctaccacgccctgcttatttaaaaaatttttttttgtagagatagggtctccctgtgttgcccaagttaggccattttttgaaaagaactgctgatagctcatgtaaataatcctgtcagctttttagaataatttttatattttatcttgtcaggttgttttttgggctatttgcaaaactgaccagtaatgcaagtgggttgtagtgtacaccttaagaatccagcaattttcttattagaaacagtttgatgatacaaaacatttaatacctggcattcctagttcttcatcttatactcagaaagtgttctccaaattattgaggaaggtttttgttcattttaaaattatcattataactatatgtcaactaataaatgagatgatgggcatattaatttatttaactgtagtaatcacttcagtatgtatatcaagataagtatatcaaaacatgtacaccttaaatataaacaataaaaataaataataaaaaattggacaccaaacaaaattctcggttgatagaaattatactgtaatatactgtatgggacccagtgctaaatatgcagcatatagtatttgtagcagaccaggtttactggggtgtgccatatttagaatactcagtgttcttatgctctcatgagatgatggagacctcatgtctagtaggcttccatcccctgattttatcatttaatctggttaaagcatttacattttacctttcttctctttataggtacctattattaaattaacagattcttttactgaagtgaaagttgatatcagctttaatgtacagaatggcgtgagagcagctgacctcatcaaagattttaccaaggtcagagaatttagcgtttatacaacaaaactattagaaacgtaattttaagattctgttgtggtggtgttctaatatttttatatgcatgttgctgtctctctctctctcttttaaatagagctagggtctcactctgtcacctaggctggagtgcagtggctggatcatggcccgctgcagcctcaaactcctgggttcaagtggtcatctcacctcagcctcccaagtagctgggactacagacgtgagccactacacctggctattttttgtattttttttttttttttagtgttggggtctcgctgtgttggccaggctggtctcttaactcctggccttagcctcccaaagcactgggattacaggcatgagccaccatgctcagcctgcaccttacttttgtatgcaacggttttgctttctttgaatctgcttgtaatgatcagtgattaacttataatgtgacctcaagtaagaattaaaagttgagaaagcttttgaagaaattgtctgctctagatccttccttgtagagacagaagagatggaattctactacacagttgattccatctgtttttaaccttcaggagttcagattaagaacctttcctttaacccatttcccatatgccccaagaatactgtgcgggcagtgagctgcactttttttttttcttttttcgaggcagagtctctctctgtcacccgggctggagtgcagtggcacgatcttggttcactgccacctccgcctcccgggttcaagcaattcttctgcctcagtctcatgagtacctgggactcgtgcctgggacgagtaccaggcacctgccaccatgcctggctaatttttgtatttttattagagatggggtttcaccatattggccaggctggtctcgaactcctgaccttgtgatccgcctacctcggcctcccaaagtgcccggattacaggcgtgagccaccgtgcccagctgtacttttttttttcctaaacaggaaataggttaagagttttaagagccttttctagatttcaatccctaaattacctttaaggtgtttcctacaggcttccttacttctgttttgaaattatttaagtttatttctattctgttttcttccaagatagagaataatttgtcaccatcatctgtggaacattttacatacttaggtagttgtcagctttctcacctctaacctaagccattaactcctttggcttctgttagaatattcacaattttttttttctgtagcagctctaaagtttctatttcttcttttttgttttttaagaaaaaaatgttaactacttgatgttacaagcattatcatcttgcataaatgtatggaagacagaaaagcagaaaaataaaagaaagattatccataatcgcactatattgggggtgtgtgtgtgtgtgtctgtctaatattttctttttctggaaaaaacttttaaaaattgaaattcatatgcatgataacattcatcagtataaagagacagtgtaaagtgagtcacccttacaccatagatacttagatcatttttacagaatttctcattgccaattattgttttttgcgttgcttttttatgttctttaaaattataagcaaaaggagtagcacattatacacacattgtcttataacttcataaaaacttaatgttttggaggtttcttccatattagcacatacaggcttgctttattctttttgttggttacacaggcagtagtcttttataaggctgtgactgcttgatttagcagttcttcagtattgttccagttttcttttgctattagaaaaagggattgatgaatatacttccatacatgcatcttgctttacacatgcaaaatgtttgtagaaagattcccaaaagcaaaattttgaggtcgaagggtatatccagataaaattctgttggatatttccctaattatttattctttcatattctcattttctctctctccctcccccttttcttctccctccccctcttcctctatccctccctttcccttttctctctttttctttccctcccttttcttttctcttttctcttcttcctttttcttccttcccctttcccttttccttccttctgcttcctttttttcctttctttcattttttgacaccgagtctcactctgttacccaggctagagcgcagtgatcatggctcactgcagcctcggcttcttgggctcaagtgatcctcccaccttggcctgagtatctgggatcacaggcttgcccaccacacctggctaactttttttttaatttttttttttttgagatggagtctcactctgttgcccaggctggagtgcagtggcgcgatcttggctcactgcaacctccgtctcccaggttcaagcgattctcctgccttagcctcctgagtagctgggattagaggcgcacaccaccacgctcagctaatttttgtatttgtagtagagatgtggttgcaccatgttggccagggtggtctcaaaccctgacctcaggtgatccgccctcctcagcctcccgcagtgctgggattacaggcgtgagccactgagcccggccacttttttattttattttttaagtagagatgaggtcttgctatgtggccacttttttttttctttttttttaagtagagataaggtcttgctatgttgcccaagctgttcttaaactcctgggctcaagcagtcctccttccttgacctcccaaagtgttgggattacaggcatgaaccaccacacctgacccctaattgttctttgaaagggaactgtatctagactgacttaaccaccatgttttgttttgttttttgagacagagtcttgctctgtcactcaggctggagtgcaatggtgcgatcatggctcattgtaccctccgcctcctgagttcaaacgattcttgtgcctcagcctccagaatagctgggactacatatgtgtgccaccacgctgggctaatttttgtatttttagtagagatggggtttctccatgttggccaggctggtcttgaactcctgacctcaagagatccacccgcctcagcctcccagagtgctgggattacagatatgagccaccgtgcccagcccacaatgtttaaaaatacttatttctccatatttttgttctttcctatgcttgcttagtttgatacaatttgcaaaagtataagcttttttttcttttttatagaagccatgcgtgttcattgtaggacatctagaaaacagagataagagtaaagaaaaaaaaatggaaatcaccggccaggtgctatgtttcacacctgtaatcccaacactttgggaggcccagacaggcagatcatttgagcttaggagttcaagaccagcccgggcaatgtggtgaaaccctgtctctacaaaaatacaaaaattagctgggcatggtgggctgaggtcggaggatcacttgagcccaggagctggagattgcaatgagccaagattgtgctactgtactccagcctgggtgacagaatgagggggaaaaaaatggaaatcactagtaattttaccaccctaagtaataatagctgttaagacttctttgaagatgttgtgcctgctttgtttccctccgtggccccagcctatggcatggtttacagaggagtgaatgaatatgtgcacagcaaaaggtggactcattctgtacatacttgcccactcaggtgttctctcgggtagccctgcctcattccctgtgaagcgtggaagggaggggtggtctgtgtgtagtcatcagcccatgtgcaagtcagcaggcaggactcttgtttgccccagggctgtggcagaataatctaaaggtcgctagtctacagtggtacatcaccaagaaaagtgattcttaaaaatctcactgatttagtgctttaagatgttggttactttgtccttgtactctttctattctctgtttacaaatgaatattagagggtcatggtcacaaatgagcatcatcagttacatgctgttagtgtttctatcctatagcaagtacttttttttttttttgagatggagtcttgctctgtcacccaggctggggtgcaatggcacgatctcgcctcactacatcctctgcctcccgggttcaagtgattctcctgcctcagcctcccaagtagctgggattacaggctcccaccaccactcctggctattttttgtatttttagtagagataggcgtttcaccatgttggccaggctggtctcgaactcctgacctcaggtgatctgcccgccttggtctcccaaagtgctaggattacaggcatgagccaccatgcccagccctgtagcaagtacttagatactattattcatttgtacatgtcttacaatttaagtataaggggagaaccattcattacctatagtttacttttttttaatagcttactcttaaaatagaaaattaagtatgttgtatatctctaccaaattttataatgtaaggaccaatttatgcccctcttaatgcttagatctgttgctgatacaggaattcattgaaaatacaattttctttttcagaaatatcctgtattgccatacttggttttagtattgaaacaattcctattgcagagggaccttaatgaagtatttacaggtggaattggttcttatagtctctttttaatggcagtcagtttccttcaggtaagtcatatgggtatagcatgctagtgcacactaaaagcaaaagtgatcaatcagctgggaaacattttggaaaaaatcgaaatcaacctgtaattgcattgctttccttgattacttaacggcttttccctttaaactgggtacattttatcatttagcaaatatgtatttttaaattcctatgaaagaatatttttggttttaaatcccatacattctagtatttttgagacttttcactgcaaattttaacatgcaaaatgtacggcctggtttccataagcataaatagtataaatgccaacaataagaatgtcttctaagcagctaaatcttgtaagtttagttggaattgagaccagctatttgggtaagcgaattagagtcttagtattgtaagtgggtatgtttatgtggcacagggttgccaactgcctgagtctattcgtgagtcagaacgactttgctgatgtgttgggccaagccagccctggttggcagcctggtgcagccgtaaaattcagccttacaaacagtctcccgccattcccgcaccatgggactttagtgttgtgtgtaacaacagtataacctgctgttagcccattatcaactgactgctatgctaaaccaaaattataataatattgcttgtagaagttagaatataatttattccccctctccttgataatttagcaaaaatccaatataatttcttcttttctgcttttagttacatcccagggaagatgcttgcatccccaatacaaactatggtgttctcttaatagaattttttgaattatatggacgacacttcaattatttaaagactggcatccggataaaggatggtggttcatatgtggccaaagatgaagtacagaaaaatatgctagatggctacaggccatcaatgctttatatcgaagatcctttacaaccaggtattgaaattaggtaaatttgtgggcattcaaagagagggcactgtcagtcaccttattatactttaaattctctttagatgaaaaatgaaggaacaacttctaattgttattcttttttcatcgaaatatttcatgagcaaacatactaaaataaacagacacagacaatagaaaaacaccttggagacttccagataagtagggagtagaatctgtttaaccctaaaagcatagtagaaaaggcattcacttatttggatgggttcatgtttggtggctgtttctccttcttgggtccttattgccttgattacaaccaattgtcagcaattaatgaggctttaatgagatgattctgaagtcctgagaggcagcaagcatagtaatatatctttgaattcatgagcagaagggtgcaaggagacaatgtattttctttttgaatttctcctttcctgtttgattttgcatgtctctttgtgctttttccagcttcatgtgggcttgaaagtaagcagaaagtaaattccttccatgcttttctgaagttctgtttgcttgcttgtgtcctgatttttgtgagcaatattttttcttgatataattgtaaaatagattctgcgttattggacttcagtggaagtgcttttagtcatttgctttaatgtgtaaactttgaaaatgagtaaggaaagggggtgaagagatagagtagttgcctaggaaccattttctggcttattgagctgccttataaacattaatagttctatgtgtttattcattgaggaaacattacattgattgggagcctgctctgttcaaaagtattgggccaaaggacacgaagacttttcagcaagacgatccttgctttttaggggctcataatttagagtgagaaatagatatatagctaatataaacccaaaaaatatagaagtatttctgatgtaacttggggtttcactcttaggagtgaacagggcactatttcttttgtttgcataactgtttatgtatggaatgggataattcttgatgggccagaatacattccggcaactgatacaccataatgaagtaccaactgcatgattcacatattcagagactggggagctttggggacagctcacagctcagcttccaggcacaactctggtgggataactatggcccttgctctcctggaagagagtcatcaacatttagtgcatattaagcacagtcaggcttactatgttacgtatatttcttttaaaggtaacgatgttggaaggagttcatatggggccatgcaagtgaagcaggcctttgattatgcctacgttgttttgagtcatgctgtatcaccaatagcaaagtactatcccaacaatgaaacagaaaggtaaaagttcatctataaccagcccattgtgtcaaaattagttgtggcttcttatcttcaaattaatgttattccctccctctccctttctttttaaacacatgcagcatactaggtagaataattagagtaacagatgaagttgccacatatagagattggatatcaaagcagtggggcttgaagaatagacctgagccttcatgcaatggtaagatattttccttggtcgattgactgagtattagaggcttttctgtgttgtgtgcgtttaatgggaagaaacgttttccaatcttttgccactctttcaggaaatggtgttaccttgatagtagatactcagcagttagataaatgtaataataatctatctgaagaaaatgaagcccttggaaaatgtagaagtaaaacctcggaatctcttagtaaacactcttcaaactcttcatcaggtccagtgtcgtcctcttctgccacacagtccagctctagtgatgtagtaagtatgaaagcctcggctcttctgaactcagatgcatgcacgttctcttgctggggttaacactgtctcgaaggctaaggctacttcctttgcttacatgttactgggatattttaataactttcatgcttgtacattttctcaacattttgttatgaaaaagttcaagcatatagtaaaagtgaacaaattttagtgagcattcatgtactcaccagtagattctgctattaaccttttacttgcttatgtcatacctgtctatccatcactctatccattaattcatcttattctttgatccatttcaaagtagattacagacatcagttcccctagagtactgtagcttgtgcatccttgtagccagactccagtatttgtttattgttttttccttttttttttttttgagacgggatctccctctgtcacccaggctggagtgcagtggtatgatctcggctcactgcaacctccgcctcccatgttcaaacgattctcctgcctcaacctcctgagtagctgggattacaggtgcgtaccaccatacccagctaattttttgtatttttagtagagacggggtttcaccatgttggtcaggctggtcctgaactcctgatcttgtgatccacccgcctcaacctcctaaattgctgggattacaggcatgagccaccacacctggcctttaacgtttttcttttcttttcttttcttttttttgagacggagtcttgctctgtcacccaggctggaatgtaatggcatgatcttcactcacctcaaccttcgcctcctgggttcaagcgattctcctgcctcagcctcctgagtatctaggattacaggcatgtgccaccacacccagctaattttttgtatttttagtagagatggggtttcaccatgttggccaggctggtctcgaattcctgacctcaagagatccacccgcctcagcctcccaaagtgctgggattacaggcgtgagcccagctgttatgactttttaacaccatagttagttttgcctgtttcagaatttcatacaaatggaaccacatagaatatagtcttgtgtaaggcttctttcactcaattttttttcagctttctggttgaattttttgttgttgttgttttgttttgttttttgagacggagtctcgctctgtcgcccaggctggagtgcagtggcgcgatcttggctcactgcaagctccgcctcccgggttcatgccattctgcctcagcctcccaagtagctgggactacaggtgcccgccaccacacccggctaattttttgtatttttagtagagccagggtttcaccgtggtcttgatcgcctgacctcatgatccgactgcctcggcctcccaaagtgctgggattacaggcgtgagccaccacgcctggccaaatttttttttagttgagatatagttaacataaaattcagcattaaaaatgtacaattcagtggtttttagaacatattcacaatgttgtgcagccatctccagtaattctagaacatttccatcaccccaagaagaaaccctgcatttagcagtagtttcttctaattcttccttccctcccttaacctctggtaacctctaatctactttctctttctatcctgatagaattttttttgttcccccatcctgatagaatttatgtgtcaattataatgtaagttaccttttaaaatcaaagtgaatttgtagtgtactgatttgagatctaaagcaggcttacctgtttgagtttaactttattaagtgtaggacatgaaaagtaatctaaatattgtatgttgttgatgatgaccatgtgtcaatatggaatcataaatcctcctgtgcagaatctccctgtgtgcttttttggttcctagagcagtatgctttggaggacagaagccaagctagatgtcacagacacagggagatggagtgttggggactgagagaatgtgactctgacatgctgggtagagtgccagggccagggtggagacctgcagagagacgtagcattgtcatggcccatgcagcccagaaataggtggagctcagcccactgtcgcgggaagtccacccccacccacaccagtatgtttggttagaatgatcactgatttgtcatcacagactctcagagattgaaccccttaaacccatcatcttgtgtctggctgaagccagggactaggacctaggttcctcactctttaccatactctttcattttctataaataaaaaaacaaataaacttagacctctgtgagctccttcaaggtcagatgtgggcagtggatttaacaatgaacagaagctctctgataaaatcagtcattttaaatgtttggaggaaaatttaaacaaacagttaattttttgtgtgcttcttttaactcccaaatgtttaaatttagtccagagagtactttaaccaaaattgtttttctttctgaatattgagtatctaaattactaatatgtcacattataactcacgtgacttgtgttaggattccgatgcaacaccatgcaaaaccccgaaacagctgctttgccgtccgtccactgggaaccgagtagggtcgcaagatgtatccttggagtcctctcaggcagttgggaaaatgcaaagcacccaaaccactaacacatccaacagcaccaacaaatctcaggtgtgtggaacgtgggtttttaattgttagtatttgatacaaaatatttagaatttcccacatgtaaataatatgcagcatgggtttgaagaaaacgctagattgaagaacaaacttattttattctaagaggttccaacacatgacagtgcttctaggaacaggatgtcctaaggatccttgtgagacaccattgtaacataaatctcttcaggaatctattgactggtccttataagatgttccagccaaactaccatataaaaagtgtctcagttgtacatgaaataagctggcatgaaggttttgtgaggcctcatggcagtgtgcatatctgggaataatgtatccttttctaatattttaatgttcaataccttgttgctggtgttgaaatgatcagctggctgtcaggcgtggtcagttgattaacattagcttggacttaaaaggccacagagatactctagtttaagtttttttgttgcctagaattgtcattaactgagtaatgactcagagtgaggggaggaagccattgatatggggctctggcctaaggctgggtcactcctcactatagctgggaacctgggaataggcctcttggctgtaaccttgtgtctgatttgactcactgagttcactttacctacgcggccttagccatgtatgccagacacagacttatcacaaaataccagttcaagtgacagggttgacagaagggactgaggtcacgagaaagccacaggccatgagtagcaggaagggagtagccacctgtgctgacccaaacctaccagtgtgcctgtcatgcccaagagcctcttcccgctctgtcacttatgatgtggtgtttgggttggtaagtttcttaagaaaacctttgcatcccacacactgttaagaaggcgggcgagtggtctatgcttttcattatttccattaaaataaagtaagggttttagagctaaaaagaacccctgtaacagctttttctgcccactagataagtcagtgatcagtaaggtaacaatctagccagcatattcctagttttgaaagcttccccaaatccaggtgtttgagaacactctgcttttctgcaatactgatgtctttgtggtcgttttctgtttctgcagcatggatcagcaaggctctttcgttcttccagcaaaggcttccaaggtacaactcaaacaagccatggttccttgatgacaaacaaacaacatcaaggcaaatccaataatcagtattaccatggcaaaaagaggaaacacaagagggacgcgcccctctcagacctctgtagatagtcagcgctgcgcggtggactgtcttctctgtgcaatgatctcatgctcaggacagttgcgcagggactcctgggagatattcaggagcctcacactgttcagacgttgacttagcaactgcgttttttcccagctcgccacagaatggatcatgaagactgacaactgcaaaaaaaacaaaacaaaacaaaaaaaaaagcaagcaaaaaagagggaaaaaaaaggctgcttatttgataagtcatatgctacaacagggtcattttaagatttaaagcttgaatgtaaaataaatatatttctcattggctttatgcagagttatagggaatagtattcagtgttggtagggtgatagaaacaaaaaacagtatcagaggatgaggtggggaaggaaaacaaaggtatctgataggaagtccagattccaaaggggaaagtgatctgtgcatgttttttttttaaatatttttgcatatatttaccattttattgtgtgtatatatagaagaccatataggagattgatatttgtaatagtggatttgttaataatactttttacataacattactgtttaaattgtaaacagattttttctcaggattagtttgaaaaataatctaaattgtcatcttaacatccatatatagggaagtgattagttctattactcaatttgtttttctcagcattgaaatgacttaatagaacccttgtgtcctgctgcaaaaatttttcctctctaaagaaaaggtttatggtggcaaatgatgtttattttattttgtaaaaaaaaaaaaatgtactatgtacttttgtgtaaacactgaaaaatctctggtcatctccgagaattaacttgcaactgttttctatagtgctgtcgtcttgggcaatgggcaattacatgactttgtgtttgcttcctttgcagtcttttttttttccccccatttcttcctaataggaaaaaaaaaaaaaaaaaggtcacccatgtctggtctcattcctgttgcagtgaaacttcgagttccacagactttgcatgctggcttctctaaccctgtgtgctgcgtgtgcctgtttctcatctcttattctttttaaaattcatgcttaactactgtgggagaataactgtaaacagctttaattaaatcatacttataaaaaactattttcttatattccactctatgcttttggtattgttgatctttacaaattaaatggtctttgataatggatctattttgtattgccttattaagaccaaatacttcttgtcatcccattctttatcctcttctttcatggaattgttatcgttaattaaaacttttttaaacattggcttgtttcaatcatactgtaaattttggttgtagtcagctttgagtgcaatgagatgtataattctgttatcattacctgttgagtttgaaactcagttgggaatatttaatataatagaatgtaagtgacatttctgaaaatgctttctttcagggtgaaagctcttatgtttagcatcaatgtgtatggctctgttaaatgcagccatttctgagacgagattcttttatatatatatacatataaagtactattggcttttaggagtttcttttatatacatttatgaaatactgaagaccaatcagaccattaatggacacttagtgtaactttttataaagaaaataatgctaaagtaagaccaaaactgatgtcatcactgaaattaacaattttcaatatgttcatattttaattcacaatggaaaaatgtgttccaaaactggaaactcatagtactcgtgtaaactgtggaagatttcaaatgtgatgttattttgacaatgttttaaattttagagtcacattttattctgatcagaatttttattgagatgttgagcttttgtttttgaaactagtttgtcataacattgtgcataatcacagtatttattttctaggacaattgtgaatgtgtagacttatgtttactgctaagggaacaattatttataaaataatattaaatccagtattagctgcctatttcagacacttaatacttgcagagatctatgttacatttaccacactgaagttttttttgttgttttttgtttgtttttaaagaatcaccctcattgttgaaagtaaatgtactcttagggtgcgaatattagtgttccaataagcatgtgattatattaaggtggtggtagcgggaagataattctgattccattgggaatcttaggttttcgtaaatttattgggaaaatagtttttcctgtactgctgaagtttctttttggtaaacagtatctttctaaaagaaaaaagcatgaaggagaaattgaggtgtgtatacatttcctcaaatgaccagcattgtattcgtgaatactgtgtatcttgcagtgaacagtgtggaagctgttcatttttcaatctgaagtaaaatactttcaagaacttttagtttgcctgctcatttgttttatacatttcatctatttgactcctatcttatttcttttttgagttttaatacttcctatattttgtgaatatatcagaaatgtgtcatttatatattagagtccattcatatccatgaatcataaccttcctttgctaatacttgttgaatgggattttacaaattctccctcactctggtgacatttctcaggcagtcatgtatgtgtacctggccattagaaatattaatatttaaagactgttttttagaggagctgatgggttggtgaggtgtcagcacaaaatcttactggttatgttttgatgataaaagtatatccattttttccctccagctttaaggtgactgtgaaggtgcctggttttgaatgtctttgtttggtttggagatgtcgcactcagttttcaaatctagcttggatctgtaggacctatgttttttacaagtaattgccctccagtcttcaacagttgattctgttttatttttatcctgttttgagtgtactttacctttacttgcattttgagcctcattaatatttaggttatttgatttggctccagatattcctagatctgcacagggcaaaacatgggctatagggtgagcatttttaattgtctttttctgctggaaccttatatctctccatgtgttttctgctccttccctcccccatgaaatggtaagtgtgacttgtgtttgcctgaacctgtggactagtgtttggggtttctggaaacactagagggtcagaaaagagtaatgaccaccgtgacgtgcaggattctcttgctgtgacatgttcattgcaaagccctctccagtgactaggaggtgtagttattaaggttgatctgttagaaatcaccattattaggtattagtggtagatgttgctgatacttttattggtcatgactacatctcagttttactttaatattgatctatagtttgatcagttccttgaattctaatatgttgatttctcagtgtttctgtcactaaccaagaatgtttctaggcagttggttgcttcacagtcaaaactaaatggtaaactatcaaaaatacattcccaattttgctgtgataaatattgaaatgttaaaattaatgaacagaagaatttattcttacccatctattcttgttctcctagttcattaaactttcagttattggaaaggcacattctcaaagtattttatgagcaaaatattctataaatgcgtctaacaaacctaattgaatataaaagttatatttagtagttactgttgatagtaattttcatcagggtcatagttcatctagtaaaatatttagagaatgatgttaacattccagcattaaagtgggaacaaagatttatatatgaaattccttaaaagagttcatcttgccttggtttctgaccctcaagactctagctacctgccatcttgtcaaaacatttgtgggtagaataagtgttaaagatcaaattttaatatgcttctcgatatttaacatagctaagaagccagattttactgtagaagttatttacatgatttgaaaacttgacctaactggaagcctttttctcagtcatcttgttctaagccatcttgacttcacacccttagcgacttttcttttttttttggtcaaagataatgagctaaatatatatagacgttgaatgttgacaaaattattaaccagaaaaattgcttataaaggctgctgatctatttgatacctagaattaaatatttgaggacagtttttagttaataaactgctaatgtttattttactgtctctcaggtttttggtttttttaaaaaaaatgtgtttggcctttacattttctacttaagtgtgtactttattgagtttaaccttgtctgtagcctagtagcctgaaagaaaaggagacagaaccagagagatggatgtagtgcattccctttggttattacacatttgtggtagctcctggatttactgagagatattttagctatgtcaataagaacagctaatgatgtggaaatcaggtgttctcttgtgtatttcagtgaacatttttattagtagttgcatatcatctctagttccacattttaacttaacgtctttgtggcttcaccactgagctacctttcactacaccagcttctgtgtggcctggtaacatggaaggtctctcctaaggacagtctggacgtattttgggggaatgttatttatcttaaagatgcctagaaacaaaacgcatatagtaccagtgagaaactatgaagtaaacaagttgctcaggccgggcatggtggctcacgcctgtaatcccagcactttgggaggccgaagcgggaggatggcttgaggctgggagtttgagaccttcatctcttaaaaaaacaaacaaaaacctgaatggtgaggtgtggtggaattgggtaggggagggaaaggaggacttggaaaagcattctccaaagccagcaacttggtgaagttcagtacttgcctcttagaggttaggccatgcctttcaaagagagtgaaatgatgggttatcagccacattcttggagttaatatttttcttcatctttcagtttgggttctgtgctattcatagttcttccctaagaccatttcattattaccttttatatttagttgcaatttattataatatgttgttttgtccctgaacttaatctcctaattttaagatcctctctgatttttgcatattgaaacttacagaagtcactttaaaaaagtcttttgaaagtcctacaatcctaaaataaatcacaagcttgtttgttagacgtgtcaagagtctccagtctttactactaaaaagcagcactgccttaacacacattgttatgggtgaaaagtgagggacgaccagtgtagtttctggatataaagtgtgaaggactgttgagttaaacatttttagtggaatatacatagataacgtgtatttagaaactttggtgaagccagtatttgtttttagtaacctttttatgtatttccttctttgattagcattgtcttcagtgttaagaaatgtggactcctgtgaggtgctggaggtttgaatcatcttgaaaactttccaatcttgtctagttaccactgcagagacactaaggaatttaccagaaaaagatatttgatacaagtgatttaagaaatctcaacatttcctgaggccgtatcactgggcaaccagtgatgaaaactatgaatgaattgcacacctggaagattttttaagctaatgacagtttcttcaaagatgtcaattatttgccttggaaattttataaattgcatttctatgcacatcggcctctagtgcttaccactcggtttattattcataatctgcaattcaataaaggctttgtgttttcatttatcttcaaaa

SEQ ID NO: 11 - DNA, 44042 bp, macaca fascicularis
ccacgctgccctgcgcacgcgcagcgcggctcaggcggcagcccggtgacaccggccctagcgcgcatgtctgcacgccggggtctgcgcgccgcggcgggccgagggcggcgtgcgggccttccagccgctgcctattccacccaacgccggcctagtcagtaatggctcaacgccaccgcctctccctccagcccctcccagtcgcgtagcttctgacgccgtcctcaccccgcccgcggccgacggggccccaacgcgcaggcgcggtaaccacggcggcagtgtctagtgaggatttgaaatcggtcgcgcgtgcgcaccggcgacacggcccggcgaccgaggccgcgcttcctcctgccgcccccgtccccgccccctcccccgcccctcattggagcggacgcggcggcggccccctccttcccccgcgctgtcgccgccgagagtgtcttttcaccgccgccgccgccgccgccgcaggagcgccgagccagcggcgcgagcgtgactgagggctagccgcacgggcggcggcgcctcccgcgggtccttcagccgctcggcgcctgggcccgccccctcggccccgccgcccgcccttctccgatggcctctccccgcggcccgagtggaacgccgccgccgccgcggcccccgcgcccgccccgcgccgcgtgaagcgggagcccggagaccgcagccgcccgctgggacgcgccaagcgccggagccgcccgccgcggcctgccggggcccatcaccgccgccgccgccccacgccggagcccgacgggagcgcggctagagcaggaggccggggctcggcccgcccgccgccgccgccgccgccgccgccaccggcccaggcccgtccgtccgtccgtgcgcgcgcggccgggcctcggggcgcggcgggggcggggccgcgtcggggcgggcgggcgcgcgggccccgcgggggcggcgcgtggatggatccgcgcgtggcctggatccagcccgagcagaaggggccggccaatgccctgtggatgcagatctgggagacctcgcagggcgtgggccgcggcggctcgggcttcgcgtcctatttctgcctcaactcgccggcgctggacacggcggccgcggcgggggcggccgggcggggcagtggcggcctgggccccgcgctgcccgccgcgtcgcccccgccgcccggccccaccgcgcccgccgcgctgccccccgcgctgctgacggcgctggggcccgcggccgagggcgcgcggcgcttgcacaagtcgccgtcgctgtcgtcctcgtcgtcgtcctcctcgtccaacgcggagtcgggcaccgagagccccggctgctcgtcgtcgtcctccagcagcgcctcgctgggccggccgggcggcggccgcggcggcgccttcttcaacttcgccgacggcgcgcccagcgcccctggcacagccaacgggcaccccgggccgcgcggccccgcgcccgccggctccccgtcgcagcaccagttccacccgggtcgccggaaacgcgagaacaaggccagcacctacggcctcaactacctgctgtccggcagccgcgcggccgctctcagcggagggggcggccccggggcccaggcgccgcggcccggcaccccgtggaagagccgcgcgtacagcccgggcatccaggggtgagtgcgcggggaggccgcgggggcgggggcggggcccatggtcctggccggcgcccgcggtgcagacacccgtcccaggcgcccgggcttttggaggatggatgttgaaggctaaggccaaggcccgactctgcactgaaagttttttttttaaacatcagactcatttatcgtggagtgacttgcccagatcctacaagtaacagtccaagaaaaggggctgctgggtaggacctgcaggtatttgtcttttttactcttgagattggaacgggaaatcgactctctacccctccaccccgcctccgggcaagtgaggaaccccttgtcaaagtggggcgtagataagtgtggagtttcacgtaagttaagttgcagaataatttagcattgccaggaactcgaatcacgtcgaaggtaaatattaacctttttaatttcattttttaaaaaaatttaactgtcaacttagaggtgattcattttttggggggtgttgtgtcctttaattttgtgctgcaattaccataagcatcgcctatggtttataaacattggcttaattcaaagaaaaaaccagatttgtcatatatgtctattctttggaaggtgccatttttattttaaatatttctacatccgcctagagggaattagaggctctacttaaatttagtgcacttacagacggcaaggaatgaaacgaaaggtggtgtgtgtttcggggttggaattgtcccaggtgaggctgttcaggtgtgatgctgttgacgcagcccctttgccattttgggcttttctgagcgtctggaagcaatttatgtgtaggttgtatgtcagtattttaagacttaaatgataatttttccttgcacaatttttccccccaatttaaaaaacaattaaggatttgctggggtatgagggttgttgcatgcagtagagtcctacaaataaccacaattgctaggtgttgggagttcttatagtaaacttttgcttgtaactctttttctcatttgaagtatgttgggaaacacgagttgatacttctttaaagcgtgtgatacactgtaatagctgcatgttctgtaacttatttcacctggcttgggctacaagcgataccttctaaatttcccgaagtgtaaacatgcagtgcagacgccggcaggagcgcagactcctcttctctccctccagttcttacctgtagaactttctgagagcaggtggttgggagcagtttcttcttgatgaatagcaatatatacctaagggctcgcttggggaggacctttaggtttccagcctgttatgtaactggaatggactccgtttctcttagcactagaaaaaacaggaagacacgtggtctctgccagtcttgggttgtacctctgctcttagaaagtggtagcgcatcaggtcccatgcacctcacttgggctccccgagctgtttcctccaggtaactctagtcaggctcagtaggtggtgttgcttttgttagtgaatgagcccactaggatcaggtgctgtgctaggatctggggatctggggcagggacggcatgggagacacagtctcatgatcttgacccaccctgaaacctgcctgcaagtgccccctgcctagagcacaagagtaccctgctcagttgtgcaggtcccctctcacgctcttcgtcacccacgtccagtctctcatcacatgctgttcgtttggcccttttaatctctccacacctcatcctccctcatgcaggctcttgttacttctgtggagattgctcaagcagccggaggtgcctttgatgcactctggtcctgcttgagtcctttcccatcacaggtaatggggcaatcttctctgccagcaggtctggtcagattccccttcaccctgtgatgtcacctcccccatctccaatcccccacattaaagactaaagcctaaaactcagcaacacctccagggctctgctgctcagatgcccctaggtcctggctcctggccccaccccttgccaacccgttagaacctagctgtaaggcagtatggtgtagggcatgagagggctctgaagcccaccaggaggtctggtttgatactgcagtcatgctcttggaactttccttttcccctttgctggagacctctccttgcctgtctctgggtggtgtgtaccatgcctccagtatggccttgggtgcatccgcttcctgccgtctctgcccaaaggggcctgtgaggaccacctgctctgtgcccagaagggcacggtgacctctgcttgggctgctattccagctactctttcagaagcaaacctaagctgtggtagagttgggcctgtggctagaggaggtaaggtcccccctgtgatcatttccacatggcctgttggtcctatataaactaacctttttgtatcaataaatagttctgtctagaacttgcttctggccatcagcttacccagagtgttgagaaaggccaccaaaaagtctttcggttgtggcttagctaaggaaataactgagttttaaaggctcacctgggctggccaatagtaaaggaccttgttgctgagaagctgcttggggttgtgatatagtcccaggacatgcacttctgaaaatgcagtgtgtattcctcatgggaggatgagcctgctgtggagcattggctgaacccagttgggtctttgcctggtagcccatgtggcaaccctcactgtttgtccttttctggggaggagttttctgcccttggacactttgcctggtggcttggccttgtgagactgccagtctgccttctgcttcaagtaggatgaagaaaaagcaggtgaaagaggacagggattggtgcaagaaccttcagaggagaggaggtgaaatgcttcttttggctctggttcttgaatcattgtttgattgaaatctcaagcctttgttttgggagtggtgtgcttagcgtgagctgtgctatctacctgggcttctgacctagagatgttgggcaggtgtttggacaggccctgggccctttgcatcccagcctctggctgctgtcacttgcaagtgctctcatcccctgacccagcagggctttgggctgttgttactttgtcatggtcgttctagcagctttggaaacctcttcaggttaagagtcttgcataagtgagagtgggagcatggccctcagatatttggccacatccttactggtgtgttacagagacccaggaagaatgtagttgaacgaggacacatgcaggtgtcccgggccctgaacagcttctattcagagtttggcctttcgaaggctgtgccatctcaggtgtgcctgcagtgtgcagcaggtgtatgcagcttcctctttgcaggtttcttggtatttaatctcatcctttaatatcttctattaactcaaaggaaattctgttcttagtttgaagtctgagagagaccgacgactgtcggcataggacatggtcagccatgccccgcaaggcgtctggtgagagtcgtttccaacttggtgcatgtttttctcaattctttcttgcgaaggagtcacagcttggaggcgcaaccaggatcccccctctccctctagcctgacctcactgacataaagtagagcaggtgtgacctgtccggaacatccttgtgatgctcagcagggcctgctgcagagcacgggaggcatcactctaggggcctttccctcccatactttcctgtgagtgtccaggatgcatgagagaggttgttgtgagacctgccttaaagggtggcggtggcacgtgtggaccttgctttctgagtttcactctccgagtcccagaggtataagcttgtgaagagaagcgtgtatgtatgatcacactaagcagatacttgctcctgcactgttggaggaggaagaggagttaatttcatcaattaactcttccaacactccttccatttagtaatagcatcacttgttcctgtcttttgttccatggccaagctccacaaggtgaaattgaaaatcgagtgcaagacactggctgtgctggagttgaggaaagttttgctggagacctgcttgcaccatatgtctggtcactgatagatgaggactggccaggtcaggacagctgacacttggagaaggggctgcccaggagggcatgacagactctggaaaaggagggtcggagtattaaactggctgggaatgagaggcctccaatcttttcgcaggaaaaaaaaaaaaaggcttaatgctcgtgctgtggaagtcagaatggagcaaagtgggttctgtctgtcttgctgctgtgagcgtgtgatggaacaacagtgtcatttgctttttctcagaaatatttaatgcatgtttgtgacataatttttcaaagtaattttaagtaaatattttaaagtaaaaagttctaagatttgtgtctcaaggtaaagtctcaaacgttctttggtcactatttaatatgagattttgtcctcattttaaatggattcatgtaagcgtcctgtggaagaagagttaatagttatccttggaaaataagaactttttatgcctcagttaggtcatatggtttaggatctgattttgtagttgtggagtaaaggttaagaaaaaaaaacagcaaaccttgatattcaaattcagaaacttgatttttgaggatgcaaccagaatttggactaaaggtacagaggggtggcagagtcagaccacccagacttgcagaagattgaagaagccgcagtgctgccatgaagaggccctttctaggaggtgtggctggcttgtcagtgctttgtcttctctgcagtgaattggatggcaagcctcgccctcttcgaaagctgccactctgaacctgccttgagaagcacctcagggagggcaggcaggtggtctcagtcagcgctgacaggtgtccaagttacctgacctgttgggaacatgtgcctgagtgaggtggccaggatgccttttctcccaacactggggatgcacactcgtcagcatcctatttttgagatttctatgttgtggtagttctctgttgctgtgtagcaaattaacataaactcagaggcttagaagaacactcacttatggtcttaaggattttgtgtgtcagatcagggatggcggggctgggttctctgcttaggcttttgcaaggctgaagtcaaggtgttggccagctgtgttctcagctggcactcagggtcctcttaccagcacattcctgttattgtcagaattcagttccttgcaggatggaagtccttgattgcttgctagctgccagcaggggaattgggtagggcgctgtcagcttcttaaggccacctgcattccatctgcaaagcaaggtactttgaatttctctgatgttttccgccagctggaggaagccccctgtttctatgggcttgtgttattgagtcaggctcctgcagataacctgcctacctgaaggtcatgtagtagtacaacatgatcatggtgtgataacctcatcagagccacaggttccaaggagtagggtgtaggaccttgaggggaggaggttcttctgtgggtagacttcccctggcatagaatccgttgatgagcaggttgtggttcttcttgtccaacacttttcccctgactggactccagcccatcgcaatgactcttgcagattgccagttccgtcctctggcttggtggttactactgaactcaggcagccactataaccaggagaacctttctgtgctgcactcagatgaacattctttaaaatatgtcatttaagaaaagtttgcaggactactcgggaggcagaggcaggagaatcctttgaactggagagttggaggttgcagtgagccgagatcgcaccacagcactctagcctggtgacagagcgagactctgtctcaaaataaataaataaataaataaataaataaataaataaataaataaaagtttgcaggaaagccgtgtgaatatatgaaaatacagtgattgaaaagtcctgttcacgaggtgtcctgcattggctagtttaggaaaggggtctttcctatgcaggtgggggttgatgacttacccaagagtcacctctggaacccagttctcttaagttgatagcagtctatctttgctttgcagaagatgtggggaacacttgtcctgcaagcccaggttcgtagcaatgttggcttccccagaaccttggcttcagagcactgtgcctcctttaggaggcacaagaaaactcccacacggttcttccctctgtcccttcctgagccccctgagtgtttggctcttgtggagttgctgctattactaagttgatcccactgccctcctgagtctcctcagggaaggaggggctgtattgtagcccgcattcttagtgccaagcacacggtagccactaagtaagtatctcccaagaaagaagagcaggaggaggatctgccaactcaggagagcaggtgggggatggcaagtcttcggagtattcataaaccaaatgctaagggaaacttttgttgtttgtcttagaattttaaaaaataaagtctgttgcagtttatctgctttccttcctggagagtggctaaactagtgttctgttttacaatgtagaatgcaaaagcagaaaacattcaagaaaattctatactgtatttgaaaaacatcaccatttagttttaactgctctttgtttcttattataaaaattaatacctaactatgaaaagttagaaagcctggagaagtatggaggtgagttgtccaccattgggccactagagagtgccctatgagcctgtccctggtgtcctggactctggtggtgtgcactgcatttgctggcagtgagccagggggtgggccacatctgggcccgggcggggtggatctctgcagaagtttatccatctcttggctgacagggtgggcgagatgggagcagctctgagggtccctgttggcagagaatgtctttgattatcaacaacatgcctttttgttgtgggcttgtgatccttttctttcctaaatcagctgccgtgcataaccagttaggctctcctgtggcttcagattggagttagtttcccaagtgctaggatgtgggtgttaggtgatttctgtctttccgtttgaaagagatttcagatcattgtaacatttctggaatcctgtcgatctgaaggaatggctaggatgtagtagtttaagggaaatgaaaagtcgaatgtattttgatgtttctgcatcagacctgctcggtggagtccatttctcagcttcgggagccacgtgcttggctcttgagagcctagctccatcagcccatgtcacacactcacaggtctggctttagctggtttcgccatggtttctaacttgagcctcagtttccccccctgtgaagcagagcctgtggcacccacctcagagagtacatgaaagacttggaagcactctgtgagttgtcatgcgagagattaaaaaggccaccgctgcccttttctcctctctttaaggaaattgaaaccaaaaattaagtccttcttgccagctggacaggaaaagcctttttcttggtttttgaaaatacaacttccactttcagaccaaagtgaaaactgctaaagactgaatattctgagtcttgggagtggggggctagaggggtgttgtgaattgaaagatacctttctatttttaaaacattttaacaatgccttaatgatgaataatgtctgttctagttttgcatttgttagtttttttttttttttttttttaactgttctgaaggtacatcagcactgttctacagctttaaataagaatctcatctccccagaggcaagggtactcttgatgtatttgctcagggctgtatgtgctgctccgtgtaactcatttaaagttggttaaggtttttttatttcttgcacatagtagaaggagtggatgaagtgttttctgaactctttgcagcttctaacatagtgttctgtgtatagtgaaggaaaacaaaattaagggccagggaacattaagtaggcaactagaacagcactgtccagtagaacttcctgtggagatggaataattctatttttgcactaatacagtagccactggccatatgtgacttttgagcacttgaaatgtgacaaatgcaactgaggagctgaattttaattttatttacttttaattaaaatttaaatggccatgtatttagacagctctgaactgcagtaactttaggctctatttgaaacagtgtttgattcagtaactgttgctgaaataaattgaaactcatacaacagtaaaagctgtgttactcagcaagttatcactgtgaaagctctagaaattgtttgagtttccaatgcaaatccttttcaaaaagccgctgttttaatagcacatgaagcataaaataggttcatagcagagcgcagcacagagcaacatggagcaactgttatgacctggagtgtctccagtccagcatgcaggtgataggtctcagcatttttgcacgcaggttaatgatggtgcagacggtcacttccttctctcaacagtcttcctggtcacgagcaccattgtggctcgtgtgtggggctcttttggcttagctctctgcacgagtttgctcctttagttcccagagctgacccttgaaatgagtgatattactcctgttttgtagacagaaaactgaagccttgacagtctgacgtgacctggcaagaggtgctgcagttggaaatgtgaattcacggctgacatctgggcactttactcctaacagtgttcagtgaacaagacgtcgctaacatgcgggggatggaacctagcaactcattctacaaacatggttcaaatatgttggtgcagggccttttgctttgttttcctaaagagattagattcagatgtggtggggtgctttgacagccaccgcaggacaaagttgatagctgtggggttgcggagtgttgaggatttcatagggaagccagtcctgcgcagtagtacgctcaggttcgtgctttcttgaggtgttccagaactggcctggagggaggctgcagtgtggaagcgggatttctgtcacctggagtattcttagaagttgcattctatgaagagtggagcatctgatgagctgtttactcgctgtttcatctgacggcagttgaaagacaaggcaggactggcagcgcagctgcctcagtcagcactgctgcactgggggcttgacctgcagtctcgcaatcctggactataactcattttgaagagagaaaaattaagcattaagtgattcaagcgtcttgcccaaggcgctactagaaaataaaggcactggtgcccagatgcaggtctgcatggtatgcaagcctgggcttcttcccacctcccccacagagagggcactggtatgttggagtgaagagccacgcaagacctctgtgaatgggcagagatgggccagtgacgcaacacagtaaagtgtattttggttataggcatcgtctctaaacttatgtaaaacattattaaaaaatggaaggacaacgatgaaatgatggccaaaaatatagaaaaggataccttgcatgtcctgtgaaatgcaaaggaattctaaagtgtcattatgagttacctcatggaagaaagcaaaaggtgaatctatctagagtttgtggttctgactcacaagagactgatgttcatgctgaaggacgagtgtgacaggtggaaggatagagcaccgagaccacactctaaagggtaggaatctatgggaactattcagggagatgaaagcatggaatgaactgaagcttgcagactcgttgagtaaaaagcgcgttttaggattggttttagaataaaataacaaggcctgtggttggggaagatgacttgctgttcacagagcctcccttaataggtggggacctcagcttttcctctgctgccatcaggtgagtggtgtacagtcctagccacagtagtaatcaccactggcctgactgagccctcaccctttatacagtgtctcctgccaccctcctgggagaggctgttctcggcacagctggcctggggtcacacagctggtaggtgtaaagcaggcattggagtccaggtagtctcactccgtagcctgtctctttagccactggaaatgtagagcaaagcgagaattgtccaaagagataagctaataaagaggaaaacaggctgggtgcaatggctcacgcctgtaatcccagcactttgggaggccaaggagggcggatcacaagttcaggagatcgagaccatcctggctaacacagtaaaaccccatctctactaaaaatacaaaaaattatccgggcgtgatggcacgcacctgtagtcccagctacttgggaggctgaggcaggagaatctcttgaatccaggaggcggaggttgcagtgagccgagatcacactactgcactccagcctgcgtgacagagcgagactccgtctcaaaaaaagaaaaaaaaaagaaaacaattatgctgagttccagagaagtgatgtctgtcttctcaggagagatgccgatgctgtctgagggcctgcccagtctccacatgattcagagactccagagatggacagctagtgccctgattttcccaagaggattctgagggtgacttctgtcaaccaaacaggaggacctggtgctgtcatcaccagttgtagagaggctgcggaccacctgctgtgtgtgccatcttacactgccatttgctgattgcttcaaagctagaggttgtttctaagagtgcttcgtgctaactaactaaaacataatgacattgtttttgtaaaactgatccgtggtttgttttttaaagcagaaagctctaaagtcactcagtcccaccacccagaagcacaagcaggtggctgccactgtaggacctctctctctaggctcgtgtagatggacacatggattggtcagtagaaatacttttattaaaagtcttatctttacataaatttgccaaattattaattttgcttgaaagggaaaggtgtccaacttcagttggaaatactagtttctaagagatactgctgagactaagagcataaaacatgatgaaaaccttaagtggctaagtgcagcaacgtcagagtaaaagctttgatgaagtcttggtttgcttgggctgtgtaggttggaggctcagcctttgtttctccctcctctggtgcccagtggtggtgtttgtgtccgtgaattttcaacctctgtagtttgtttgtagttatgaccactgttgcaccgaacccttaccgagggccaggccctgtgctaagcacttgccagtgtggatttattaagtcttcatgacagcaccatgtagggggagctgcgtccctgtgttgtacttgggacgcgatctgacctcaggcacttcaggctcctgaagggtctgcagtctcgtctctgcctgggaaaccacgatttgcagcatattccacagacctcatgctcatcatcaggaggcttcccgggactgctgcctgagatttctaagttcctaatgtggttcatgcttctggtgagtttctttgaggcgacgccccctgcgttgcctctggtcagctcagtcctgtggtcctgcagggcatcctacagtgtcctctgtctgtgacttgtgccgtgccaccttgacctggcatccactgtcctctaccgcgtttgcagataggagccactgttggtgcctttttgtcgtgtgtgttgaatggtcagggtcccaaatagctgattgggagcactctccttgaatctgccatgtgcctgggtctcaggtgactgggcccctccttgcttcagaacccacgtgcgttgcctgtcctctctggcttggagggttgtgtggaatcagaggtgagacccagtccccagggatgggcagttgcctttgattgcccagctgtcctcagcgccctccctcctgcgcccaactgctgtctcagttgcttgcttgaggatccggatatagactgaggtcggccttagcgtggcggggggttttctcttgagtcttggatactttgttaccggtcccatcttcctgtgggtgggagtgtctgtcttgcttggcccagcctcccagagaccttagctctcttagtacatgggctctgcctaccttgatccccagctcaccaccctagtgcagttgcttcttcgctcttgttccactccttgtcgccatccaccctgtgctttctcgatgtgtccttactcggtgtttctgtggagcagggcatcctgggcttcctttctgatccctggctcctgtgatcttccgtgctgggctccctcttcccttcccttttccactgtgttgccctcacacagctggcatgccatggatgtcgctcacccaagcccttcctaatgttgctcaccaaaacccctcccaccttgcccctgggaccttctccccttccaggctgcatgcaggccgagggcctggcgtctcagcaggaggcagtggggcctttgctggcacctgggctctgcatcctgaccttctgagggcttggtcctttaggtccatcttgaatctcctccaggcttcggactctctgctctgtagctggcccatggagacgggtacactcaggcctggtcttagactccgctgcttgggctgtgctggtgcctttggtgccctcttagtccatcccacctgggggccctgtcctgctgtccattgtgccagagtgctgtccccttgtctttccgtaactggctgctcgttacctttcccatctcagcctcagtaccagccacttggtatcagggaggctctccctgaccaacctaaagttcacagccgtggttgccagtttaaatttctgcatagcaactttttggtttattttggctacttatcttccccatcatgccccctgtccctcccatataaactcagtgagagtaggggccacatctcatcatcctgcccacagctctgctgtctgtatcagccagggtatgctgtgcagaggctcacggtaaatagctgcagaccacgaatcccatctgcttgctgtgctttaatattggcttacatctttggatccagtgagttcttttctctgtctccctctctctcactcgctcatacttactttgtgtaattggtgatttccagccttttgtatagtcctttctcgaatagttgttttctgtcatcttggcgggggcctcaaggggttgactgtacggagggcaggggctgcagagctgcagctgctgcctggggtctcacggcgcccgtgaggtgtaggcaggtgctttgcctctgagctgtctgtagaatggggtgacggcggtttcatcagactcagtgaagcatgtcatacagtgagtgtctggtcacagcaggaagatggtgaatgtcagctaatgagtattcatcaccaatgaatagtaacagttttttttactaaggctatgtaatgtagcctcagaattccactcagcacagccccctggcagcggtgcctctgagagctggcatgatggagagagcctggttggccttactggtgtggttggggcacttgggagaacgccttcctcacaaagctcatctggagggttttcggacttgtaggatagctttttcaggggccttgcctttggcagggcagggacgtgtactgctgcagtctagggtatgggataactttctaaaccagacccagaacttcatggccgcaggggccttttagccatgcggggctaggagctgacacagcgtcagcagcatgagggcctgtggtgctgggcggcagagcccagagggagcccctgctggtgtgactttagtgtaaaggctgggggataccagattcttacagaagacttaagacgggcacagtgatgtctgctctttgacccttgcagtatgaattagtaaaactgaaattattacatttcctttattaggattataaaagcaatgatgacttattgaagaaaatttggaaaatacagaaactacctataatttttccattgttaacatttgagcatatttcttgtcacttttaatggtgctttaaatatgtagcaaatgtatcatttcgtattttaaaaaaatgctaggtaagcatttcctcctgtccttaaaaagctcttttaaacaactttaaaatattgtatagatagatgtacacaattttctgaataattggagttatatttacatcttttcactctttaggaaaggactggcctgtttctgtgttgggttccttcctgagtgtggcttccagctcagtggctcagacttcaagatgaagacttcagtcctggttgtgtatggtcttgggccagttaccatatgtctaatgaatacttagttttgtcatctacaaaatgaaaatagtaatatttgcctcaaagactattatttgggaggatctagtgcaaatgttagtaatgtggatattgtgtagtgtcccaggatattaatgtttttagcctcttggcttttattctgtattgttgccccaaaagatgatgctcacttatctttcatccagtgtaaggatatctggaaagacaacagaaagtatagctgttttcatttcaaaagtgatcagctgcttgagctagcaagcaaggcttgcactagcttccaggcgcagtcacgcagtttcacagcaggcgcggttccctcggagcacccagagctgccctgcggtagtcagcagttgtgctgtggctgcactgccaggctgggtggcaggtggatcggagccagcagatgtggctcaggaagtgccttcttggcctctccttaatctctttcagagtctgtgggcccttgattgcactgtgggttgtttcagactccagtattaggagactgaaccccttggtggtttttttgtgtgtgtgtgctgagctgggttgaggacatgttaagcaggtggggtgcctcccctgggtttgctccgggtggtacctgtggtgtggggtggttctgagtagttctggccccactgctggagtatctgcccactcagtttgtgagatggcagggcttcatcctggtctggtgcctcattttcttctttagcagtgggcttagaaccaatgcagattcccaagttaagtattttttctgtagcttaattattacaggcttctggtacctaagccctttcttactttctgttctgaggggaagagaagataatgttgtttctccgcccccccccggagtggccccaggaccttgcatggcatttgcagcatttgcagcgtgcttgggtttgctttactagggtgaaagtgttgcaccccccagcacccacaaaggcacctctgctcacactccggtgaggttctgactggccctgggacatcacctgctccaggatcctatgtggctcatcccaggagagatgtgggagggaaggggaaaaaaggcttacatttgctgagtggaattcatgtagatctgagttccgcattgattcctaagctgcagagcccttatgccttggctgttttgtgaatgttagtcggtcttaacctttttcaccgagttagcattggctgtctcaggaggctcacagctcctgctcctcctccaggggagtgcgccctcctcctctgtcggtagctgtcaggtgcccctttcctctgcagcagactgtcctgggtccttgcctggccttccccttacacgtgagcctgcagcttcattcacagcccctgtgtagaaagataggcacatcgataggtccctccctgcccagagtgggcggaactgaggcaggcactaaaagcagctgactggcagccctagaaacatgaagggtttcatttatagtttcagtccttttccttctttcgagccttaatttaaaaaaaaaaaaaaaaaaagccttgaagtcctgcttctgagttttctaatttgtgcaggtattagttgccttgtaacataatcaaaaataaataaaaatgatttataattagcttattaactgtatcagtaaatggatactttaaagaggatcattgatccctcaaaatagaagcaatgcagtcattccctcattatgctttacttgtgatttgcttacaacccactcttcctagttaaagttaaatattaatccagaccctatcagtgcgatgtagtagtgtctgaatcagttgttgttttggtgtaatcgtatcaaagcatgttataaaatctacaaaattgcagggttaactccaaatattttcactaaggtattgtttttttgggcaaaaatgcatagtgaacattgtggagctgaagtgagggaacttcgatttctgagaaaccactagttttaagggttttgaaggaagagttggaggaggagaggaagagaataaattcacagttaatgagtttccagtattttctgtcgcattttacgttgtaatggaaaagactgggaactgaactcacatgcagtttgtcaaatcactttttccctagaattcaggattgatgagattaacggggtgttaaaggtaaactgaggcacataattaacatggacagaactgtagacctgagtgttgagagttgggaaatttcagtgagttgggaagactggaagcacctgttcttcagagtgcaggtcctcatattcagtgggtttaaggtgctgaaactttttttttttttttgagatggggtcttgcactgttgcccagactagagtgcagtggtgtaatcaccactcactgtagcttcgaatcctgggctgtcagcctatcctcccacatcagcctcctgactagctggactgcaggcctgggccaaaactcctggcttgaaacttcttgtaaccagattggaggaggagggcatgttcattttcgtgacgtttcctttcccttaaacatccagtgaaatctgacctttgaccatcactttgcttaaaagaagctactggatttaaagtctaggagaatgtcctagacaagcccatagtatgttcctgtatgttccccacccagagacctgcgttatgaagtgtttggtgtgcttcttccagccccactgttctttctaaagtgttttattttacatacgctgtcctggcttctgggctatgacctttgccttttttgccctttagttcctttgccctttacctactgcagtgcagctgcctgtccttgggttgactacaaagaagtcacctttgaacaacttagaaattgtgacttttggggaaggcagggcagagccttggggctgagatgggggaggagccagctctgccctgggagagatacaaagcgcctgcctgggtgaggcagtgcacgggtgggcttgcttcacctctttggccccagcttcaaaaccagccagtcctccctggctttggctttaattcacatttacaagcttgaaaaccagttaatcccattagctcagcttctaaagctgaaaatcgtcccctaaatgggtcacctgttgtcatcaatagctttattagctatggaataatatagttttgttctctaactgtaggatccttcttttgctcttaaaatagctcagtaagttgggtctcataaatacatacagcaagcatataccagatactaaaatacaaaaacattgctgatcttgcttttcagtactaaaagcagaaaatcgggaatttactaaattgagaagtcagtcattacctttcgatgggtttggactcttgcaaggcagtgattgtaaacgagagtgatcttttgttgtttttcaatgaactttattctctaatttttagtaaagcacactaggaaataatgcttcagaattctgttttcgagtagtttcctgactaaaataaaaattcactaaaaaaaacctctgctgtcaccatttccttttttcttaagataactaggaaatgaatcattaagagtttgctccgtggcaatggatcgggaagctgaccctgctctctgtggggctggagccttgctaatgtcccaggatttcacttcacagagacaagcatcagaggcttgcttcatttatagatcctacttcttttctacaccacagccaactcaaaatggtgacagaatctaagacgaggctagaagtcaccacggagcagttggaagctctgcttccggttctgggggcagtgttcctggcgttgtgtcctttggccccacctcagtttgtccgtttagctcctcagctgagaatgagatgtgtatcatataggagtttcctgggccactcacagccccaagctggagagtgccagcctaatgtgtcaggagtagggggtgaggccagagggctgtgtgccaactcctccctaagaagcctcctgggaaagccctcccaggcacttcccaggtctcactggccgcctgaggctgcaggggaggatggtcaggccgcctcttggctggcactgcttcccggcgtgccgccagcctttctcatggggaggggaatgatggcatgcctggggggcagcagggccccagggctgcctagggctctcactgtgtcctcctggttctgagatgccacctttgtgatccactgtagagggatttattctattatgatcaatgcatagaaatttcttcgatttggagactgaacactagtgagcagaactgaaattgagctttaaaagatattgatgacgggtctgtggataggagactttagtgtggtttttatgcagacgtcctgccagctgtaaattccctggaggtttggtatgtgagaacataagactaaacttatttctattttgttgaggagaaatgattaaaacttttcattgatgtacttctgtggcagactttttggagaattgaaccagcgggcatattcagtatttgaagtcatagatgagtaaaggaggtatgttgtagtttgcgctggcggcgtggcctgtggtcggcagggcttatctgtgaaggtatgtgcacagcttcctaaggcagtgaaaagtcctggcagtgttagtattgaatgagataatccaaaaaatgtaaaaatgtttacatttttaaagggatagttggcgatttaaatggtttctgctaacaaatcaaattattcattgcagaggtaaaatattttcagaatgttaattttagatgtcgtagagagtgtacatcagcaatgacaaggtcagcaaaatatcttagcaaaacttgattgattgattccatgcacaggcaagcgctgttctgggcaccggagacggagcagtgcgctgttgcgtccatccacagatggcctccagagtcatgcggttgcagggaggccgaagggccagggaggccgctgggtgggcacggctgggcggtgccctcacgtgggttttgttgggctactcttactgtgcactttttctcagtttggtcagtgttccgccttgctgcctggcccccaaccctcgccctctgagggcctcacaaagagccaagcagaaggcaggctgggggcttttcaggccagcccagaggatgtaatgatgatggttggcactgtcccacggccgccaccagtctcacactgcctcgtgggcagtcctggagtcgtgcggcaccttgctggtccctgctctccttgaagaagggccagtggggcacttcgccagagccttcttgtctgactccgtcatccaagaggcatggatggccgggcccccggcagtttccattctattctgagaaggcaaaacaaaattattcctgtctcttattatctaatatttgttacagcagttgctcacttttaggtgcattttattacagatttcagacaggtgtggttattagtgcagcttactgtttggacacaatgccaaggtcaggaggacagtgttcccctgagcaccacttctgctaggagcatgggcaggccatgcctcgccattaatctctcctgatttaggggaggaataccaggccaccccctcttctccctgtgcaagggaacagacatttgacaaaaacggatgccatgttacgctgattttgtgtgtctaaggcagactgcagcaggtgttatctccgtgctcttcctttcctggagtgttgagcatctcttgatagtaggggatgcccctgagggtggtgaatgtggctgcacaggtcctgaaagctatttgatgttgccgttacttcaggtagaacttaaagttgacagtacattctactctgcaggtggaaatgtggagtgccattttgacaaattggaatgccctgtttacaatatgctttaatgagttaaatctgggggatgtggatagaattttagtatcctagctttggcattcttccatgactttgggccaattatttaataattccaagcctgcatctttgttagaatctctaaatttctctactcctgttattatcctcagaacaggactgtgaggtgcagtaggccacatggtgtagtggtttaggtggacagacttgccagtgctgttctcatggatagcctaggactgtccctagctctctgcagtgacagtgatagtgactggtgaaggtgaagggatccacccagacgttcttcctgatggagagaggctggcctgtggctcttccctggggtggatgttaacctgctaacgtgacatatctagtcctgcttacattactaagtggtaggaaattttaggtaacacctcagactttaaagtggcctactgagctggtagaaaagtgtgtagttggtgctcagtaattgttgaaaagatagaagctttacttcaaagctcttgtagtttgatcagtttggaaaaaatattttaatgttgggctctgttaacagctggactggtggctgtctgaattgggaccatgcttggggtgaggttttttcttacttttttttttttttttggtgagacagagtcttgctctgtcgcccaggctggagtacagtggtgcaatctcggcccactgcagcctctgcctcctgggttcaagcgattctcctgcctcagttttctgagtagctgggactacaagcatgtgccaccacgcctggctaatttttttctatttttagcagagatggggtttcaccattttagtcaggatggtcttgatctcctgaacttgtgatccatccacctcagcctcccaaagtgctgggattacaggcgtgagccaccgcatctggccacatatttttttaaattaaatgtgatacataaaattaggctgcaggcatggcctgatttgcaggtgcttcatgagcaagcgtgcacagcatttatttgctgctcctggagtctctcgtgtgtgcttgtagcctagccttaagccctctgtggacggcttggaatgcgtactccaaatgactcttttggcggggtgggaagtggcaatactttaggtgactgacagttgaaattaaccttacacaagagccaaactgtaggctgatgcagggccactcacctttgtactcacccctggcaggtcctgtaagaggtgctacttgcttccactttgccagctgttcgttggccctgttttgtcttctgctgtttgccttatttatgaaacagaatggaaacaggcgagtttgatttgttataattcctaggagtcatagaatggaagcaggtgagtttgatttgttataattcctaggattggataatttgccttcccctctctccatctttaattaatcccttaaaggaaaagaggacgacagcacttttcctgcagtcatctgtgtaggcctcagccttaactcatgacataggctggtgccactggccacagggctgacctcagctcttggagcccatggggtgacaggagatcagcacctttgaggtggcggcgtgaggcgtcttccaggccttgctcatggtgcttgaaaacactgctttagagctttgttaagagagagaggccctacttactcctgtcccacaggcatttgggtgttgacctccttgttggcctcttaaggagagaatacttgagtattgaattcgatcagcttttctgcctccagggaccctgtttctctctgctgagactgtggcggatgaaaccaggatttagtggatggtcaccaggtagcttgggcagacctgggccgcggggcccctgaggactcatacgtctttttcctgttcacatgttccttccccacaccttggcccattctcagtccctcccatgctccttagcgtgaggcactcagggaggtgcccatggggccttggggcctgtgctggagctggttcccagcctcagaagtgtgcctaactgtgccacattcattggaaagctgctttcacacttcctggatggaattctctcattttttcaatataaagtcactgagatgatttttttggagaagtctttaaaggccagttatacatttattgatacttggtattgacaaagttcagttgtttagtgttgctaagtcatactgtgtaagtttgttgagcacagagttttcattttatactttcagaggagaaatgaaactgaatttcgtggccagaaatatgtttgagcgtcatcctgatgtaagaacagaacagaaaatgtggtgacatttcattgtaactctagtatgttttcttttttgtccattagactacatgaggaaataattgacttttataacttcatgtccccttgtcctgaagaagcagctatgagaagagaggtggtgaaacggatcgaaactgtggtgaaagacctttggccgacggctgatgtgagtatgttctttggagttctgtgtcgcacgtcacgtgcgagtaaatttaaataccctgtgatgatgatgtgtcggctagatccacacagaccttttctcgttggcccgaggcagcagttctccaagtgtgctttgagaaggcctccgttgcctggaatgcatggcccccggcgcacctgcacctgctgtcttagacacctgcggtggccgcacatcttcgtgatgctggcgcgcactcaagtgcgaagaccatcggctgagggatttgttgggttttttttttttttttttggaagggggagaatggtgtgattgtttctcttaagttcaccttaaaatttagaaatttcaccctgtcacccacccctgcttccccaccaccacacatagtagcatataatgtgctcatttttgtaaaacttggaagtgttccctcatcacacaccactcttgcagtgaaggaacaagtgttttttgacatgtggagtggggccttctggaatgcttggtgcaggtggcgtgaagcctgcccctggccggctctattcagcagccttccctactgctgactgggctcagtggaccagcagggctggccgtgccccagctgtgaggggcatgtgtgctcttggtgggcaagggcaacccagttttctgcgcctcttttaaaatgatacagatttttggctttaaacttcagagtcctaggacaaagccctgccccagtgccttagctgtgggtttaagaagaggttgaagggtttgaagctagctctgaaaagtcctcagctttgaagggttatagggtgaggacaaaacttgtttcacctcttaattttgagtttttaaacattccttttttgggcatgtctttaacttaaagggaattttctggttgattgttatacggtcccctccatcagtttccaaggtagttttattttttacccaagggtatagtgagggctttcttttagtaagaaataatggtagtgtgactgcttggtttgtggtatacattttaaggcaaccactctttctttcaggtacagatatttggcagctttagtacaggtctttatcttccaactaggtgagtaccagactgcatggcatgggctagtggggggctgggatggtgtctatgcaatattaagggctacaaatagattctttgtaattgagtctaaggcgagaaatgccagctaaaggaaaagactgtggttacagagggaaattggcagaaagatttaatttagtgttatgatgaattcattgctttgcatttttcctctcacacttaatttgttggggtgcaaaaatgcttcatgctggaaatatgaagaagacaggtgggaggactgtgggaagtaaacgcaatagaagacattctgctgatattttaggacatgtgtttgaaaaattgatcttatgttttgatgaagattcaagcaaaattctctttaaatagtattttctaagtatttttacctgataggaaaatgtcaaacaagtttgcattctaaaatacaaactagtattttctcattaaggattcttgatagccaaataaatttcctgtgcactgtctcattaaaagcttaccttctattaacccactgctagttagcatttggaggccgaagaggctataatctcaggatttgggggttgacattagcagggccagtgggtaattgaacaggtttgggtatccaggaatctctgggtccgcaggagtgatccagcgtaggcagtgccggagtaggtgctgggagagcggggcctcagcctggtttgggggcaggcattttcatttgaatcccctcacatacctagtgctgttgggagaatgatttaaccttcttgctttccatcttatgctacaaatatggaagtcttcccttaagttcagcgaggacttgctgtagttcatgaactgcacttcacctccttaggggccataggctagtgggattgtgtcttggcctttgtgggagacacaggcacatgtgccttggtgcttatcctccccacacgagtgtgtaggctgtggcgaggggagcagtggctgacgtgcgttttcttctgtcagcgacatagacctggtggtcttcgggaaatgggagcgtcctcctttacagctgctggagcaagccctgcggaagcacaacgtggctgagccgtgttccatcaaagtccttgacaaggctacggtgagtgcctggctttggcccctctgaccgggcaggagccttgtcacatcccaggtggtcacaggatacgcctgcgtcacgagcttgtggtattttacacagttattggctacagttttgaagattaatctgcttctggtatagacatgtgttttatgtttttgtttcatagtcgtgatcaccaactgagaacatgtttagtgacagtctgaacttttgggacttgtgagcccattaaactgttcttggaatgaaaatatatgattgtgtctacttgtgttaggatgaataggaaaggagagtcatctgaaaccggacactgacattcaggtgctgcccattatggagagtgtggctcaatgattaaaccatggtttttatgattaccatttgctatgttatgttaaagaggaacaacttagctgttcctttcgtggttccaaaaaatatacatatatgaaaagccttttatctttgggggaagtttgaagatgagactgtttctggtgtgtacttgctaaggtttatgtcagttcaagattataagccccccagggactatgaggtacttgcctgttgtatgacagttcttagctcacctgtgcgaccggctagcatttcatttttaaatttgtgtgtcaacttgtgtgtgattcacatccttatagtgtttagcagaatgtaagttaaggcaggagcttcctcctgcctgtgtggtgataggggagggggcattcacatgtttctcattgtcaggtgcttttgattgaggctgggggcaagttttaaaacatgatatatgcactgaaaagtgcacatgtaccaggtgcacctcttggtgagagttaacgaagtgcacatgctcatgtcactgtcatgtggaccagagcgagcaggcagcaccagaggttccctccaggcccaggttccagaaggggctgttggctcttctcattagcacgagacaagccctggccggccactttctcaaatgcttacgggccttattgcacttagctctcccagccactctcatcagcagatgctgttgctgttcacattttacaggtgaggaaactgagatgcggagaggtgaggtcattagcccaaggtgggtcagcggcatagtccaggccgctgttgtctgctgctcctctgtgtgtgccaaggggcagcggggaggtgggtgggaatcctgaccaggcgaccacctttggagtagaggaactaaggcgcggctgtcctgaggccacacagtaggttgagcagttacagtaactgcttagtcccagtgacctcgttactgtcgcatattggctactaagtatcttttcctctgttacctgagggccagtgtagactgtagggagagcctggagcctgccactgctcatttctggggagcactgtgcagccggccagtcatgggcacaagagacccagggcgagggctgagtttaaggtgaaatcttgtctatttggaacaacaacccaaaactgtgttacagtgttaactcctcacctccaggatttggggttcctgccgtgagtgagtgtgtgcaagagtagggcaggagagtgccaggagtgattgtgggaaggagtctatgagatggaaaggaagctgcttcctaaactgtgggtgtcagggaggcatagccattgagtgttggcttcttccaaagcagtttctgatgagttctttgggaaagtatttctttctctgccttcttaagaacatactggcctcagggcttaccctgcctggtggtcgcagtggtgtccaggtgactctggccccactggcatgtcctcacacgctgagtccttggttggttgccctcaagtgtagacattaaagcccagaataggtgtgtactgaatgcactgtccctacgttgcctatcactggcatttgaacttttcgttagacactgattgttttggttaaaggaattcctttttttaatccttcaaggctgaaggaaacaaaacattgccttttcttctggaagaattcagttttactggtggggtggagggtggggcatgagtgtggtctggacagttgctcaggcagattttgaatgccattcggtgacagttcttgttggtgagaatatttctaaaatagccttttatttgctgaattttttaggggaaaaatttttttagtaaagttgtcttaaagagtgaaaacccaaagtagagaaacaatatcagtataacatacaatttaaaaaatggcttcgaagttacattaaatgatttcaaaaattctgccaaataaaagtctggggccaagcacctctctccatcccagcacatagggtgggcgtggcagagactaactcctgttccctgttggctccctcccctcacgtctctttgatgcttggtcacctctggtgctgatccagggctacaggggctgggcagaatgtgggtcctgctgtgaggggctggggcctgggagtcgtcctgggttcagggactactgatgctgacagtgttctctgaccccctttcattactaagaaaaaacaccaaacctctgtacagctttggcagcattttgatgcctggctgtggagagtcctgcatgttaaagcagtttttaaaatgaaatctttacaggtaccaataataaagctcacagatcaggagactgaagtgaaagttgacatcagctttaacatggagacgggcgtccgggcagcggagttcatcaagaattacatgaaggtactgtgcttggtgacccagcgcggcgagagtgcaggactggagtgcttgtgcttggtggcatcctacgatgtttacagctgtcagctgcacacacaagtctttcgtaacacagactacacttacattatttctcctacaatattatttctagagatactttgaaattacatagctgtttttaaaatttgcttttcctgagtaaccattttataaagttgacaattattttagagagctttgttaaaatgttctttctagttattacagactttgcttctagctcagtgtgcctcattcgcaggttttacccaggtggaagttgataaatcatgaggtgccttaaatatactcactttgggaggtctcagtgcctgaggatgggcagagagacttggttgagctgacatgtttgggactctgaccatgtgcctggtcttaaacgggtggtcatgacctcctgttacagtagaggccgtgcagtccttagcaggggcagacgcacctccgggtggtcgtgacctcctgttgcagtagaggctgttgcaatccttagcaggggcaaatccacccctgcaatctggtcccatcttgttccattttcaagggccttgctcttcaggttcccccttcccccttgtcatctggtctgagggagcatgtccaccccaagcgcaacacgaacagcagcagccaggctttccctccctcctgccatctcctgccgctctgccttccttgccagcctcactctgctctcctgctccggaggcccccactgtcctcatggcctgtgtagcaagcacataaacactccagtgaacgcgctggtctcttcctgagttcctttgtgcctgtggactcgtcatggtaggggtgcacccctgctgagtcgtaacccagggagagctccacagtctcgattttcacaagcccctcaggaaattaattcttagcgtcccccaaccaaagtttgagacttaatgactgagagccttcagatgggcaagaggatcgaggaaactttcctttctgtcttgtgtgatttgctatgtgaaatctctttgaaagtatggtaattactcagtaaatctttttcttttggaatttacagaaatattcattgctgccttacttgattttagtattgaaacagttccttctgcagagggacctgaatgaagtttttacaggtggaattagctcatacagcctaattttaatggccattagctttctacaggtatgtatgctttcttgagactgtttctgttgagacatgtgtaagagtagactcttccaaccagttgcctagtgggttccagcagcctttgctctccttttactgtattgtttcaatttggtagaggctgatttctgattcttacaatcaaaccctcttgattaatgcacctttctggatgctcattttgtactgggtgtaactgttggtgcaggggtgcccgtctggttctgtgagtccagtgcacatcagtccaagctcagggaattctctgtattcagaaatgtccatttcatggtaaacaataaacatttcttggtgcttgtctgtgatttatattgaaaaaaatttgtctcagaataaagttgagtaccacatatgagaaaaggatttacaagagagctttctcagactgatgaaacatcattattttgtcttaaattatatgtggtccttattttgctgagtaacatggaaaatctatcaatagaaaacctacgtgttttaaaaagtattgttaaatgctgtgatgtattgataaactgtaattatactttttaaacatataaaatcatctctaattggaacagtaattattccgtttatattttcttgagtgaagaattctgtcctttacaaaatcttgcctatataatttagccgcacggctgtatttctccagtgtttaccattaatttggtctttgtgattgtgctgagattaccgaatctgtccatgatttggtaatgttctcactgtcatgaatgctatgatagtagaatcactgggtaactacctgtgatgatcgcagcttccttggtctgtctctgccaagatgctttaaaagtagtgaaaatggaattccatgtctgttttcttacagttctagtcacactgtcctgtcttcactttcccctctgagatgtggcccttatatatagcctttcttccatagtttttggacattattttgaattaaacatgggcctctgttctttactgatatactcctgacttgcactattttcatggccttgtagtaacaacagctacttaatactttgatcatgcatgtgccatgtgccaggcctgggtccagggcctcctccaccccctcagggggtcctttcagtgatcctgtgaccccacaggaggccaccacagcatgagtgggattcctgtgttcactgccacatccctgtgccttgtccagtgcccagagcttgtcctgcctcagcggtgtgactgtggcagcatctgagtttcttgactaagtgaggggaggaggcccaccctggcaccggccaggctcttggatatgtgattttggctaaaagacaaggaataaggaagggaataaaggtcaggccagaatcggaatcctcctcttgtgtggtggaaatatgcagagaactccggaattcttctgaaccctaaaaacatttgtatgctttctagctgcagctcctcctggcactctgtgttataaatagtttcaagcaccgtgcttctctgagggctttctctcatgtgccctcgtccatccctttcgagttggcactgtccgatagaattctgtgatggtgatggccacttctgcatggtccggcaaggggcagggcgccacatgtggctactgagtattgcagtgtggctggtgagagcaacaagctggatttttaattaatttgttttaattcatttaaatagacatgtgggcaatgcaggtctggacagctgagaattatgaccctcaggaggtgtggtggacagtggtttacttccgaacaagcccagtgcctgcttttgaagacgatatggcactgaactgagagtggtgctcatctgtgtgacaagcaggatggaagcttgctataaatattgtgatataatgctaatgacctttacacagctaaaatcaatcctttcacttttccggttttatgtgatactgccatactagtcagtctaacactgacccctgttggttgtgcttcagcataacgaaattaggatgacgagaatctgaaattacatctaccatccaggtgactaagttatgcagaatatagtccaacttatttgcccatatttggttaatcagatatctgtgtttgcaggaagtttgctgtatggattaccaatttcaaaaatcaaactacactaaaattcagatgagtccgttgtgttccttttgaacactcctcgttgaagaggctgctgttcaggcttcctcgtggtgctggtgagtgagcgagtgccactcactggtattgccttgaagaggctgctggacagcagacttcgtcgcgtgctattttctttagaacatgccatgaatccatacaaattgtgggtgcattgcttttacagttgcatccaagaattgatgcccggagagctgatgaaaaccttggaatgcttcttgtagaattttttgaactctatgggagaaattttaattacttgaaaaccggtattagaatcaaagaaggaggtgcctatatcgccaaagaggagatcatgaaagccatgaccagcgggtacagaccgtcgatgctgtgcattgaggaccccctgctgccaggtaagggcgccctgatctccactgctgagagctgggccagcctcggggacgtgctggtgacagggcctgtgttggggctctgagagccccgggcagttcatttgctcttgatgcaggtttctcttatactaaccagttaataatcacactttgagaaatccttatttaatgcttctaattaacttttgtctttctaactgtttacattctataataaagaagaattaaggaaaatcttttctttttctgattattgaagtataacatatccaccctaaaccatttgtttctctgaagtatgtaatatagaaaaaccatggatgccataatccccttttatttggacatgtatttctccactttttccctatatggatattaatgtttattattgttatcttgttgaacacatcccacaacgcaaacacgtttgtcacttggcttttgacttaacgcttacccttgaccctttcctatgtgtgtaggttgtgttttgtcgtgaggattgccgcattgaagagtctaaggctgggctagaggtttcccggttttattcccattggcgtattcaggggtatttatgtcctcattcctttggtgacagtcttttaaaatctttgccaatctgataaaaccatgtgttaacgcttttaaatttatatttctttaatgattagtggggttaaacacattgctatttatgaattccacaaattttgattgagcgtctgttaggtgagataccattcttactgttggtgataaaatcgttggcggacgggtgacagaacaggtggtggagagcccagctccaggcgcgtgtccctgggccttctcctctgtgtggctctgtgtgctgtccgcccggttgctggctgccctcctctgctgtgtgcaaggcctgtgtgtgtcggggaagcctttcttgtcacacatgtcatactttttccaatttgttttttgcatttgtatttttttattcagctcctatacatttaaaaaaacacctcagatttaatggttgtttttgttttatggcttctgggatgtgagctttatttatttcctaaagatcgtctcaaggaaaacacattggctgatgtgttttgttgttgtttatagatggcatgatttgtgcaggctcttgagtggttttcttggtagcacggtatggcagtgtatcatccatttttgtccgttggatgagtcacattggagacattggcattgtcttcaagtgtctgctgaaatgtactcaaaaaacaaagacccacataatcgttgagttataatataaatctagaaaagataaaactccagtacttagaacatatatcctttaaaagaaatccacacttaacctgattgtgaagaatgagttgtttgtagattaaaattagaaacagtgcttttcttatgaaaattaagcttctcctgactggcttccttggtgactgctgtgacagattcctttgatttgctgtcccagttttccacacgtgagaattcacattccattctaaaggatttacttcctgtaggttccattagcgttgactgagttgtgatgcacttggggtgagctgcccttctacctgccctgttggggcactgtgaggcctcctgattgtcagatcagcgatcacagtgggtcggtgctgctggtctgcacaatggtagtctttggcttcctcatgtttctgccacctggagaggtggctttttgtgggctgtcactccgtctgtgaatggcagccgcctccgtgaggtgggccatgagcacaggggcactgatgatgcagaccagtcctctcggcactcacagactgtgccctgtgcatggtgattgacagggcctttgccagtgccaagtgccacccgtgcccattgtgttcgcctgtctgggctttgctggtagggtctggaagagtttcagtggtgagggcctgcttcagagtcacttgtatgagaagatccaaaacatgtggacgatggtgtgcatgtggggagggtctgacatagcctttttgctgcagggaatgacgttggccggagctcctatggcgccatgcaggtgaagcaggtcttcgattatgcctacatagtgctcagccatgctgtgtcaccgctggccaggtcctatccaaacagagacgccgaaaggtaatgggttgtgtgtctgcgtctgggctcagcgtgcctgtgggatggtacttatccctttcctgtgtcatttacctccatgaaatttatgaagggatgttctgccgtatttcagtagaatctagatatgttggtgaaggaaggccttctaggaatatgggatggctgtgtgggattcatccatggttgagagttgaaaatttctttcttggagatttgacattttcttcagggtcttttgttttggggaggtgatttctggcttttaaaattcagtccctaccatcttctcttatgtacactcgtcccttgttctacattttggggcatttttacagtcccaaaatgtagtcagaagtatttacttctcacccagatcattctgtggtagtggaaagggtggtatttgaaggggtgggagatgagataggaatgggaaggaagagtaacgtggtcgtcaagagtggaattcgaaacagtttgatagatctgttctgtggtggatgatggaataaacaggtttcgaggcctggctcagcagccgctgcaggtgctggtggtgctggagctctgtgtgttcctgagccgctgtctgctcggtgttttcaggcggagctctgggccccatgtagggcactcgtctcggtaccgtctccattctcgtccgtgcagtgggaagtgaaatgtcagcactgtatgatcatcgtgggtgggaaggccccgctcccctacttggagctgcatttcacagtggtcttctgtaggtagatgtactgcgatcccagggtatgcttgagctgaatcattaaaagtcagagatatttgtcaacgtattttagctcctttcctactgtccttcacctagcgagatgatctgttaggggtataaggtagctgttcgagaggggttctcagctccctgacacctgttgtactctgttgatctccaacaatgtccctttgcagtactttaggaagaatcatcaaagtaactcaggaggtgattgactaccggaggtggatcaaagagaagtggggcagcaaagcccacccgtcgccaggcatgggtgagagattaattcatttgtgttcatcctaaccactggctggcatgttcatgcagaagtgtctctattcctttgtggtaaattggtcaaattaagaaaatagctagtttttctgatgagcattaattaagaagacaataagatctagagcagcactgtccagtagaagcaatataatgcatgccacacatagaatttcaaagtttctaggctgtgtcaaatgtgaaaagaaacaggtgaaataattttgatagattttattccactcaagtcaaaatattaacatttcaacatgtaatcaacataaaaataattaagatattttatagctgtttcttgtactgtctgaaatccggtgtgtatttattcgtacttatagtacatcctaattaggatgctaaattttcgtaaaaaatacttgatctatatttagattttagaaagttcacagttgaagatgatttgcatacccaagttattacaaacatgtttaatgttttccaacaactaattgaatgtaatttttaaaattaaattaggcaaaacctaatgttgggtttgttagtcacattagcagcgttcccggctcagcagagcccgtgactgatgctgccggggcggctccacgccgcagttctcaggagttattaaccaaggctttttccctccacagacagcaggatcaagatcaaagagcgaatagccacatgcaatggggagcagacgcagaaccgagagcccgagtctccctatggccagcgcttgactttgtcgctgtccagcccccagctcctgtcttcaggctcctcggcctcttctgtgtcttcactttctgggagtgacgttgtaagtgccctcccctcctccgtgtgtctgttggacagtttgtgtctctggtaaatgtccatagccgcgagcttaaaatctcccccttggttttgctcaggttttgtttccttgtatgtgtgtggaggtgggtggggggcagccccgtgatgtgggcaccaggcttcctttcccctgccgtgaaccttcagaacctgtctgtgcgactcatgcggctgtcgagggcagtaatcctctaaatggttgaactacagtggacttccttgagtagtttttaaaaatttatttgaagattaaaaaaaaaattaaatccaagtatctcttctgtatttcctttaacattctttttcagttgtgatgaaattacttgaaggaagcctgggtaggtttgggctgcctgttcagaagttagacttaatttgaataacctttcatagccagcctggatgcaggcgtttcttttcatagctttaaggaagtagtagtgcacctttgtggtacagctgtcctttttgttttttgtaccgggttcaaggattcagacacaccgccctgcacaacgcccagtgtttaccagttcagtctgcaagcgccagctcctctcatggccggcttacccaccgccttgccaatgcccagtggcaaacctcagcccaccacttccagaacactgatcatgacaaccaacaatcaggtacgtggccctctggcacccttcccgctggtggcccctgggaacagcatccgagctgtgatatgcactagaggagattgatggtcctttgaattagaagagtaactttttgagtatttggccattggtgtgttgttctaggaaatcctctcttttttgtggtgttgaggtcccccatgtatagtttcagcagcgaggacactgtggttcttgagtgctgccgtggcttttcacgggggccaggttgactgccttcctgcaagtttcctcactgccccagcatgagactgctgtcgagggtcatcttgagagagcgactcagtcacgacccacttagctgggcgccaagccgtgccagacacttgtccctacttcctctcagaatctcaatgaaagttttaatgtgaacttattagacttttttcatgtttgaaattaggcataatttctaaggctttttctgttggaatatactgtttttaaaatttagataaaattagaaatctaaaggataattttataaatactaaattttgtatctacttgcgattatacatcacttgaatatgtgtgggtataaaacccaacatgttaattgacttaaaaccattttctgaaatgtggggtataatttgagcataaagctatgtaggtacatgcaaaagtgttttgactcatttcttggagttttgcactctgctctggggaagacattctcacaggatccaccgtgattctggcggagcttctgggatgctggctctgtaatgacccacagagctgatgagcagagccatggcccagccggacaccgtaacgtgtctaattgcagcataagtgtaaaattcaggggcaattatttacactcttaaaatgaattataccacagataaacttggtcgcctttttatggtcatcacagtggccctgacgtcctggccatgtgtcacaaaggtgtttgttttaaccacccacaagccttggggcccttgagagcccagtgcggctgctgagctacagagccacactctgcggctgcttgtgtggttcgagtgtgaagtccagggacgctgagggtttataggtttttatctaagaagactcttggccacagtcaatctccagaggttgttggggtaaatgcacgggatgccaagatgcaaccaggtcagtattgcaagtctgagaaaaggggttctcgttagcgcacttctgctgctgacagtaacgggtgatgctgacatagaagcagcctgggacctggacagcaggcaaggaaggaactgccagccgtcccacggcctctcaggccaccagttgggccagccttgggctgtgacccctgagttcagcgtgtgagtagggggttcaccacgggggtgacggttgttcttctgatgactctaatgtcttgatcgtttgatcttcaatgagtttcaaactttatgacttggattactgggcatactttatatgccagttgctgttttagaatacgaagtatttccaattcaaagcacaatattgttaggtaatagtaaaacagactgctctatggagcccacatgcaactgtgccatttatcagctgccctttggtggtgctgagcttagaagccggatggttttcctctgattgctttggtacccatggccgtctctcattttgttcctagaccaggtttactatacctccaccgaccctaggggttgctcctgttccttgcagacaagctggtgtagaaggaactgcgtctttgaaagccgtccaccacatgtcttccccggccattccctcagcgtcccccaacccgctctcgagccctcatctgtatcataaggtatagctctgtcctggtgcattcacctacctgttcaagctgccatgtgagaggcggtgctaaatgttttctcctccagagagaattccagagagatcatttgaaaacggaatttgctttgttgtcattcagcctgtttgcttgtctttccaaacaaaacttaaaaaagttaaattattttaagatgtaatatatagtttaattggttgccacaaacatctcttaattcctctgttgaactgattagcataaaactgaagtttgaaataaggctcaaaatgaagacttttcccatttacataattcatttatatgctaaataccttggttttcaagaagcaaatgataaaaccaagagcagatcttgccatgatgtcccgtgtatgctgctgtcattcccacgttgcctgatccccgcctggggcaggagcaagcgtcagggctggcagagctgtgtgctgggcctcagcagggccctggcatgcgtgcccttgtggctcctctcaagtccagctgtgtgcatggaggaaacaggtcacgttaagtctctatattcttgaagtacctgaatgattgggagagccatggcgaggatcttccaggtcagcccccgtcgtgtgtgatgttccttgggctctgcggatgctcggtgctttcatcggtgtccacacctctttattccgctcctcctttgcttgtctaatcctattttgccagtaagttttttattcttgaggctttgttggccctgtgttgtatgatgattgtttttaggagttaagtaatagaacatttcctcttggatttatccatccccgatagacacattcagggtgaaagaacaacttcgcacaccggcctcttctttgcattttggctttgctttcccagtctcctcctgctgtttttcttgctctgagactttcctgaagccggcgtgtgttccctctcagtctgcttggccgcgactttgcagtgcagggaatgtgctttgggtgtagcccaagcacaggctgctgcatgctgggatcgacaggctgctgagggcgagagcgccaggtcctggcacgtgtgacttgcttggttctttctagaaggtcacagctgggggaagaacatgacagggaccttcttacttctgtttttttggagacagaatctcactccatcacccaggctggagtgcagtggtgtgatctcagctcactgcaacctccgcctcccgggttcaagcaattcttgtgcctcagcttcttgagtagctggaattacaggtgtgtgccaccacacccagccaatttttgtatttttagtagagacggggtttcaccatgttggtcaggctggtctcaagctcctgacctcaagtgacatgcctgcctcggcctcccaaagtggtggaattacaggtgcaagccattggcacctggctagggaccttcttatttctatggataagtggaacaagttagaagtgaggttctgctgaatttgtgtggtttgatcctggtacatggttcttgcctttagtcattcacggaatgggaagaatgcttttctctcagatggaggagttgggaagtcccagagggcaggtgtccatccctgctctctatgtaacatcacgtcggtgcttagtgtggtcactgcccgaggacgtgggcattgtgcctgctgtctggctccaacactgctgtctctctctttctccagcagcacaacggcatgaaactgtccatgaagggctctcacggccacacccaaggcggcggctacagctctgtgggtagcggaggtgtgcggccccctgtgggcaacaggggacaccaccagtataaccgcaccggctggaggaggaaaaaacacacacacacacgggacagtctgcccgtgagcctcagcagataatggctcctggctgcgtcagcctcccccacccctctgcagactgccccgcggcctcggccaccggcaggggaaccgagaccagcaccccgcacgtcagccgggctcgcggcacgcccgccgctgatcactctgcatgtttcttcgtgtggtggtcgcgtccatcttcaagaacagctcgttgtgctcatctgtgaagccttattaaacgtggacgttgttttctgccttcccaggattcttccttcagtgctgaggcaggtcgggctcaggaactgcagggacgtgaacatgcgcttgcggtttgaggtagccgtgtctgttccttcgcggtttgctattttcatttcctgttcgtcaaagcagcagaggagatcaaaccccgttcgtgtgtctttcctccacggataagcttgggaggtcattgttttactgccctcacattttgtttgaaatttcagaactgtttttctatgtaaatattgaaaacttatgatttgtgcaataactcagatattttttatttaatttcctattttcacataagttatatttaagggaggagggaattttttttaaacaagcttaggtcctttcccgagctgcattttctaagttgggtcatcgtgtcggctggttgtctgacgagcatcgttacaaacaccatgatgaggggtttggggttttattttgatgtcttttcttttggtcggaagtgagtgaaggagccaggtcgccctgaaggttttccaaagggcttggctccagagccacctggcagactgcccgtggccctgctgtcgggccccaggccgttgtcctgctctgaccacagagttttaatgttttggttttcacttcttttaaactggacaacaaatccagcatttcaagtgccagaagtataactttctaaggagagaagggttgtcacattataaaatctttaggaaaatgtgaactggaaaacgcttcggtcagttttagtgacatagcctgtgatgatgggtctggtgactattattgcggaccgtggtacccagttttaggaatgtggagaaaggaattctgttgattccgttgaggaatctgtagcgtatgcattcgttctgttaagagcaaatctaggagaagtgcttcagctgcccagtgcgccgtggggagtgttttaacggatcgtgtcgcaggagagcacagcccagcgttggggccgggaccgctggcgcccgacgtcggaagcatacaggtatactatgcaagtgtattctgccacaacaaccactgtctttgttacctttttttgaacaagaatatatccatcctgcctaaccctgagtttttggagcaccacagttgtcctgggagttggttgcatcttgtaggccatctgacttcctgtttttaaaacgggggtctggtcttgctaaacactacaggtaggttggtctttgaagtccactagtggagaatgtcaagacaagatacttattaccatgacatctgatgcatgtgcagcagtggggagttctagattgatctctgaatgtgatcgacgcccagcaaggacaagctttaaaatgtctgcggtctgcccttttgaagcaggactggctcactctgtcattgggagctgtcagctgcgactgcaggttctctaggaggcattccagaatagagtagcacactgtgtctgcagttctcgatgaccgaaagttatcaaaaatatttaaaatatttaaattgtgaacctattgataaagaatatttataaaaactgatctgtaggcctgtactaatctctacgcattagcaatattgactgtaaacccacattaaggaaaccactacgggtctggcagtgcgtgtcccgtggggtgtgcattttaaaactcgattcatagacacaggtaccatgttccatttccgtcatggtgaagcaaatgaattggcctggctaccactgtggtcgcgtgctacaggtttgacaaaaagatatcatgtttcgatttttttgtgtgtggacaacaatatggaagctaaaattgacatatttttatgtaaagtttttctattctttgatttttaataaactttggaaaccagttt

SEQ ID NO: 12 - DNA, 19 bp, Artificial sequence
  oligonucleotide motif
agggtagatgtgtttaact

SEQ ID NO: 13 - DNA, 17 bp, Artificial sequence
  oligonucleotide motif
cagcctaaacttagtgg

SEQ ID NO: 14 - DNA, 20 bp, Artificial sequence
  oligonucleotide motif
aagccctcaatgtaaaacac

SEQ ID NO: 15 - DNA, 19 bp, Artificial sequence
  oligonucleotide motif
aatagcaagtagaggagag

SEQ ID NO: 16 - DNA, 18 bp, Artificial sequence
  oligonucleotide motif
aaataaggatactggcga

SEQ ID NO: 17 - DNA, 20 bp, Artificial sequence
  oligonucleotide motif
gagggaacacataataaaag

SEQ ID NO: 18 - DNA, 18 bp, Artificial sequence
  oligonucleotide motif
gtaatacctctcacattc

SEQ ID NO: 19 - DNA, 19 bp, Artificial sequence
  oligonucleotide motif
agtaacaccaatctcattg

SEQ ID NO: 20 - DNA, 19 bp, Artificial sequence
  oligonucleotide motif
gtgacagtattcaatgatc

SEQ ID NO: 21 - DNA, 18 bp, Artificial sequence
  oligonucleotide motif
cagttccgtatcaccaac

SEQ ID NO: 22 - DNA, 20 bp, Artificial sequence
  oligonucleotide motif
aagtctaactcaaagccatc

SEQ ID NO: 23 - DNA, 19 bp, Artificial sequence
  oligonucleotide motif
aggcttccattttattgaa

SEQ ID NO: 24 - DNA, 18 bp, Artificial sequence
  oligonucleotide motif
ttttagaaaacgaggcta

SEQ ID NO: 25 - DNA, 17 bp, Artificial sequence
  oligonucleotide motif
gtattcttattcttgct

SEQ ID NO: 26 - DNA, 18 bp, Artificial sequence
  oligonucleotide motif
attattcccacagtaaga

SEQ ID NO: 27 - DNA, 19 bp, Artificial sequence
  oligonucleotide motif
aacaacaaacaggatgggc

SEQ ID NO: 28 - DNA, 19 bp, Artificial sequence
  oligonucleotide motif
atatccacaatattctgat

SEQ ID NO: 29 - DNA, 20 bp, Artificial sequence
  oligonucleotide motif
aaagaaataatgtcgtctgg

SEQ ID NO: 30 - DNA, 17 bp, Artificial sequence
  oligonucleotide motif
ccagagtaaacaaatcc

SEQ ID NO: 31 - DNA, 20 bp, Artificial sequence
  oligonucleotide motif
attcaacatttttagtcacc

SEQ ID NO: 32 - DNA, 20 bp, Artificial sequence
  oligonucleotide motif
tttggtaattctttttttag

SEQ ID NO: 33 - DNA, 20 bp, Artificial sequence
  oligonucleotide motif
caatgaggaaacaagagtca

SEQ ID NO: 34 - DNA, 20 bp, Artificial sequence
  oligonucleotide motif
ttcaaaataatgtgggaggt

SEQ ID NO: 35 - DNA, 20 bp, Artificial sequence
  oligonucleotide motif
ggatatttgatacggcaaat

SEQ ID NO: 36 - DNA, 17 bp, Artificial sequence
  oligonucleotide motif
ctataagaagcaaaccc

SEQ ID NO: 37 - DNA, 20 bp, Artificial sequence
  oligonucleotide motif
atataattcacgtttcactt

SEQ ID NO: 38 - DNA, 20 bp, Artificial sequence
  oligonucleotide motif
aatgattcacatgaaggtta

SEQ ID NO: 39 - DNA, 17 bp, Artificial sequence
  oligonucleotide motif
gttaggattttgctatg

SEQ ID NO: 40 - DNA, 19 bp, Artificial sequence
  oligonucleotide motif
gtacaaatatcaaccgtat

SEQ ID NO: 41 - DNA, 20 bp, Artificial sequence
  oligonucleotide motif
cacactatttcaagatgcta

SEQ ID NO: 42 - DNA, 20 bp, Artificial sequence
  oligonucleotide motif
cacctatacaatggagtatt

SEQ ID NO: 43 - DNA, 20 bp, Artificial sequence
  oligonucleotide motif
atcatacgtcattagagaac

SEQ ID NO: 44 - DNA, 19 bp, Artificial sequence
  oligonucleotide motif
cagaacagatactttgcca

SEQ ID NO: 45 - DNA, 19 bp, Artificial sequence
  oligonucleotide motif
aagaatggttggttaaggg

SEQ ID NO: 46 - DNA, 20 bp, Artificial sequence
  oligonucleotide motif
agaattggtaaactggactg

SEQ ID NO: 47 - DNA, 17 bp, Artificial sequence
  oligonucleotide motif
agaattatattggctgg

SEQ ID NO: 48 - DNA, 20 bp, Artificial sequence
  oligonucleotide motif
cctaaaccagacagaaaaga

SEQ ID NO: 49 - DNA, 19 bp, Artificial sequence
  oligonucleotide motif
accaattagagcagaaatc

SEQ ID NO: 50 - DNA, 20 bp, Artificial sequence
  oligonucleotide motif
ttctaaataacagatgggtc

SEQ ID NO: 51 - DNA, 20 bp, Artificial sequence
  oligonucleotide motif
tttataatttttttccatct

SEQ ID NO: 52 - DNA, 20 bp, Artificial sequence
  oligonucleotide motif
gcaaatatcagattaacctc

SEQ ID NO: 53 - DNA, 20 bp, Artificial sequence
  oligonucleotide motif
aacggtatggcagaagacaa

SEQ ID NO: 54 - DNA, 17 bp, Artificial sequence
  oligonucleotide motif
ttcaacctttactgcat

SEQ ID NO: 55 - DNA, 20 bp, Artificial sequence
  oligonucleotide motif
actgataaagggcatttcaa

SEQ ID NO: 56 - DNA, 17 bp, Artificial sequence
  oligonucleotide motif
cagtaggaatgtggctt

SEQ ID NO: 57 - DNA, 19 bp, Artificial sequence
  oligonucleotide motif
ttttatggcagggtttcac

SEQ ID NO: 58 - DNA, 17 bp, Artificial sequence
  oligonucleotide motif
tcactgttaaacctcac

SEQ ID NO: 59 - DNA, 20 bp, Artificial sequence
  oligonucleotide motif
caattttctaattcaatggt

SEQ ID NO: 60 - DNA, 19 bp, Artificial sequence
  oligonucleotide motif
aagatataattcacccact

SEQ ID NO: 61 - DNA, 19 bp, Artificial sequence
  oligonucleotide motif
gccacataaaggataaagt

SEQ ID NO: 62 - DNA, 19 bp, Artificial sequence
  oligonucleotide motif
cccattagaagtaaggtga

SEQ ID NO: 63 - DNA, 19 bp, Artificial sequence
  oligonucleotide motif
atgtaaattaaaacttccc

SEQ ID NO: 64 - DNA, 20 bp, Artificial sequence
  oligonucleotide motif
tgagagcataaaagtacgga

SEQ ID NO: 65 - DNA, 18 bp, Artificial sequence
  oligonucleotide motif
ttcacaacaggtaaaggg

SEQ ID NO: 66 - DNA, 20 bp, Artificial sequence
  oligonucleotide motif
tgcattcctaagtaacataa

SEQ ID NO: 67 - DNA, 20 bp, Artificial sequence
  oligonucleotide motif
agagaaaagtgatgagggaa

SEQ ID NO: 68 - DNA, 19 bp, Artificial sequence
  oligonucleotide motif
atacggatcaccagctaaa

SEQ ID NO: 69 - DNA, 19 bp, Artificial sequence
  oligonucleotide motif
catgttatgcacagaagat

SEQ ID NO: 70 - DNA, 20 bp, Artificial sequence
  oligonucleotide motif
cgctgaagaactaagtatta

SEQ ID NO: 71 - DNA, 19 bp, Artificial sequence
  oligonucleotide motif
caaacagatggtggtgata

SEQ ID NO: 72 - DNA, 16 bp, Artificial sequence
  oligonucleotide motif
agtagccattaggatg

SEQ ID NO: 73 - DNA, 19 bp, Artificial sequence
  oligonucleotide motif
atacacaggctccataata

SEQ ID NO: 74 - DNA, 20 bp, Artificial sequence
  oligonucleotide motif
gatttttgtatagtccacaa

SEQ ID NO: 75 - DNA, 20 bp, Artificial sequence
  oligonucleotide motif
gcatctataaaaaagggaca

SEQ ID NO: 76 - DNA, 15 bp, Artificial sequence
  oligonucleotide motif
agtgcaagtatcgct

SEQ ID NO: 77 - DNA, 20 bp, Artificial sequence
  oligonucleotide motif
ccaaaagaatcaagttcgta

SEQ ID NO: 78 - DNA, 19 bp, Artificial sequence
  oligonucleotide motif
cctcagaccaaatttattt

SEQ ID NO: 79 - DNA, 20 bp, Artificial sequence
  oligonucleotide motif
ttcaacaagcatctattgta

SEQ ID NO: 80 - DNA, 18 bp, Artificial sequence
  oligonucleotide motif
caaaggttgttgtactct

SEQ ID NO: 81 - DNA, 19 bp, Artificial sequence
  oligonucleotide motif
tcataaatctttttccacg

SEQ ID NO: 82 - DNA, 20 bp, Artificial sequence
  oligonucleotide motif
cttgttacggatttaatgtg

SEQ ID NO: 83 - DNA, 18 bp, Artificial sequence
  oligonucleotide motif
gctataaaaatagaagcc

SEQ ID NO: 84 - DNA, 19 bp, Artificial sequence
  oligonucleotide motif
tccttagcaaactaaacat

SEQ ID NO: 85 - DNA, 20 bp, Artificial sequence
  oligonucleotide motif
agcaaaaggcaggtattcaa

SEQ ID NO: 86 - DNA, 20 bp, Artificial sequence
  oligonucleotide motif
gaatccatttacatattcac

SEQ ID NO: 87 - DNA, 19 bp, Artificial sequence
  oligonucleotide motif
tccagtatccaaaacatac

SEQ ID NO: 88 - DNA, 19 bp, Artificial sequence
  oligonucleotide motif
agcttaaagaagaacggtt

SEQ ID NO: 89 - DNA, 17 bp, Artificial sequence
  oligonucleotide motif
cacaacgtgcctacctt

SEQ ID NO: 90 - DNA, 19 bp, Artificial sequence
  oligonucleotide motif
ccagaatccaagaaaatgg

SEQ ID NO: 91 - DNA, 20 bp, Artificial sequence
  oligonucleotide motif
tcacctcgaactaaacaagt

SEQ ID NO: 92 - DNA, 18 bp, Artificial sequence
  oligonucleotide motif
gtatctttctgtactatt

SEQ ID NO: 93 - DNA, 19 bp, Artificial sequence
  oligonucleotide motif
gtcattctactaacaaacg

SEQ ID NO: 94 - DNA, 19 bp, Artificial sequence
  oligonucleotide motif
tggaaaaggaagaaccatt

SEQ ID NO: 95 - DNA, 19 bp, Artificial sequence
  oligonucleotide motif
aatacaactcttccgtgat

SEQ ID NO: 96 - DNA, 17 bp, Artificial sequence
  oligonucleotide motif
aataccctgacgagctg

SEQ ID NO: 97 - DNA, 20 bp, Artificial sequence
  oligonucleotide motif
tcataaaacatgatccttgc

SEQ ID NO: 98 - DNA, 19 bp, Artificial sequence
  oligonucleotide motif
ctaaagcagatccatagaa

SEQ ID NO: 99 - DNA, 20 bp, Artificial sequence
  oligonucleotide motif
agactataacttttgctaca

SEQ ID NO: 100 - DNA, 20 bp, Artificial sequence
  oligonucleotide motif
agcaatgacttgaacatagt

SEQ ID NO: 101 - DNA, 19 bp, Artificial sequence
  oligonucleotide motif
ataaaacaagcatacgggc

SEQ ID NO: 102 - DNA, 19 bp, Artificial sequence
  oligonucleotide motif
atgagataccagcagatag

SEQ ID NO: 103 - DNA, 20 bp, Artificial sequence
  oligonucleotide motif
agaagaaatcctgagtaatc

SEQ ID NO: 104 - DNA, 17 bp, Artificial sequence
  oligonucleotide motif
ccctaaaaagtgacgta

SEQ ID NO: 105 - DNA, 17 bp, Artificial sequence
  oligonucleotide motif
ttaagttagatcacggc

SEQ ID NO: 106 - DNA, 17 bp, Artificial sequence
  oligonucleotide motif
gtggatacagaaagcca

SEQ ID NO: 107 - DNA, 16 bp, Artificial sequence
  oligonucleotide motif
gtatcggcaggagatt

SEQ ID NO: 108 - DNA, 20 bp, Artificial sequence
  oligonucleotide motif
taactaattgattccattgc

SEQ ID NO: 109 - DNA, 18 bp, Artificial sequence
  oligonucleotide motif
agaagaacggaaattgcc

SEQ ID NO: 110 - DNA, 18 bp, Artificial sequence
  oligonucleotide motif
ataatgattttcctatcc

SEQ ID NO: 111 - DNA, 18 bp, Artificial sequence
  oligonucleotide motif
atggttttgtggagaagg

SEQ ID NO: 112 - DNA, 20 bp, Artificial sequence
  oligonucleotide motif
tgctgctgtgaaaagaaatg

SEQ ID NO: 113 - DNA, 19 bp, Artificial sequence
  oligonucleotide motif
gtgtccaattttttattat

SEQ ID NO: 114 - DNA, 20 bp, Artificial sequence
  oligonucleotide motif
gatggaatcaactgtgtagt

SEQ ID NO: 115 - DNA, 19 bp, Artificial sequence
  oligonucleotide motif
gatggtgacaaattattct

SEQ ID NO: 116 - DNA, 17 bp, Artificial sequence
  oligonucleotide motif
tgcttttgggaatcttt

SEQ ID NO: 117 - DNA, 20 bp, Artificial sequence
  oligonucleotide motif
gatgtcctacaatgaacacg

SEQ ID NO: 118 - DNA, 19 bp, Artificial sequence
  oligonucleotide motif
gtacaaggacaaagtaacc

SEQ ID NO: 119 - DNA, 17 bp, Artificial sequence
  oligonucleotide motif
tgaaacgcctatctcta

SEQ ID NO: 120 - DNA, 20 bp, Artificial sequence
  oligonucleotide motif
atactatttatgcttatgga

SEQ ID NO: 121 - DNA, 20 bp, Artificial sequence
  oligonucleotide motif
ttgtaatcaaggcaataagg

SEQ ID NO: 122 - DNA, 18 bp, Artificial sequence
  oligonucleotide motif
gaagtccaataacgcaga

SEQ ID NO: 123 - DNA, 20 bp, Artificial sequence
  oligonucleotide motif
atatccaatctctatatgtg

SEQ ID NO: 124 - DNA, 20 bp, Artificial sequence
  oligonucleotide motif
gccttacacaagactatatt

SEQ ID NO: 125 - DNA, 19 bp, Artificial sequence
  oligonucleotide motif
tgctgaattttatgttaac

SEQ ID NO: 126 - DNA, 20 bp, Artificial sequence
  oligonucleotide motif
cacaagatgatgggtttaag

SEQ ID NO: 127 - DNA, 16 bp, Artificial sequence
  oligonucleotide motif
ttagtggtttgggtgc

SEQ ID NO: 128 - DNA, 19 bp, Artificial sequence
  oligonucleotide motif
agattgttaccttactgat

SEQ ID NO: 129 - DNA, 20 bp, Artificial sequence
  oligonucleotide motif
tattacaaatatcaatctcc

SEQ ID NO: 130 - DNA, 19 bp, Artificial sequence
  oligonucleotide motif
taccaaaagcatagagtgg

SEQ ID NO: 131 - DNA, 17 bp, Artificial sequence
  oligonucleotide motif
aattatcttcccgctac

SEQ ID NO: 132 - DNA, 17 bp, Artificial sequence
  oligonucleotide motif
gttgggtggaataggca

SEQ ID NO: 133 - DNA, 17 bp, Artificial sequence
  oligonucleotide motif
tcgatttcccgttccaa

SEQ ID NO: 134 - DNA, 20 bp, Artificial sequence
  oligonucleotide motif
acaacctacacataaattgc

SEQ ID NO: 135 - DNA, 19 bp, Artificial sequence
  oligonucleotide motif
actataagaactcccaaca

SEQ ID NO: 136 - DNA, 19 bp, Artificial sequence
  oligonucleotide motif
gagaaaaagagttacaagc

SEQ ID NO: 137 - DNA, 19 bp, Artificial sequence
  oligonucleotide motif
aactggagggagagaagag

SEQ ID NO: 138 - DNA, 20 bp, Artificial sequence
  oligonucleotide motif
tttctaagagcagaggtaca

SEQ ID NO: 139 - DNA, 17 bp, Artificial sequence
  oligonucleotide motif
agaagtaacaagagcct

SEQ ID NO: 140 - DNA, 18 bp, Artificial sequence
  oligonucleotide motif
agtatcaaaccagacctc

SEQ ID NO: 141 - DNA, 17 bp, Artificial sequence
  oligonucleotide motif
ccacaaccgaaagactt

SEQ ID NO: 142 - DNA, 19 bp, Artificial sequence
  oligonucleotide motif
aatacacactgcattttca

SEQ ID NO: 143 - DNA, 17 bp, Artificial sequence
  oligonucleotide motif
ccaggtagatagcacag

SEQ ID NO: 144 - DNA, 20 bp, Artificial sequence
  oligonucleotide motif
ccatgacaaagtaacaacag

SEQ ID NO: 145 - DNA, 19 bp, Artificial sequence
  oligonucleotide motif
cagaatttcctttgagtta

SEQ ID NO: 146 - DNA, 20 bp, Artificial sequence
  oligonucleotide motif
ccttcgcaagaaagaattga

SEQ ID NO: 147 - DNA, 18 bp, Artificial sequence
  oligonucleotide motif
tcatacatacacgcttct

SEQ ID NO: 148 - DNA, 17 bp, Artificial sequence
  oligonucleotide motif
tgcgaaaagattggagg

SEQ ID NO: 149 - DNA, 20 bp, Artificial sequence
  oligonucleotide motif
cacaggacgcttacatgaat

SEQ ID NO: 150 - DNA, 19 bp, Artificial sequence
  oligonucleotide motif
gctgtttttttttcttaac

SEQ ID NO: 151 - DNA, 19 bp, Artificial sequence
  oligonucleotide motif
accataagtgagtgttctt

SEQ ID NO: 152 - DNA, 20 bp, Artificial sequence
  oligonucleotide motif
acacaagcccatagaaacag

SEQ ID NO: 153 - DNA, 17 bp, Artificial sequence
  oligonucleotide motif
cagtagtaaccaccaag

SEQ ID NO: 154 - DNA, 19 bp, Artificial sequence
  oligonucleotide motif
cctgcaaacttttatttat

SEQ ID NO: 155 - DNA, 17 bp, Artificial sequence
  oligonucleotide motif
acttagtaatagcagca

SEQ ID NO: 156 - DNA, 19 bp, Artificial sequence
  oligonucleotide motif
atgaatactccgaagactt

SEQ ID NO: 157 - DNA, 20 bp, Artificial sequence
  oligonucleotide motif
aaagaaaaggatcacaagcc

SEQ ID NO: 158 - DNA, 19 bp, Artificial sequence
  oligonucleotide motif
agacagaaatcacctaaca

SEQ ID NO: 159 - DNA, 20 bp, Artificial sequence
  oligonucleotide motif
tagaacagacattattcatc

SEQ ID NO: 160 - DNA, 18 bp, Artificial sequence
  oligonucleotide motif
agttacacggagcagcac

SEQ ID NO: 161 - DNA, 20 bp, Artificial sequence
  oligonucleotide motif
cactatacacagaacactat

SEQ ID NO: 162 - DNA, 18 bp, Artificial sequence
  oligonucleotide motif
agctgtctaaatacatgg

SEQ ID NO: 163 - DNA, 20 bp, Artificial sequence
  oligonucleotide motif
atgaacctattttatgcttc

SEQ ID NO: 164 - DNA, 18 bp, Artificial sequence
  oligonucleotide motif
accatcattaacctgcgt

SEQ ID NO: 165 - DNA, 18 bp, Artificial sequence
  oligonucleotide motif
agtaaagtgcccagatgt

SEQ ID NO: 166 - DNA, 19 bp, Artificial sequence
  oligonucleotide motif
ttccctatgaaatcctcaa

SEQ ID NO: 167 - DNA, 20 bp, Artificial sequence
  oligonucleotide motif
cactcttcatagaatgcaac

SEQ ID NO: 168 - DNA, 20 bp, Artificial sequence
  oligonucleotide motif
aatgcttaatttttctctct

SEQ ID NO: 169 - DNA, 20 bp, Artificial sequence
  oligonucleotide motif
ttagagacgatgcctataac

SEQ ID NO: 170 - DNA, 19 bp, Artificial sequence
  oligonucleotide motif
tgaatagttcccatagatt

SEQ ID NO: 171 - DNA, 19 bp, Artificial sequence
  oligonucleotide motif
cagcataattgttttcttt

SEQ ID NO: 172 - DNA, 19 bp, Artificial sequence
  oligonucleotide motif
atgtcattatgttttagtt

SEQ ID NO: 173 - DNA, 18 bp, Artificial sequence
  oligonucleotide motif
cagcagtatctcttagaa

SEQ ID NO: 174 - DNA, 16 bp, Artificial sequence
  oligonucleotide motif
cggtaagggttcggtg

SEQ ID NO: 175 - DNA, 19 bp, Artificial sequence
  oligonucleotide motif
catgaaccacattaggaac

SEQ ID NO: 176 - DNA, 19 bp, Artificial sequence
  oligonucleotide motif
cattcaacacacacgacaa

SEQ ID NO: 177 - DNA, 19 bp, Artificial sequence
  oligonucleotide motif
aagtatccaagactcaaga

SEQ ID NO: 178 - DNA, 16 bp, Artificial sequence
  oligonucleotide motif
ccacagaaacaccgag

SEQ ID NO: 179 - DNA, 19 bp, Artificial sequence
  oligonucleotide motif
tggaaaagggaagggaaga

SEQ ID NO: 180 - DNA, 17 bp, Artificial sequence
  oligonucleotide motif
agagagtccgaagcctg

SEQ ID NO: 181 - DNA, 18 bp, Artificial sequence
  oligonucleotide motif
atgggaaaggtaacgagc

SEQ ID NO: 182 - DNA, 18 bp, Artificial sequence
  oligonucleotide motif
ctatcctacaagtccgaa

SEQ ID NO: 183 - DNA, 19 bp, Artificial sequence
  oligonucleotide motif
cattgcttttataatccta

SEQ ID NO: 184 - DNA, 18 bp, Artificial sequence
  oligonucleotide motif
ctttttaaggacaggagg

SEQ ID NO: 185 - DNA, 20 bp, Artificial sequence
  oligonucleotide motif
gatgaaagataagtgagcat

SEQ ID NO: 186 - DNA, 20 bp, Artificial sequence
  oligonucleotide motif
gaagcctgtaataattaagc

SEQ ID NO: 187 - DNA, 18 bp, Artificial sequence
  oligonucleotide motif
caccctagtaaagcaaac

SEQ ID NO: 188 - DNA, 18 bp, Artificial sequence
  oligonucleotide motif
gcaaatgtaagccttttt

SEQ ID NO: 189 - DNA, 17 bp, Artificial sequence
  oligonucleotide motif
acctgacagctaccgac

SEQ ID NO: 190 - DNA, 17 bp, Artificial sequence
  oligonucleotide motif
aagagtgggttgtaagc

SEQ ID NO: 191 - DNA, 20 bp, Artificial sequence
  oligonucleotide motif
tagtgaaaatatttggagtt

SEQ ID NO: 192 - DNA, 18 bp, Artificial sequence
  oligonucleotide motif
tttcagcaccttaaaccc

SEQ ID NO: 193 - DNA, 20 bp, Artificial sequence
  oligonucleotide motif
ttaagggaaaggaaacgtca

SEQ ID NO: 194 - DNA, 20 bp, Artificial sequence
  oligonucleotide motif
gtaggtaaagggcaaaggaa

SEQ ID NO: 195 - DNA, 18 bp, Artificial sequence
  oligonucleotide motif
gtgaattaaagccaaagc

SEQ ID NO: 196 - DNA, 19 bp, Artificial sequence
  oligonucleotide motif
tgtttttgtattttagtat

SEQ ID NO: 197 - DNA, 20 bp, Artificial sequence
  oligonucleotide motif
gaggttttttttagtgaatt

SEQ ID NO: 198 - DNA, 17 bp, Artificial sequence
  oligonucleotide motif
gaggagctaaacggaca

SEQ ID NO: 199 - DNA, 20 bp, Artificial sequence
  oligonucleotide motif
gtttagtcttatgttctcac

SEQ ID NO: 200 - DNA, 19 bp, Artificial sequence
  oligonucleotide motif
caaatactgaatatgcccg

SEQ ID NO: 201 - DNA, 18 bp, Artificial sequence
  oligonucleotide motif
accatttaaatcgccaac

SEQ ID NO: 202 - DNA, 20 bp, Artificial sequence
  oligonucleotide motif
cagtaagagtagcccaacaa

SEQ ID NO: 203 - DNA, 20 bp, Artificial sequence
  oligonucleotide motif
taacggcaacatcaaatagc

SEQ ID NO: 204 - DNA, 18 bp, Artificial sequence
  oligonucleotide motif
actgagcaccaactacac

SEQ ID NO: 205 - DNA, 20 bp, Artificial sequence
  oligonucleotide motif
cctaattttatgtatcacat

SEQ ID NO: 206 - DNA, 20 bp, Artificial sequence
  oligonucleotide motif
ctaggaattataacaaatca

SEQ ID NO: 207 - DNA, 20 bp, Artificial sequence
  oligonucleotide motif
actccaaagaacatactcac

SEQ ID NO: 208 - DNA, 20 bp, Artificial sequence
  oligonucleotide motif
taagagaaacaatcacacca

SEQ ID NO: 209 - DNA, 19 bp, Artificial sequence
  oligonucleotide motif
tgtcctaaaatatcagcag

SEQ ID NO: 210 - DNA, 19 bp, Artificial sequence
  oligonucleotide motif
cttttaatgagacagtgca

SEQ ID NO: 211 - DNA, 20 bp, Artificial sequence
  oligonucleotide motif
ttgtagcataagatggaaag

SEQ ID NO: 212 - DNA, 20 bp, Artificial sequence
  oligonucleotide motif
aaactgtagccaataactgt

SEQ ID NO: 213 - DNA, 20 bp, Artificial sequence
  oligonucleotide motif
attcatcctaacacaagtag

SEQ ID NO: 214 - DNA, 19 bp, Artificial sequence
  oligonucleotide motif
cacgaaaggaacagctaag

SEQ ID NO: 215 - DNA, 16 bp, Artificial sequence
  oligonucleotide motif
acaacaggcaagtacc

SEQ ID NO: 216 - DNA, 18 bp, Artificial sequence
  oligonucleotide motif
gctaaacactataaggat

SEQ ID NO: 217 - DNA, 18 bp, Artificial sequence
  oligonucleotide motif
cccgtaagcatttgagaa

SEQ ID NO: 218 - DNA, 20 bp, Artificial sequence
  oligonucleotide motif
agccaatatgcgacagtaac

SEQ ID NO: 219 - DNA, 20 bp, Artificial sequence
  oligonucleotide motif
taaccaaaacaatcagtgtc

SEQ ID NO: 220 - DNA, 18 bp, Artificial sequence
  oligonucleotide motif
aacagggaacaggagtta

SEQ ID NO: 221 - DNA, 17 bp, Artificial sequence
  oligonucleotide motif
atttatcaacttccacc

SEQ ID NO: 222 - DNA, 17 bp, Artificial sequence
  oligonucleotide motif
cgtttaagaccaggcac

SEQ ID NO: 223 - DNA, 20 bp, Artificial sequence
  oligonucleotide motif
acaaaggaactcaggaagag

SEQ ID NO: 224 - DNA, 17 bp, Artificial sequence
  oligonucleotide motif
tcacagacaagcaccaa

SEQ ID NO: 225 - DNA, 20 bp, Artificial sequence
  oligonucleotide motif
tactttttaaaacacgtagg

SEQ ID NO: 226 - DNA, 19 bp, Artificial sequence
  oligonucleotide motif
gcacaatcacaaagaccaa

SEQ ID NO: 227 - DNA, 18 bp, Artificial sequence
  oligonucleotide motif
tcagtaaagaacagaggc

SEQ ID NO: 228 - DNA, 19 bp, Artificial sequence
  oligonucleotide motif
catatttccaccacacaag

SEQ ID NO: 229 - DNA, 16 bp, Artificial sequence
  oligonucleotide motif
agtaaaccactgtcca

SEQ ID NO: 230 - DNA, 17 bp, Artificial sequence
  oligonucleotide motif
tcctctttggcgatata

SEQ ID NO: 231 - DNA, 19 bp, Artificial sequence
  oligonucleotide motif
cataaatacccctgaatac

SEQ ID NO: 232 - DNA, 17 bp, Artificial sequence
  oligonucleotide motif
cgattttatcaccaaca

SEQ ID NO: 233 - DNA, 20 bp, Artificial sequence
  oligonucleotide motif
acaatcaggttaagtgtgga

SEQ ID NO: 234 - DNA, 17 bp, Artificial sequence
  oligonucleotide motif
gaagccaaagactacca

SEQ ID NO: 235 - DNA, 20 bp, Artificial sequence
  oligonucleotide motif
tggtagggactgaattttaa

SEQ ID NO: 236 - DNA, 15 bp, Artificial sequence
  oligonucleotide motif
cggtagtcaatcacc

SEQ ID NO: 237 - DNA, 20 bp, Artificial sequence
  oligonucleotide motif
ctatcaaaattatttcacct

SEQ ID NO: 238 - DNA, 20 bp, Artificial sequence
  oligonucleotide motif
acgaaaatttagcatcctaa

SEQ ID NO: 239 - DNA, 15 bp, Artificial sequence
  oligonucleotide motif
tggtaaacactgggc

SEQ ID NO: 240 - DNA, 17 bp, Artificial sequence
  oligonucleotide motif
gattgttggttgtcatg

SEQ ID NO: 241 - DNA, 19 bp, Artificial sequence
  oligonucleotide motif
aattataccccacatttca

SEQ ID NO: 242 - DNA, 19 bp, Artificial sequence
  oligonucleotide motif
tgcaattagacacgttacg

SEQ ID NO: 243 - DNA, 17 bp, Artificial sequence
  oligonucleotide motif
ggcaaccaattaaacta

SEQ ID NO: 244 - DNA, 17 bp, Artificial sequence
  oligonucleotide motif
cagttttatgctaatca

SEQ ID NO: 245 - DNA, 20 bp, Artificial sequence
  oligonucleotide motif
gcaaaggaggagcggaataa

SEQ ID NO: 246 - DNA, 20 bp, Artificial sequence
  oligonucleotide motif
aaacagaagtaagaaggtcc

SEQ ID NO: 247 - DNA, 18 bp, Artificial sequence
  oligonucleotide motif
tccacttatccatagaaa

SEQ ID NO: 248 - DNA, 19 bp, Artificial sequence
  oligonucleotide motif
gctttgacgaacaggaaat

SEQ ID NO: 249 - DNA, 20 bp, Artificial sequence
  oligonucleotide motif
ttccgaccaaaagaaaagac

SEQ ID NO: 250 - DNA, 18 bp, Artificial sequence
  oligonucleotide motif
gcgacacgatccgttaaa

SEQ ID NO: 251 - DNA, 15 bp, Artificial sequence
  oligonucleotide motif
ccccgttttaaaaac

SEQ ID NO: 252 - RNA, 19 nt, artificial
  Human PAPD5 target RNA
caucaaugcuuuauaucga

SEQ ID NO: 253 - RNA, 19 nt, artificial
  Human PAPD5 target RNA
ggacgacacuucaauuauu

SEQ ID NO: 254 - RNA, 19 nt, artificial
  Human PAPD5 RNA target sequence
gauaaaggauggugguuca

SEQ ID NO: 255 - RNA, 19 nt, artificial
  human PAPD5 Target mRNA sequence
gaauagaccugagccuuca

SEQ ID NO: 256 - RNA, 19 nt, artificial
  human PAPD7 target mRNA sequence
ggagugacguugauucaga

SEQ ID NO: 257 - RNA, 19 nt, artificial
  human PAPD7 target mRNA sequence
cggaguucaucaagaauua

SEQ ID NO: 258 - RNA, 19 nt, artificial
  human PAPD7 target RNA sequence
cggaguucaucaagaauua

SEQ ID NO: 259 - RNA, 19 nt, artificial
  human PAPD7 target mRNA sequence
gcgaauagccacaugcaau

SEQ ID NO: 260 - DNA, 58 bp, artificial
  shRNA
ccgggccacatatagagattggatactcgagtatccaatctctatatgtggctttttg

SEQ ID NO: 261 - DNA, 58 bp, artificial
  shRNA
ccggccaacaaatctcagcatggatctcgagatccatgctgagatttgttggtttttg

SEQ ID NO: 262 - DNA, 58 bp, artificial
  shRNA
ccggcgcctgtaatcccagcactttctcgagaaagtgctgggattacaggcgtttttg

SEQ ID NO: 263 - DNA, 58 bp, artificial
  shRNA
ccgggcctgtaatcccagcactttactcgagtaaagtgctgggattacaggctttttg

SEQ ID NO: 264 - DNA, 58 bp, artificial
  shRNA
ccggcgatgttggaaggagttcatactcgagtatgaactccttccaacatcgtttttg

SEQ ID NO: 265 - DNA, 19 bp, artificial
  Primer
ctgtgccttgggtggcttt

SEQ ID NO: 266 - DNA, 24 bp, Artificial
  primer
aaggaaagaagtcagaaggcaaaa

SEQ ID NO: 267 - DNA, 25 bp, artificial
  probe
ttctttataagggtcgatgtccatg